European Patent Application EP 4 722 390 A1 - sequence listing, part 2

SEQ ID NO: 8 - DNA, 96311 bp, brevundimonas massiliensis
  source 1..96311: mol_type = genomic DNA
atgtagatcggctggggcgggttctgggcgggcggcgcgacggccgtgggaagcgtcaccggcaccgacacggaggcgagcggagccgccaccatgaagatgatgaggagaacgagcatgatgtccacgaaaggcgtgacattgatctcggcgttcgcctcgacggtgtacttgccgccgccggaacctgagagtttggcggccatccctcttacgccccccggtccagctgacgcgagatggagttaatcagctcggcgttgaagccgtccgaacgcgtgccgtagttcgagatgcgggtgttgaagtagttgtagaagataaccgccgggatggccgcgaacaggccgatgccggtggccagcagggcttcagcgatacccggggcgacgacggccaggttggtcgtgttcgattccgcgatgccgatgaaggagttcatgatgccgtacacggtgccgaacaggccgatgaacggaccggtcgaacccaccgaagccaggaactgctgtccgcccgacaggcgcttggccaggccggactgaaccgcagccacggcttgttgagcgcgcagcagggccgagtcgcggtgatcgccggtgaccgaaaggccggcttgacgagacagttcgatttcctcggtcgccgcagcggccatgtcggccagcgggttgccgtcgaactcgtccgaggtggcgacagcgcgcatgtccgagatcgaacgcgcaccgcggaagctttccaggaactggtcggtcttcttgttgagggcgccgaactcgaacagcttgatgagcagcagggtccacgagaagatcgaggccagcagaagggcgatcatgacgaccttcacgaccacggtcgcttccatgaacatcgagatcggggtgatgccgccgctgccgtgtccgccgctgaccgattcacccacggaagcgggtcggccggggcggcttcgggggcgccggcaggagcgcgccggcgagccgggcggcggccggggtcggctcggccggagcctgagccagaaccggcgtgctcgccatcaggacggcggcgccggccatggcgagaaggatgttcgtctttttgctatcgagcatagttcgccagttcctgcttggtctgactcgtggaaccaaaggcgcgaccggtgtcggccggccgccccccaacctgaaatttcccatttcagtcacgtcgtttccgacacgctgaatgaacctttggcttcgtcgtccggtcgcccggacgttttggcctttcgaccccttaacgaataaggcgtcctaacccctttgacgaagcggccatggagcgtcaaggccgaagcgcccctatccgccgctttgacgcagggtcagccctccaagaggagctgcaaaggcggcgatttcataatctgggacccacacgccgcccaccaaggggcgaaaagcgggatggtgcctggaggcggattcgaaccaccgacacgcggattttcaatccgctgctctaccaactgagctatccaggcaagcttccgctcgcgggagcggggtctataggcgagcgccgccgaggtgtccagcgtctgcgtcagtccttttcgacatcttcgccattggtctcgatcggctcggcggggatgctgtaatcgccgccgaaccagcggccgagatcgatgtcggcgcagcgcttggagcagaagggccggtacttcggatcagccttggccttgcggcagatcgggcagagggtcatgcgtcaaagttcctcgaaacggacggcacccgccggctggtccgcatcgacgatcaggccggcgcgcggacccagtcgacgaatgagcggctgggctatggcggccagatccggcgcggcgcaggccgcgacgcgcggcgcggtcgtatccgtcagcaggtttcgcctcatggctctgaccagggccagagccgtggtctggagtgtgggacagcccttgctgtcgcaaagtcgctcgacgaccggtcggcgtcgccacggcagcgccagctgaaccaggccaaagcggctgacaggcccgaaggcgaccgattggacgccggcgaaggcgtcgcgcgcctgcctcagcgtcgcctccccttcccggccgtcgccaacgagatcgacgacgaccaagccgccgagcgccttcagcgccagcagccgggcggtctggcgcaagccttctgcattcgcagccgcccgcgcagccgccccgtcgcgccccggcggaggccgatggtcgaagtccacggcgacaagcgctcgcgtccgctggatcgacaggtcgagcgcgcccccctgaaacacgaagtgttcggcgagagcctcgtcctcggcttccatggcggcgtcgatcgccgcgacgcccgtctgaacggcgctgtccggcgcggcgcgaatcagaagcgcacggacgtcaggggccggctgaagcagacgcggctcgccagcgccgacacccagccttcgcaggacgacgcccttggcttcacgcggttcggccgccacgaccgcttcgatgatctccccctgatgcagccgcagtctgggcggcagcggcaggaatcccggccggtccgttccaagatcgacaaaggcgcccttcaggccgggattgatctcgatgattcgaccgacgcagcgcgcctccagccgatgtcgcggctcttcgtcgtgtcgctggattaggagctgttcatagcggccgctgcgtcgaacgacgccgcgcgtctcgccaggcgtttcgtcgaggaagacctcgacgtcttcgttcatggccggacgcctgcgccgcgcagcagttgcacggtttcatagagcggcaggcccatcacggccggatggctgccgacgatccgctgcacaaaggcgccggccggcccctgaatgccgtagccgccggccttgccgcgccagtctccggaggcgacgtaggcggcgatctcgtcttgcgaaagcggcttgaagctgacgcgcgtctcgttgacccgtgcggacagccggcccgcccgcaccacggcgacgccggtgaagacccggtgattgcgaccggacagcagtttcagaaagcgggtcgcctccgcctcgtccgccgccttctccagaaaacgacgtccgaccgcgacaacggtgtcggcggcgatgaccacggcgtccggccgccgggcggcgaccacacgggccttggtggacgccagacgctcggccaggcgcggcggggtttctcccttcagcggcgcttcgtcgatgtcggcgggatcgatgtggtcgggcgtgatcccgacctgcgccaacagttcgatgcggcgcgggctggccgaagccagcacgagttcaggacggctcaccgagagcccgtccttacttgaagcgataggtgatgcggcccttggtcagatcatagggcgtcatttccaccagcaccttgtcgccggccagaacgcggatgcggttcttgcgcatcttgccggcggtgtgggcgatgatctcgtggtcgttctcgagcgtcacccggaaggtggcgttcggcagcagttcgctgacggtgccgggaaactcgagcagttcttccttagccatgcggcctctcgcgcccgatcaaaacggcatagagcccgcgccgggcgggcgcgcgggctgaaatgatcgggcctcatgcccgaaaaccaacgaatagtcgaggtcagccgcgccggtacagagcgcagaccagggtgaacaggcgtcgggccgtctcatgatccagggcgatcttgccctccagacgatcctgcagcgccttggcgccctcgttgtgcaggccgcgcctgcccatgtcgaccgattcgatctggctgggcgacgatccgcgcaacgcctcgtaatagctgtcgcagatcagaagatagtccttcagaacgcctttcaaaggggtcaggctgatggcgtaggtgcgcgagaaggccggccccgacacgtcgaacaccagccggttcagctgcagcgacaaatggaggtcgaacgggccgccttccgctcccgtcggcttgaaagtgttgtgctcgatcaggtcgaagatggcgacgcggcgctcgtgctcgatttcggccgtggcggccggcagggtggcgctgtcaagcgtgacggacgccagccggtcaggcgtgctcacgcgtcagcctcgccgggatgggtcggcgcgaccttggccggccagcgctcggacacgtccgtgaccaccgcatccaggcattcgacgtcgacgcgcaggtcgccaccgcccgaaaacatcaggatcacccgcccgcccggcgcttcgcccggttcgaagtcgagcgccagcagttccagggacgcatcgggattgcgcggcaagcgacggctcttgaccgcctgcacgtcgccgaactgcatcgccgacatcacacgcgtaccgccgcattcccagcagaagcggctaaaggcgatggtcagcctgcgcgccgccctttcccagacgatgtcgaccggccgcaggatggcgtcctgcagcgccgccgagatgatctgcaggtccgccgcgtcctccgccagcaggcgcagcggctcgaccgggccggatggcgcaggcggggccgcatcgatctcagtgctcatcaccgcttcccttgatccggcggatggtcgctccgcaggcgccgagcttttcctccaaacgctcgaacccgcgatccagatgatagacgcgtcccaccgtggtctcgccctgggcgatcagcccggcgatcaccaggctgacggaggcgcgcagatcggtggccatgacgggcgcgcctcgcagttccggcaccccggtcaccttcgcctcgccggcgtgaaccgagatgtcggcgccgagacgggccagctccggcgcgtgcatgaagcggttctcgaagatgttctcgtgaatggtgctgacgccctcggccgtggtcatcagggccatgaactgcgcctgcagatccgtggcgaagccaggatagacctcggtcgccacatcgacggccttaaggcgctgcttggggtcgcgcttgatgatcacgccgtcttcggttggcgtgatctccacgccggcctcgaccatcctgtccgtcagcgaagcgatcagatcggcgcgagcgcgggtcaggcgcacctcgccgcccgccatggcggctgcgacggcgtaggagcccatttcgatccggtccgggatcaccgaccaggtcgcgccgttcaacgaggtcacgcccgtgatcgtcagcgtatcggtgtccaccccctcgatcttcgcccccatggcgatcagacagcgggccaggtcgccgatctcgggctcacgcgcggcgcgcttcagcacggtgacgccttcggccatgacggcggccagcagggtgtgctcggtcgcgccgaccgacacgaacggaaattcgatctcggcgccccgcaggcccttcggcgccatggccgagacatagccctcctccagctcgatggaggcgcccagcttggaaagggcgtccaagtgcaggtccaccggacgggctccgatggtgcagccgcccggcagcgacacccgcgcatggccggtcctggccagcaaaggccccagcacgttgaaggaggcgcgcatctgccgcaccaggtcatagggggcgaaggtggagcggatctcgcgcccgtcgaacagcgtctcctgcccgtccgctccgtcgcgctcggtcacttcgatcccgaactggcgcagcagctggcccaggaaacgcgtatcggccaggcgcggcatgttggtcagcagcagcggctgatccgtcaggatcgaggcggccatcagcttgatggcggagttcttggcgccgctgaccggaatcgatccgttcagctgggcgccgccctgaatggcgatgctgtccatgacgtccttgaggcgagcgctccgaagctgactgtcgcttcggagccggcctctctagcaagccccctcgccgccgccaaatcctgcgggtgtcgccgcgatgactttcagttgcggctgaccggcggggcgggatcggacttcggcgccttgcgacggcgcagattctcccgaagcgccttggccagacgcgccgcgcgctcggcctttgcacggtccgccggactgatccgtacaggctcgtcggcggtcggatcgagcgccggttccgtcgaaagccggtcgcgaggaggttgggtcatggcgcgatgatgagcccggccgaaagttttgatcaagacgcgatatgggcttcccacgccggaatcgtttggctatacggccgcttcctcagatcagggccgccgtagctcagtggtagagcgcatccttggtaaggctgaggtcggcagttcaatcctgcccggcggcaccatctgaaggtaagtgtggcgggctcttcggagcccgccctcatctcactccccaccgattcaaaccggaacaaacggcgaagcccccactcgaatgtggggataatccggggacacgttccgggtctgtttcgagaatcgccgtcgccttcagagcctaaatacaggcatgaggtattcggaaattgtcgcggaggacacgacgcgcccggcgtcgaagacccccgccgtaaaggccgccgaagccgcgcgtaagcgcagcgatgccgccgcgaactatcaagacaccctcgccgcagcacgcgacaaaaacgccgcagcgagccgcacgcgggcaaaggcggcccgaacctatcagaacgcgatgaaggccgcccagtgaccgcctgagaggctgtcagaccctattgcaacgccagcgagcgacggacattgctatccgctgctggacgccactacgttcgctatgggctgaacgtgagcgcgctttgcgcaaggcagatggggcacccggatgaaccaagcgacattcgcagcacggtatagaaacgagccagatgaggctctggctgcgcttcaagagaccgtcggggatttggtgccggaagcgcaagctgccctcgcagccgagattgcacgacgcggattagacaccgaggccgttcgcgcgcagggcgtcgccatcgacacggcgataaagacgaggaagtcagccgccctgaaacgcaccctgtgctttctcgtcgggatggtgctcgcagtattcacactgggcgcattggggcttcaactgggtgcgataccctacatgatggtcttagccgcatctggtcttctcgcccaatggctcatcatgatgcttttcagccgccgttgagcacggtcgaactcaggctggcctttcccagccgctgatgttttcccgttgcctcacagctacgcattgcctcacagctacgcattgcgtgtcggatcgacaggcaacagccagttcaaaacgcgacgcccatccgatttcaggaaccctactctcggctggctgaccatcgctatcggaaggactgcgcgctccaaaactggaacgagcagaccgcatcatctgacatcacgccgttctctttggtggcgtagtcgagcgcgcccgcgctgcgcagggcttggcagttcacggttcccccggacaccgcgcgcttccaacagtgctcgatgtgcgcggggaaatcggcgaccggttgccgtgcgttggcgtcatccggcctcatgaacagaccgtggaaatgcgggtaggagtcgaacttctccggcacgacaaggaacagcgtccggtcaggtgcgccgtagttgtagaagcgtccgccgagccgcaccgcgtcgaggtcgtgggacaagtcgcgcagcgcggcgaccgccgatgccgggcgaaccatgccccgccagttgaacgtaagcgtcacgaagtaagattcacctcgactgaacagttccgtccagttctcgttcagttgttttcgtttaatactcatctcgtcagacattatcatacctccgccttgcatcggtatatttacttgtgctgttgacgtagaaatagatatcgcgcaagatggtcgtgaaggcgcataatacagacagtcttaggaactgtctttcgtgcttacatctacttggccaaccgtgaggagcgtgcgtgatcttgtgtcatcgggaactgtcccgtgctcggaagacacgcttcggcggctggcaaagaagcacggcatcggcgcgaagttcgggcgaacgctcggcttcaccgaagacgactaccgcaacctcttgaaagccctgtcgtgcccctcaaactcgtccgccgtcacaactccccgaactactacatccgtggctccgtcaagggcatgcgcatcgacgaaagcactggcgttgatcgagaaaaagctgcgcgagaaatcctcacgctccgggaagccgaactgatcaaggagtcgattcacggccccgccgccgtgcgcaccttcgccgacgccgtgagcagctatgtgatggcgaacggtgaggtgacgcacctgtcgccgctcgttcaccacttcggttcgaccaagctggcgcgcatcggtcaggaacagatcgacgccgccgcgcgcaagctcggcgacggcaagtcgcccgctacgatcaaccgtcaaatctacacgccgatggccgccgtgttgaaccatgccgcgcggatgaactggtgctccaagcccatcatcgcgcgacccgagcagcccaaaggtcgcgtgcgctggatttctgaagtcgaagccgacgcactgatcgacgctgctgctccgcacctgcgcgcactcgtcgtcttcctcctgtccacaggcgcgcggttgtcagaggccctctatctggactggcgtgatgtcgatctcgacgcccgtcgcgtcgtgttcgtcaagaccaagaacggcgagcgtcgcagcgtgacgcttcacgaacgggtcgtgcgagaactgcgagctacaccgcaccggagcggcgcggtgttccgcagacccgatggatgcggctacgtcgaccgtggtggcgcaggtggcggtcaggtgaagacggcgtggaagaccatgtgccgtcgcgccaacatcacagatttcagcccccacgactgccgacacacttgggcgacgtggcactatcgcgcgaaccgcgacctgaccgcgcttcaaacgctcggggggtggaaatccgtggacatggtgatgcgatacgcccacgcgaaccgcgacgaacacgccgccggaatcgaccgtttgtggggaaaaggcggggagacttccgcaatggccgcttaaagcccgccattactgggttccacaacccaccccatatccttggtaaggctgaggtcggcagttcaatcctgcccggcggcaccatcatcaaggggccaggtcaccgacctggccctttggccattctcctcatcgtctctgatcggatccagcgcgtttcgcgtcgcagctacaccgcttcggcgtaggagcgcgcgctggcttcataactggacagcgagcgcatccgctcggggttgagcagcacggcctttccgcttcggatgtccgccaggccctcctggcgcagctgttgcagcgtgcggttgacgtgcacgaggctcagcccgagcatcgaagcgagttgctcgttcgtcagcggcatgtcgaagacgccggcctccgccagacccaccgcgcccagccggtcatgaacttccagcatcagggtggcgagccgttcgacggcggtctgctgacccaggcggacgacgtggtccagcaggcgcatctcgtcgtggcgcgacaccagggtcagagcctcccacagggcgggattgacggcgccgcgggacgtcatggtctcgatcagcgcggaggcgtcgcaggtctggaccgaagtcaccgcgacggttgaagacaaggctcgcgggctcggtcgccagcacaggccgatcaggtcgcctgggagaacaagcgcgaagacttggcggcggcctgtcggcagggtccgcgtccgccacgcccagcccgaggtcagcacgcgggggccgagaacttgctccccctgctgcaagagcacagaaccggccgcatgcggtgcgccgggccggaccatctcctggacgaatcgcgcctcgtcttcgccaagagggcagagagccgacagacggcgcaccagattctcgctcgtgatctctctcatccccatctccaatggcgccgcctgatccggcgacgtgtcgaggcagctacgaaccggcgaccggggcggatgaccaaagccgacgatcgccgcggatgtgtcaggcagagacatggaagtcgtcccgacctcctcgctgcaaatctcgcgcaagggtctgctggcgggcgacgacgttccgcgcgataaggcgggcgatgaatacgacttcttccatcgacgtgctgctggtcggcgcaggtctggccaacagcctgatcgcgctgcgcctccgcagcctgcgtccggagcttcgcgtcgtgatgatcgaagcccggccggccgccgacgacgcccatacctggtgcctgttcgacgccgatgtgtcgacttccgaccgcgcctgggtgcggccgctgctggaccatcattgggatggctacgatgtcgcctttccggagttccggcggactttgtcgaccggatacggctgcctgaccagccgcaccctggcccatgaggtcgagcaggcgctaggcgaggacatgcgctacggctgcggagcggcggcagtgggcgcgcgctctgtgacgctggacgaccgggagcgcctggaggcgtcgctggtcatcgacggccgcggcgcccgaggttcggacgcggtgtccctggcatggcagaagtttgtcgggctggagctgcgcctgaagtcgccgcatgggcttgaacggccgatcgtcaaggacgccaccattccgcagcgggacggctatcgtttcatctatgtccttcccctgtcgggcgacaccctgctgatcgaggacacgcgctacagcgccggggccgagctggatcaggacgatctctccaacgaggtcctggcctatgctgcggccaaaggctgggccgtagggtcggtgctgcggcgcgaaagcggtgtcctgccgatcacgctgggcggcgatccggaccgctactggtccgaactggacggagacgcagcgcgctccggtctgcgcgccctgctgtttcacccggtgacgggctactcgttgccggaggcggtcggcctggcgtcggcgatcgcctcctgttcagcgctggacaccgcgacggtggccgcgttggcgcgacatcgatccgacgccctgtggcggcgcaacgcctatctgcgccttctgaaccgcatgatgttcaacgccgccgagcccgcggaacgctacaaggtgctgcaacgcttctacaccctgcctcagccgctggtggagcgcttctacgccggacggctgacgtggggcgaccgactgcgcatcctcagcggcaagccgcccgttcctgttcacaaggcgctccgcgcttttcgcctcaagggagatcgtccgcatggctgacgcggttgtcatcggcaccggcttcggcggtctggccctggccatccggctgcagtcggcggggcaccaggtgacgctggtcgaggcgcgggatcgccccggcggccgggcctatgtctaccagcaggacggcttcaccttcgacgccggccccaccgtcatcaccgatccctcgtgcctggaggagttgttcgccctgtcgggccgcaagctgtcggactatgtcgagctgctgccgatcacgcccttctatcgcctgctgtgggacgacggcgcgtccttcgactacgtcaacgaccaggccgagctggatcgccagatcgccgccatgaacccggacgacgtcgacggctatcgccgctttctcgactactccacctccgtcttcgaggaaggttatctgaagctcggccatgtgcctttcatgaccgtcggcagcatgatgcgcgccgcgccgcagctggtcggcctccaggcctggcgcagcgtctattcgatggtctccaccttcgtgaaggacgagcacctgcgtcaggcgttgagcttccacaccctgctggtgggcggcaatccgttctccgcctcgtcgatctatgccctgatccatgcgctggagcgcaagtggggcgtgtggttcccgcgtggcggcaccggcgctttggtggatggaatggtgcgtctcttcaaagacgtgggtggcgttcttcgcacctcgacgccggccgagcagatcctggtcgagaacgatcgcgcggtcggcgtgcggctggccggcggcgaagtgctgcgcgccgatctggtcgcctccaacggcgacgtggtccacacctatgaccgcctcctgggcgagagcgggcgaggcaggaaggcggcggctgggctgaagaagcgccgcttctccatgtcgctgttcgtggtctacttcggtctgaagacgcccgcgcctgccgacatgaaacaccacacgattctgttcgggccggaatacaaggcgttggtcgactcgatctgcggggccaagccgctgcgcgaggacttctcgctgtatctgcacgcgcccagcgtcacggatccctcgctcgcgcctgaggggtgcagcggctactacgttctgtcgcccgtgccgaacctgtcgcaggatatcgactgggccgccgaagggccgaaatacgcggaccgcatcctcgaggctctggaacgtcgcgccatccccggcttgcgagagaacctggtcacgatgcgcaccttcacgcccgccgacttcaagaccgaactcggcgcgcacctcggctccgccttctctctggagccgatcctgacgcagagcgcctatttccgcgtgcacaatcgcgacgacgtgctgggcaacgtttatttcgtaggcgcgggcacccatccgggcgcgggcgtgccgggggtggtgggatcggctaaggccaccgcttccgtcatcgccgaggatttccccggcgttgcgcccgcccaggccgcctgacatggaccagatcgtccagcagagccgcgagaccatggcgcagggctccgccagctttcgcgccgccacccgcctgttcgaccggccgctgcgcgaggacgtctgggcgctctacgcctggtgccgctattgcgacgacgagatcgacgggcaggagctgggtcacggcttccagcccatgacgcgcgaggagcggctggcgcgattgcagcggctgcgcgtcctgacccgcaaggctatggcgggcgagccgaccgacgagccgccgttccaggctctggagcgcgtcgcctcccaccacgcactcgacgatcagtggccgcaggagttgctggacggtttcgccatggacgtggaggagcgccgctaccggaccaccgacgaactgctggagtactgctggggcgtggccggcgtggtgggcgtgatgatggccgccatcatgggggcgaccacaacgccggtgctgcggcgtgcgcaggatctcgggctggcctttcagctgaccaacatcgtgcgcgacatcatggaggacgccgaggccggccgcctttatgtgcccgaacagactctggcccgcgccggagcgcccgcgacccccgccgccttggcgatcgcgcggcgcgaggcggtgtttcaggccgcgctggaactgctggatctggcggaggtctattattcctcctcgcgggcgggccttcgcgccctgcccttccgcgcggcgctggcgacggcggcggcgcggggagtctatcgcgagatcggccgccgcatccgacgcgccggtccgcacgccctgaacggacgcatgaccgtgccgcgccggatcaagctggttctggtgctgcgggggacgctggtggccttatggagccggctggagaagctgccgcccctcccgccgcgccagcccctatggtcgcggatctgagcctgcgcgctccagccgacgctgtcgcaactcggccgagaagcgacgcacgtcgccgggcagcagaaagccgaacgaaacgccgtcctccttgcccttgacggcgtggtgcattcggtgcgcctgcaccagccgcttgaagtagcccttgcgcggcgtgtagcggaacggccagcgctggtgcaccaggccgtcgtgcaccagggcgtagagcgcgccataggcggtgatgcccgccgccgtccagaacatccacggctggtccagcgccgagcccagggcgaacaggccgatggccatgccggcgaagatcacggcgaacaggtcgttcagctcgaatgcaccatgcctcggctcgtgatgcgagcgatgcagcacccacagcggcccatgcatgacgtagcggtgggtcgcccacgccacccactccatgcccacgagcgcgcccaggaaacaggcgccgttgatcagccattccgacatggcgccagcttacgcgatccgaaggcataagccgagcggcgccgttcgtattgacgcggaagctgcgaactggcgttgaggtcccgtgcggttcctcttcaccaccttcgagggcggcgggcacgtcgccccggccatcaccttcgccgcccggcttcaggctcggggacataaggtgctgttcgtctcagatgaagcgaatcaggcggccgccgaacgggccggcctcgtcttccgatcctggcggcgggcgcccaacagatccgccggcggccgtgccgacgatccgcttcaggactggcgccacatctggccgcccgccgtggtcaaggcggtgtgcaaggccgtgatgaccggtccggccgaggcgtatgcgctggacgcccgcgaactgatctccgacttccagccggatgtcgtggtgtcgaacgaactgctgctcggcgtcgccgtcgccgccgaagcgacagggacgcccctcgccttcctctcggccaatgtctggagcctaccgacacgcgccgacacgccgcctttcggaccgggatttgcgcccgcgcgcaccagcttcgaacaaaggcgcgaacagtcggcgcgcggcatgatcgccggcttctacgacgtgggcctcgccgacctgaaccgcgcccgcgccgcgctggaccttccaccgctcgcgcatgtcatggatcagatcgacgccgcccgtatgatcgtgctggccacaagcgccgccttcgacttcggcgacacccctccgcccgagcccttcgtctactgcggtccgctgctggaccggccggcgtgggtcgaggacgtctcgatcgagcatctgctcagcgaaacggaccccaatgtgctgatttcattcagcaccaccttccaggaccagcgcggaatcatggcccgctgcatcaaggccttggccaggctgccggtgcacgggatcgtcacgaccgggccggcggtgcggcccggcgatctgccctctgcgtcgaacatcgtggtggtgcagagcgccccccacgaccggctggtcccaagatgcgccgccgtgatctcgcacggcggccacgggacgctgctgcgccccctcctgcacggtgtgccggtcgtctgcatttcgatgggccgggaccatccggagaacgcgcggcgtatgaccgagcgaggggccggcctgcgcgtctcgcgctggtcgtcggcctcgaccatccgccgggcggccgtgcgggtcctcaacgagcccgccttcaccgacggcgctcggcgcctgtccgcgtcgatcaaggcgctcggcgacgaatcagggccggcgatcgagcggctggaggttttggctcagcgcagccgcagggtctgaacgctgtcgccgcgcacctcgaacgacgccgcctgccacgacgccaggccgaagcgtccccgggcgttgttggagaagccataaggctcgctgggcatgccgatgggccaggtgttcagccggccgtcgttgttcttgtcgtgaaagaccatcaggccgtagcggccgggcgccaggccgtcgatgcggacgcggctgttcggaccggcggccaccttctgggtgcggacgggccggtcgcgcgacttccagtccgcctccttgtcgaacaccgcgaccacgacggagccctctgcggtgagacctggcgtgcggacctcaagggcggcgccgcgcgattgcgccacggccgcgccggcgcccacagcgacgacaagggccgcgcaggccagcgagatggatcgaaacatgtcagaactcccccgagcgtgacgttgagatcagtcgttcagcatcgattcgagccgctgctcgcgccacggctcttcgcgcctgtcccggctgttgctccagtcgagacccaccgccacgctgcggctgcgcccgacgcggtgaggatcatatccaaacccgcccaagcgcccatagccatagccgtccaacgcgcccggaccgtagccgtagccgtacggcaggttgcgtccttcgctgtaggcgacggtcagatcggcctgttcgccgatcggcatggtcaccgccgcgccgaagctgcggtagccgccggtgccgattccagccgagacgaccccgtgcatcttgcgctcttcgggcgagccgacgaggtcgtcctcggcgtagggcgcggcgtccgagcgggttcgggcggccagccagcgctcaatctgctcgtcggtggtcaggtcgtgcggcgcggcgtcctggctggtcggcgtggcggcgaccaccggttcgggtgcggtcagggcgcgtgcgagagctgcggtgtcgttcggggcggtggtcaccacgccgtcaggatcaccggcgaggctcgccaaggccgcaagaacaaggatcatggccgtctccttcgccgcctatctaccacagcgaatacggccaacgtcaggccgttccgtcgccgcgctttaaaggatcgggcaacgcctcgccttcggccacgaactccagcgccacagagttgatgcagtagcggtttcccgtcggcggcgggccgtcgggaaagacgtgcccctggtgactgtcgcagcgggcgcagcgcgtctcgattcgcaccatgccgtagctggtgtcgcggatcgccagcacatggtcctcatccaccggctcggtgaagctgggccagccggtgccgctttcgaacttggtgcggcttcggaacagcggcaggccgcactcgcgacagcagaagacgcccgcgcgcttttcgcccagcagcgtgccgcagaacggcgcctcggtgccgtgcgccagcaggacccgcttttcttcggggctcagcgccgcctccagccgggcgcgctcgtcgtcgctgggcggcgtcaggtcaaagccggcggcggagcgggtctgggtgggggatgctaggtcggtcatggttggaaaataggtgccgcggctccaggttccagcggcgccgtctcgccgaagatgcggcgaaagctgatcctcagcgcctcgtccgcatcgtccatggtgacgggcacgcctaggtcgatcaggctggtgacgccgtgctcctggatgccgcagggcacgatgccgccgaagtgatccagatccggctccacgttcaggctgacgccatgaaagctgacccatttgcggaccttgacgccgatcgcggcgatcttgtcctcgcgcgaccagccgggtcccttgcgctcgacccagacgccgacgcggccctctcgcacgtccgcctcgacgccgaactcggccagggcaccgatgatccattgctccagcccgcgcacaaaggcccgcacgtcccgcccgcgccggttcaggtccagcatcacataggcaacccgctggcccggcccgtgataggtgaactggcctccgcgtccggtctggtgcacctcgaaccggtccggctgcagcaggtcctccctccgcgccgaaacgccggcggtgtacagcggcggatgctcgatcagccagacccgctcgggcgcctcgccggcggcgatcgccgccgcgcgcgtctccatctcggccaccgcttccagatagggaatccgcccgggtgacacgacccactcgacggcccggccgtcgtcacggcgcagcttcaggaggtcgggacttaacggctcggcaagcataaccgcttcaatgtggatggcggggcggcggcgccaggtcgcgcggcgttccttgtccttttgggagaccagtctcttgagccagatcaacgccgtcgacgtggagatttccgtcgtgctgggccgctcggtcctgccgatgagccagctgctgcgcatgggccgcggcgcggtgatcgccttggacgcgtccgagcaggacgaggtctggatcctggccaacaaccatcccgtggcgcgcggcgagatcgagatccgcgacgatcgcatcgccatcacggtgacccggcccgccgacgtctacgacttcatggcgggcgcggcctgattgtcacgcggggtgtgacaaaccccttccttttggccccgacctccgctattgccgccgctccgatgcgagcggtcgtggcggaattggtagacgcgcagcgttgaggtcgctgtggggcaacccgtggaagttcgagtcttctcgaccgcaccatctgatggaacaggataggcgttcggctctaccaggctgacatttcgagggaggtccaccgcgatgagcgacgccgcaaccctcgaacctcctgtcgatgtcgaggagcacgccgctctcgacgaggactacgtcctcaccaccggctttgtcgaaaaggtcgtggacgccgccgacgacggcgacggcgtgcggctgcgttcgctgctggaggacctgcacccggccgacgtcgcggacctgatgggctttctgacggccgagcaccgggccgtcgtggtgctgtggctgccgcccgaactgctggccgacaccctgcccgagctggacgacggcatccgcgaggaggtgctggagcgggtccccaacgccaccctggccgaggcgctgcaggagctcgattcggacgacgccgccgccgtggtcgaggacctggaggacgaccagcgcgagcgcgtgctggcggccatgcccgagctcgaccgggcggccatcgaaagctcgctgggttacgaggaggactccgccggccgcctgatgcagcgcgaggtcatggccgcgccgcagttctggagcgtcggcgacaccatcgaccacgtccgggcccagggcgaggacctgcccgagttgttcttcgacgtctatgttgtcgatccgttgaacaagccggtcggcggcgttgcgatcagccgcctgctgcgcagcccccgcgacaccaatctgacggacctgatggagccggtgaacgccatcgccgtggaccaggatcaggaagaggtcgcctatatcttcgagaagtaccacctgatctcggcgccggtgacggacgcggccggtcggctggtcggccagatcaccgtcgacgacatcgtcaacatcattcaggaagagaaccgcgaggacatcctgcgcctggccggcgtcgccgacgaggatcggggctcgggcgtgctggagatcgttcgtggtcgcgtgccctggctgaccatcaacctggcgaccgccgtcctcggcgccagcgtgatcggttggttcgagggcaccattcagcagatcgtggctctggccgtgctgatgcccatcgtctcggccttgggcggcaacgccggcacccaggcgctgaccgtgaccgtccgggcgctggcgacgcgcgagctgaacgcctccaacgccgtgcggaccttctggcgcgaactgctggtcggctgcgccaacggcctggtgctggcgccgctgatcggcgtggcggctggattgtgggccggagactggcgcatgggggcggtgatcggcgcggccatggtgctgaacctcctggtcgccgcgaccgtgggcgttctgacgccgctgacgctgtccaagctgaagttcgacccggcggtatcgtcggccgttttcgtcacggcgacgacagatttcttcggcttcctgatcttcctgggccttgccacggtggtgctgctctgagcgggaaccgtcagtcgggctcggaccttgctaagccttctgaaaaccgtcccgctcgtcttcaaatggaacagatcgtgtcctccgacaggcagaaaccgacccgcatctcccgcgaaggcgtggtgctcatcaagagcttcgagggcttccgctcgcgcgcggtgtcgcgcccggacggcggctggatcatcggctacggccatacggcctcggcccgggagggtctgactgtttcggaagcggacgccgaactgctgctgcagtacgacctgatccccgtggtgcgcgccctgcacgaagaggtgcgtgtccctctgaaccagcatcagttcgacgccctcgccagcttcgccttctcggtcggcgtcgagcgcttcctcacctcgcgcgtgctggaccgcgtcaacgccggcgcgctcggcgaagcggccgaggccctgacgcaggagccggaggtcgagcgcgctccgaccccgccgcgccgccgcacggccgagcgcgccctgttcgtcgccgcgcccggcgcgccggtgaccctgtcggacctgttcctgaccgccctccccttccccgcccaggaagacggcctggcggccaacgacgcgtccggcgacttggcgcagaccgccgaggtgctgcccttccccttcgcggctcaggacgctgagcccgaaggtagagaacccgccgtttctctgtcggagcccgtcgacgggccaggcccggccatggccttcgcctcgccctacgtcgccgccgcaggctctcttccggacctgacgccggcggcgaacgcggtggacgccgcggctccgctggtcagcgaaggcccggctcccgaaacggccatcacggtcgcacccgtcgaggctgccgccgcatcggctatcgctctgcagccgtcgccggagcttgccggcgagatgcagcctcaagccgaggctgcgcccgctgttgacgcgcccgtcgccgctgaagcaacgccggctccatcgcagactccgccgctgaagaagggcaagcagcgatcgaacgcgggcaagttcgactggaacgaaacaggcgcctttctgatcatggggggcatcggtctggtggcgttcggcgccgccgccgccgcctttcgtcgcgcgggcgtcacctcgagccgggaggcgttcgtcatagggtcggtgctggcggtgatcgccctggtctgcatcgtcacctccagcttcagcctctactccaagtggagcacgccggacgcccggtgacgctttcgcagcccggcgcccggtgctaggccaacggcatgagcacccatgcgcccctgaacttcggcctcggcgagaccgccgacgccatccgcgacaccaccgcccgctgggccgccgaccggctggctccgctcgccgccgagatcgacgcaagcaacagcttccgccgcgagctgtggcccgagatgggcgagctgggcctgcacggcgtcacggtcgaggaggaatacggcggccttggtctcggctaccttgagcatgtggtggcgatggaggaggtgtcgcgcgcctcggcctcgatcggcctggcctacggcgcccattccaacctgtgcgtcaaccagatccgccgctggggcacgcccgagcagaagacgcgctacctgccccggctgatctcgggcgagcacgtcggttcgctagccatgtccgaggccggcgccggctccgacgtcatgtccatgcgcacgcgggccgagaagaagggtgaccgctacgtcctgaacgggaccaagttctggatcaccaacgccccgcacgccgacaccctggtcgtctacgcccgcacgggcgagggcaacggcggcgtcacggccttcctgatcgagaagggcatggcgggcttcagcgtgtccaagaagctggacaagatgggcatgcgcggctccgacaccgccgagctggtgttcgaggactgcgaggttccggctgagaacgtcatgggcggtgaaggacgcggcgcggccgtactgatgagcgggctggactatgagcgggcggtgctgtcggccgggccgctgggcatcatgcaggcggcgctggacgtggttctgccctatgtgcgcgagcgcaagcagttcggccgagcgatcggctcgttccagctgatgcaggccaaggtcgccgacatgtacgtcgccctgaacagcgcccgcgcctatgtctacgccgtggcgcgcgcctgcgatgcgggccagaccacgcgctacgacgccgccggcgccatcctgctggcctcggagaatgcggtgaaagtcacgctcgaagccgtgcaggccctgggcggcgccggctacaccaaggagtggccggtcgagcgcctggtgcgcgacgccaagctctatgacatcggcgcgggcaccaacgaaatccgccgctttctgatcgggcgggagctgcttggcgcctgagggaacgggcgcgaccagacggctttcctctgagaacgcagaggagagctcgtcatgcccgccaaatccgccgcccagcagaaggccgccggcgccgccctgtcggccaagcgcggcgacacgcccaagtccaagctccaaggggcttccaggtcgatggaggagtcgatgtcggaaaagcagctggaagagctggcccacaccagccgcaagggcaagcccgagcacaaatccaacagctgacccgacctacaaattcaacagcctggcggacggcggtggtcacggcgaggcgcaggctctacatggcgctcaccgcctagtgagccccgccatgtccgagtccagtcagtccagcgacgcgcgccgcttctcggacgtgcttgagcagttggccggcggcgccgagcctcgtctgacgctgcgcgaactggtcgccgccttcggcgagcggggcttcggcgccctgatcctggttctgtcgctgctggcgctgctgccgtggccgcccggcggcaaggcggtgttcggactgccgatcatcctcttgtcgatcgaactggccttgcagcgggacgaggtctggcttccgcgctggatcttgcgggcctcggtcagccgatcggccttcgggcgaggcatccgccggatcatgcggcccgtgcgattcgtggagaatctgacgcgccctcgcctgctgtttatgacaggcgaggtggcggacgtcttcaccggcgtggtctgcgtgctgctggccatgatgatggcgctgcccatccccttcggcgacatgctgccgggcgtcgcgctggcgctgttcgccctgggcatgatgcagcgcgacggagtggcggtgctgctgggcggggggggggcccgcccgtgcggcctctatctctttctgatctggaccaccgtggtcgaggtcggggggcgtgtgtggcagtggatcacaggtctgttctgacctacgggcgaaaataaaaagggccggcggatcgttccgccggcccttcattgtctgaccgctgtgacggtccgaccacgtcgacctgaaaggtgatcaggcccgaacctctccgaggcccagggtcgcggccgccgtacgcgattgatgacaatgagacactggatcacctcctttcgataccacgtcacacttgacgctccgaacaacataggaacatcgggcggactggcaagagtgtcggaaatctcaggcaaaaatggttgccagatgggagttccatgagacgcttcgaggtcatcccccggtctggagcctcatgtccgctacgccttgcatcatctatgcccgtttctcatccgcccagcaggagcgcggatcgtccatcgagcgtcagcttgaacttgcccgcgcgcacatccagcgcatggggtggaccgaagtcgaagtggtcatggacaagggtcgttccgcttggaagggcgaccaccttcgcaaaggcaaccttggcaacctgaacaagaggatcatggccggggagatcgcgccggggacggtcctccttgctgaaaagctggatcgtttcagccgtcaggatcgcagaatcacccgacgctggcttgaggacgtgaccgaccttgggatcggaatcggcacggtggacggcgggcggctctacaccgccgccacgctggccgcgaacatgaccgaagacatcgaaattctgatccgcgccgaacttgcgtggaaagagagcgagcagaaatcggaaaggatcatgcacgctcaagctcgcaaccgggagaaagcggcgcaaggccgggtgatgtcaaagcgttgtcccggctggctccgagtggagaatggcgcgttcgtagtggtcgaggaacgggccaagatcgtccgtcagattttcgagtggacggttcagggcttcggcgcccgcgccgtggccaagatgctgaacgacatcccggtctccagcttcggtcgcaagggttgggagccgacttatgtcagcgagatcatcgcctccccggcggtggaaggcgatcaccagccgacgcgcaaggtcggaggaaagaaggtcgccaccttcgcgccgatccacaactattaccctcggatcgttgacgccgatctggttcagcgcgcgcgggaaagccgtcagacccgcaccaagaccggcggctctcaccgctatggatgggcgaacctttttcagggcgtgatccggtgtgacgtgatggtgtggacgacctccgcctgacgggctgttctgggtgtgtcgtcatcagggacgtcacgtctaggagcggtatcatgcagaccatcgctgtcgtcgggctcgatctggcgaagactgttttccaggttcacggtgtagccacagacggcacggtcgtcgtgagacggcaactgcggcgcggccaggtgctggccttcttccagtcgattgggccgtgcctgatcgggatcgaggcgtgcgcctcagcccaccactgggcgcgtgaactgatggcgatcggccacgatgttcggctcatgccgccggcgtacgtgaaggcctatgtgaagcgcggcaagaccgacgccgccgacgctgaagcgattgccgaggctgtcacccggccgaccatgcggttcgtggctgtgaagtcgaaggcccagcaggcggtgttgatgctgcacaagacccgggatctcctggttcgtcagcgaacgatgctgatcaacgcactgcggggccacctcggggagttcggcatcgtcgcgcctcaaggtccagctggggtgcgggcagcgctgaagagtctgcgtgaagagggtcaggccctgccggatctggcgcatgccgcgcttggcgggctggcagaacagctcgaacaccttggcgcagagatcagccgtatggagcgtcggattctcgattggcatcggcaggatgagacgagccggcgactggcgaccatcccaggcatcgggccgatcactgccagcgccatggcggccagcgcgccagatccgagtctcttccgttccggtcggcagtttgcagcctggctgggactcacgccgcgggccaatagcagtggcggcaaggaacgccagggcggcatcagcaagatgggtgacagctaccttcgacgtctcctggtcgtcggggccacggcggtcctgcgaatggcccggcagcgaggacgcgagggctgggtcggcaatctcctcgaacgcaagaagccgaaggtcgccgccgtggccttggccaataagacggctcgcatcgcctggaccctgatggcgcgacaggaggactacaagcccacagcggcatagagatcgggccggtcttcacccaggaccggcgccgtagacgaaggagtggtgagacgtgatgacgaaccggccgcagccggggatcggtgaaacccagggggtcagagcgcctcgagcgcgttgacgtgattagggagccggtccgcggacttcatcagggccagcagcgcaaacagctgcatcaacaggccgaacacatgactgcactcgaccgagcgccaacgtcgtttccactcttgcgtcttggaggtcgtccacacatgacgtccctgatgatcttcccccgtaaaagtggacggggttaagccgctttgcgctcggcctcagcggggctgatatagcccagtgctgagtgcaggcgatggggattgtagaagccctcgatgtatccgaacaggtctcgccgcgcctggtctcgggtggcgtagacgcggtgatgaacgcgttcggtcttgagggtgtggaagaagctctccatcggggcattgtcccagcagtcgccctttcggctcatcgacggggtgatgccggatcgggccagggctgatcgataggcttcggctgcgtattggatgccccggtccgaatgatggatcaggccgggcgcggggcgctgacgttcgacggccatgttgagggcgtcgagggcgatctcggtgtgcagggtctggcgcatggaccagcccacgatcttgcgggtgtgcaggtcgaggatggcggcgagatagagccagccttcgccggtcgggatgtaggtgaggtcggcgagccagacctggttgggcgccgccgcctcgaagttccgggccagcctgttgggcgcgatgggataaccgtggcggctgttcgtcgtccgggcgcgacgcggcaaggccgccaagccccgcaggccggcgcggcgcatcagccgctccacgcgggatcgaccgacccgacgcccatgccgccgcagggtggcgtgaacgcgcggcgagccgtaacagccgctgctctccgcatggatcagccggatatcctcggtcagctcgcgattggcgacagaccgctggctctcggggcgaccgcgccaggcgtagtaaccgctggccgacaagcccaggaccgcgcacatcacgcgaaccggccagacctgacgatgctcatcgacgaacccgaacttcatcgggaggccgctccgaagatgagcgcggctttttttaggatgtcccgctccatccgcagctgaccgttctctcgccgcaaccgggccacctccgccgccagatccgacggcgacggggacgacgcctgcgttgtggggcgccgcgacgcccccgtcgcctgcaccccgaactgcgtcatccatcgacgaagcaccgtctcgtgcagcccaagctcgcgggccaccgccccgacgctcaggccgccgttggcgacgcggtcaacggcctcgcgcttgaaagaatccggaaagttccggcgttgaacactcatcagacactcctctccagctccgaaaagctagcatgggtgtccaccaaaccgagggaggatcactgatgacgacacacccagaacagcccgtcaggcggaggtcgtccacaccatcacgtcaaacgtgccgaccatcacatccgaagcttggaccttctccctgttcactacggcaatcctcgaattggccaacgaactgccgaaccgggtgaccattcgccagcttctggccttcgcgatgatccttgaggaagtcagccttggtagaagcacgaccatcaaggggcttcggaccaaggcgggcaatgacaagcgcggcgccgaagtccttggccagtccatcggccgcacctaccaaatctttctggctcccacgagaaaggaaccggacggcctcggctggctctatgtcgaggaaaacgaatccgaccggcgcgagaagttcttgcgcctgaccaaggagggagaggccgtcgcgctcaagctggcgcgcatcctcaaagagaagccgtgaacgtcagcgaccttctccgatactgcgaactgcacgagtggcgtggccatcggtccaaggccacccttcgcaccaacatcaagcagcttagggctctgatcggcgacgaggacatcgcgtcgctgcactacacaaggctcaagcgtctagcctcggacctcgaaaactacggcgggcgaacggcggcgcccgccaccatcaagcgcaagctcgacacgctgtcgaacgccctgaccgtggcgaccaagatgacgaacgacgatggctcgcctgtcctgatcgcgaagccgaccttcccgacgttcgagatcgacaacatccaagagcgcgtgatctccgacgaggaagttgcggctctgttcgaggtcatcgccgcacggcgcgaggccgaaccggcgcgggactggacccggttcgacgcactcatgagattcttgctggccacagcctgtcgccgaggcgaggcgttgcgggtttggcccggccatatcgagcaacgcgatgttgatggcgtcgcccgtcacttcgtgaggttcgaacgctacactaccaaatcgaagaagccgcgcaccctccccctctccacggagatagtcgccctactcccggcgctgcgcctacaggcgggcaatggcccgctgttccccttcactgccagccagctttggggtatgtggaagtcggtgcggcaggacatggcggcgcgcgggttcgatttctcgctcgtgcgctatcacacgactcgccacaccacgctgaccaaggccatgaagcggtttccgctggccaaggtctcgaagctcgcaggacatgcgagcatccagattaccgctgaccgctatggccacctgtcggctgacgatctcgtcggcatggtggacgatctcgcagcctaactaagcctctgcccttacagtcgtaagcaaaacccgttcgtctcgagtgagaccaagtgggggtttacttcctttcgactgttgaacagggaggttcaatctaggtcatcaccgccacgccgcaagcgtgacctttgacattcttcaggcggcttcagcggttgcgccggcgagcccctgcatcaccatgcggttgatgtcgatcagggtcgagaaatcctcagcgccccgcatcacctcggacgaatgcctgttcacgaacaggctcagcgagatgatcgaggcgcgcagcggccgggccatctgattggccggatcgccgcagtcggaagccagcgccgtccacacgcgccggttccagtccagcgcctcgatacgggtcctgaagtcggaaggatcgctggtcgaggcctcgaccagcgcccgcgtcacctggccgaagagacggtactcgacgtcgcgaggcgcttcattgcgcgccgccgctgtcgtgtaggcttggaacgacattcagcaccttttcttcgtaatcaacgatcttacgggcggccatcagagccttgtagtagtcgcggttcagcacatgcttggacaccgcgacgcactcggccaggatttcggggttgcgggatgcgcccatgaactcggtgatccgcagcgccatctcgtcgtacagcttggaggcgtccgtctcgtccaggtacatcatcatgaccgggaagtagatccggcgggccggcgtgttcacgtcctcgacctgcatgatgtccttttcgcgcaggacgctggccttgttctgcaggatcaggacgctgcgacggtccccgttctgcaccacggcgccgttcagcacgaacttctcgccgggtttcagggacagtttcagcggcattgcagcgggctccagaaccaacccgacgccacacataggcggacaggcgctgatcgtggctaaacgatcatggttaaccgtgtgttgtgccgcccggccggaacgccgtgaaccgacagcgcgttgttgcggcgaagaggagcccgcaatgcccgactatgacgaacaggaccaggccgaggtctatgatgagacccatctcgacgatgaaggcgacggcgagttcctgctggacgaggccgacagcgtcctggacgtgacccaggcggacggcgacgccgacgaagaggagttcgacgaggacgacatcgacatcgacggcgaactcgcgctagacggcgtcgaggcggaggcggacgccctgctcggcgtcgacggcgagaagatcaaccagtcggacgccggctcgaacggcctgcaggccgacgacgaggtcgaactggtctacgccggactgatggagaacgagcgcggggcccaggccagcgccgcccattgggaagccaagaccctgtcggacgacgacatcgccgatctgggctacggccccgaaggcgacgccgccgatgaaagcaccgcctgaggagagccggaaatgaccgtcaagaccgacaccagcacccagaatgaaagcgtcgacacgccgcacgcccgccgcatcgatccgaacgagggcggccacgaccacctgaagcgcggcgatgaaagcgaagaccgtcaggaagctctgctggacgaaggcgtggaagaaaccttccccgccagcgatccggtttcggccaagcacatcacctgatcgctgttcaggctttcgccgatccgctaacccgcttcgtgaccatcacggagcgggtttttcatgagccggtttgaaggcgccgagcgatacgtcgcaaccgaagacctgaagatcgccgtcaacgccgccatcgcgctggagcggccgctgctgatcaagggcgagcccggcaccggcaagacggtgctggcctatgagctggcggccgcactggatgcgccgctgatcacctggcacgtcaagtccacgaccaaggcgcacaacggcctctacgactacgacgccgtctcacggctgcgcgacagccagctcggcgatcctcgcgtcgcggacgtgcgcaactatctgaagcccgggaagctgtgggaggcgtttacttcgcgggtgcggcctgtcctgctgatcgacgagatcgacaaggcggacatcgagttccccaacgaccttctgcaggaactcgaccgaatggagttctttgtccaggagacggcggagacgatccgcgccgaagtgcggccgatcgtcatcatcacctccaacaacgaaaaggaactgccggacgcgtttctacgccgctgcttctttcactacatccgctttcccgacgccgagaccatggcggcgatcgtcgagacccacttcccgggcgtcaagtcgcggctggtggccgaggccctgcgcgccttctacgacctgcgtgacacgccaggcctgaagaagaagccctccacctccgagttgctggactggctgaagctgctgctggtggatgacgtggatccggagacgctgcgccagacatccgccgacaagctgatcccgccgctgcacggcgccctgctgaagaacgagcaggacgttcacctgttcgagcggctggcctttctggggcgtcgcggcggcgggtgattaccgcgatttcactggatcggcgccgtcgccggggcacaatggcggtcatgaaccgtcgccttttgctcactcccttgctgctggtcgccggactgctgtccgcctgtgacggcgacggcgtgcggatcacgaccagcacctccgacagcggcgacaagggcgtgctgaaggtggtggacgccctgcaatgccctgaaagcgagggcgtgctgacgcgcaaggggtcggcggcgccgggcggcgacatctgcacctacggcggcgcgcgcggcgcggaggtcaccctgcacctggtgcggctggacggagagacgccggacgccgccttggcggccttcgagcagcgtctgagcgcctccatgccggacgcggcgaaccaggcgagcgcgaacggcgacgcccgcgtccgcatccgcgccaacgatgaggacgcctcagtggacctgcctggtctcaagatccgcgccgaaggcgacgccgccgacatccgcatcggcggcttgcgcatcaacgccagcgacggcggaaacgccggctcctcgacccaggtgtcgaccggcggcgaccaggtggacgttcaggcgtccggcgacatggccgtcgtgcggacctccgaggggggcgacagcacgcgcgccacctttctgctgaccgacgaccaaccgtcccccgaaggttggcgcatggtcggctttcaggcgcgcggaccgaacggcggtccgatcgtggtggcgaccgtgcgctccaaggatcgtcgctcggacgagctgatggacgccgcccggcggctggtgaccctgaacgtcggccgttagcgacggcttcggccccggcgtcttgatcccagggcggctttgcgtcaccagacgcgcccaagatcgatcaggataaaacccgtttggccgagcgtccccgaaagcctgctgaagtccgagcctggcagcgcatgctgtccggccgacgcctggacctgctcgatccctcgcccttcgacatcgaggtcgaggacatcgctcacgggctggcgcgtgtcgcgcgctggaacggccagaccgtcggcgagcacgccttctccgtcgcccagcacagcgtcgtggtcgaggagatcgccgcgcacatcaagccgggtctggagccgaagtggcggctggcggccctgctgcacgacgcctcggaatacgtcatcggcgacatgatctcgcccttcaaggcggcgctgggcgtctcctacaaggagttcgagacgcggctggaggcggcgatccacgtccgctacggcctgccgcccaagaccccggcggcgatcaagaccctgatcaagaaggcggacaaggcctgcgccttcttcgaggcgacgcagctggccggcttcacgcgccaggaggccctgggtttcttcggccgcccgcccgagggctacgacctgaccatcgagcctctgccccccgcccaggcccaggcccgctatttggagcggtatcgggtgctcgcgggcgcggtcggcatcatccccgctcctgacgcctttcacaccgagtgaacgatggctcagccgacgcaagccggagttcggatcggcctgtcggcggtcgtgatggcgctgcgcgatcgccaggcggtggtgttgaccaccccggccgaggacggcggacgcgccctgccctttggcccgttcgatcccgtccgcgatcgcacctttgagcgcgccctgcgcgacttcgtgacggcccagaccggatttcggctcggcttcgtggagcaactctacaccttcggcgacgccgggcgcggcgccccgcgcgccgcccaggggcccgagcgccaacgtgaggtgtctgtcggctatctggcgctgacgcccgacgccgggcgtgaccagcagacgccgcaggcccgctggaacagggttctggacgtcttcccctgggaggacaggcgcgacgcctccgcccgcgtctcatctgtcatagtcgatcggctgcgggaatggagcgacggcgatccacgtcgtggagcgcgagccgacagcctttttgcgctgacgcccggtcaccggtggaatgaggaacgcgttctcgagcgatatgagctgctctatgaggcggggatcgtggaagaagccgcgcgggacgccgggcagccgccgatcccccatgcgcccggcctcaccatggcgtccgaccaccggcgcatcctggcgacggcgctgggtcgcctgcgaggcaagttgaagtaccggcccgtgctgttcgacctgatgccggaggctttcacactgtccgatctgcagactgcggccgaggctgtgtcaggtctggcgctgcacaagcagaacttccgccggggcgtcgagcgcacaggcctggtcgccccgaccggacggatgtcttcagccaccgggggacggccggctgaactgtatcggttccgcggtctcgatccccaggacggatcggcgcctggcctgtcgctgccggcgcagcgctgatccgcttcactttcttcgatcaacccgcttgcggcccgtccccggtccgactacacagcccgctcgctcaaccatgccttcatggaaacggcctcgcggagaggtggcagagtggttgaatgtaccgcactcgaaatgcggcgtgcctttacgggtaccgggggttcgaatccccccctctccgccacttccattaatttctggtgctgaaacagcgccctacggggatgactggctgacctgttgtcgaagccggtcacggtgtcgtcgccctccgtcaaatgacggggtctggcgagtgttagtcggcgttcgccagctaaggccagagcgggcgtatccaaccaagtgctgagcattactgcacgtccggcgtagcaggcgggcctgacggagcgaggttgtccggcttctttcggtcaccggacttcgcaagccggcgcgttgtcctgttcgaaacaaatgttcttgctttgttcttcttgttgcatcatgttctcctcatgtcggcggcgatcaagggacgaggcgcgaaatcgaatgcgacaggccgctacgaagtcggtgtccgagaggcgttcgatgacggctggaccgccgacgatgcggatatccagccgctccgcaccacgctcagtcccgaacacgcccgcacgctcatcagccggaacaccagtccggacatcggtttcgaccgctccatcaacccgtacaaaggttgcgaacatggctggccctattattctgttacatacccatgaccgaggctgtgaaactgaggtcatccgttcgagggcgcggcgcaaaatcgaacgccagcggccgcttcgaagccacccaggtcgaggctttcgacgacgggtggaccgatgaagacgccaccgcttctacccagattccgacgacgataaccccactccgctctcgaaccatcatcagtaagaaccagagccccgacatcggctttgagcgttccatcaacccatacaatggttgctcccatggatgtagttactgctatgcgcgcccgtcccatgcctacttgggcctatccccgggcctggatttcgagagccgcatcttcttcaagcccgacgccgcgcgtctcctggaacaggaactcagcgccaggaaatacgtctgcaagcgcatccacataggcggcaatacagacccctatcagccggacgagcgcgaactgaagatcacgcgtagcgtgctggaggtggcggctcggttcaaccagcctgtcagcgtgataactaaatccagcctgatcacgcgcgacctcgacatcttgggcccgatggggtgcgaccggctggcgacggcatttgtctccatcacgaccctggatcgcggtctggcccgcgcgatggagccccgggcctcgacacccgctagacggttggaagcgatttcccgtctggccgacgccggcgtgcccgtcggtgtcggttttgcccctgtcattcccggactgaacgaccatgagttagagtccgtcttggaagcggccgccaaggccggtgcggtgaccgctatgtacgtcaccttgcgcctgccgctggagatcaaggacctgtttcgcgaatggctggcagacgcccgaccggaccgtgcggcccgggtcatgtcgctggttcgccagacgcgcgggggcaaggactacgacgctgactgggcccagcggatgaagggcgccggccccgtagccgacctgatcggggctcggtttaaggcggccgtcaaacgctatgggctggacggaccccgccacgatctggatacgacgaagttcaccgttccacacgggtcaagaagccagatggacctttttgagtagaccgcgcgagtatgtccgctgctggcggataccgttgaaaaagtcggcaattgccacgggcggcgagtgctgattcactctggtcattgaggctggaggcagcgcgatgatgggcgagcggcgggtcgatcaggcggccctgttctatactttctcgctggaagaccacgtccctgcgaaccatctgctgaggtcgatcgaccggttcgtggagttggaaggtctgagagggcatctggcgccgttctacagcgccatgggtcgcccctcgatcgccgccgggctgatgatccggatgctgctggtcggctattgcttcggcattcgctcggagcgtcggctgtgcgaagaggttcacctgaacctggcctcccgttggttctgccggctaggcctcgaaggtgccgtgccggatcattcgcccttctccaagaaccgccacggccgctttcgcgacagcgatctgctgcgccagttgttcgacacggtgctgcgccgctgcatggctgaaagcctggtcggcggcgaaggctttgccgtggacgccagcctgatcaaggccgaggcgaaccgggaacgcagcgtgcctggcgatccgggccttccgcccgaggcgtcgagccgggccatcgacgagtatctggcggtgctggacgacgcggcgttcggtgcggctactccggtgacgcccaagttcatctcgccggtggatccggcagcgcgctggaccgccgccaacaaggggccggccttcttcgcctatgccaccaactacctgatcgacctgaagcacgccgtcatcgtcgatgtcgaggcgtccaccgccgtgcggccggctgagctgacggcggcccgcaccatgatcgagcgggttcaggataggcatgatctccaccccgaccgccttgccgctgacaccgcctatggctcggccgagatgctggaatggctggtcaacgaccaggggatcgcaccccacatcccgatcatcgacaagtctggccggacggacgggaccttctctcgagccgacttcacctatgatcccaccgccgacctttatcgctgtccgggcggcaaggcgctgaagcagtatcggcgtgccttccgagccgatcatcccgagacgccgccggatgacacctatcgctatcgcgcctccaagatagactgcgacgcctgcgctctgaagccgcgctgctgtcccaacacgcccgcccggaaggtcacgagctcaatccacgaaggtgcgcgggacttcgctcgcgacatcgccaggaccgacgcctacgtcgtttcacggcgcgagcggaagaaggtcgaaatgctgttcgcccacctgaagcgcatcctcaggctggaccgactgcgtcttcgtggtccctgcggcgcccgagacgagttcctcctcgccgccaccgcccagaacctgcgcaaaatggctcgactgatcccgcaaccgaccgctcccacgcccgcctgaaggcctgaagcgtcacgatcccatcacagcctgaccacgcagccgtgctgtcccgtcagccatccgactttttcaacggtatccgccaacagcggtcattggcgaagttgcgagaaccagacatgagcttgggttcgatgaccgagcttaactgcgccgatcccggcacctcattgtgccgcgatggcgatggatgacaaatcggacgcggcgtcgaccggaacgccctccgcctttcgttcggaataccgatcgacgagctggacggcgtggggccggaccagaatggtgaagcgcaccagttcctccatcacgtcgacgatccgctcatagtaggccgagggcttcatccggccggccccgtcgaactcctggaaggccttggccacgctcgactggttggggatggtgatcatccgcatccagcggcccagaaggcgcagggtgttgacggcgttgaagctctgcgacccgcccgacacctgcatgacggcgagggtccggccctgcgtcgggcgcatgccgccctggctcaatggcaggtgatcgatctgcagcttcatcagcccggagacctggccgtgccgttccggactgcaccagaccatgccctccgaccagaaggcgtgttcgcgcaactcgcgcaccgccgggtggtcgtcgtcgccgggcgcgcccggcagggggaggtcggaggggtcgaagatgcgggtctcgcatcccatgcgctgcagtaggcgggccgcttcctcgacgcagagccgcgaatacgaccgctcgcgcagcgatccgtacaagagaaggatccgcggcgccgggtcggtcgagcccaatccccgggcgggctcggcggacagataggccgcgtccagggccggcaggttatccggatccggcagcgaacgcagacgggtgaaggtcattcaaaggtccttggtcaaatagacggcagacgccgggcagaggtccgcgaactcgcgagtttgccggatcgcgggcggcgcggactcacgatcggcggcgacaaagccgcgcccggtgaagaagcgctcggccgtcgtggtgagcaggtgcagacgtgcagcgcccaggtcgccggcggtggtctcggcggcggccagcacccgacttcccaggccgcgggccttctggtcggcaagtacgaccagggagcgcagcagcaggtcgcgccgctccccttccagcccgccgtagccgatgaccgcgccgtagtggtcggcgctgaagtatcgcccggcgcccggctcaggcaggttctcgccacgcagggccgcgatcagatcgacatcggtcgagtcgaccaaatgcagactgaccatcagccggcgtccttcggcggggccgtgtccgggaaccagcgtcggcccatccagagcgcgaccgacacgagcaggatcaacaccggcacctcgacaagggggccgatgacggccgcgaaggcgaccggcgaggtcaggccgaaggccgcgatggccaccgcgatggccagttcgaaattgttcgaggccgcggtgaaggccagggcggtggtgcgcggatagtcggcttcgatcagcttgcccatgaggaagctcaccacgaacatgacgagaaagtagatcgtcaggggaatggcgatgcgcagggcgtccagcggcaaagccaccacctccccgcccttgaggctgaacatgaccacgatggtgaacagcagagcgatcagggtgatcggcccgatgcgcggcaggaagcgccgctcgtaccagtcggcgccgcggcgagcgatcaggctgcgtcgggtcaggaagccggctaggaacggtaggccaaggtagacgagcaccgcgccggcgatggtccagacgctgacgtccaccacgctgccctgcaggccgaacaggggcggcaggacggtgaggaagatccaggcataaaggttgaagaacaggaactggaagatcgagttgaaggctacgaggccggcgacatactggttgtcgccccgcgccagctggttccagaccaggaccatggcgatacagcgcgccagcccgatcaggatgacgccggtcatgtattccggctgatcacgcaggaagatcaccgccagggcgaacatcagcaccgggcccagcacccagttctggaacaaggacagggccaggacccgcttgtcggcgaagacgcgcggcagttcctcgtaccggaccttggccagcggcgggtacatcatcaggatcagaccgatggcgatcgggatattggtcgtgccgattgagaggctgtcgacccaggtcggcaggcccggcgccagcgtccccatagccacgcccaggcccatggccacgaagatccacagcgtcagccagcggtcgaggaaggacaggcgacgcggcgcagcgtcctccacgcgggtgtcgatcatcgcttcacccgctggccggcggcgtcgatgacgacctcgccgtcctccttggtgaagggcttgagatcatcggcgggcaggaggtccagaacggcctcggacggtcggcacaggccgacgccgagcggactgacgacgatcgggcgattgagcaggatcggatgggcctcgatcgcatcgagcaactgatcgtccgtcaggcccgggtcccctaggcccagttcggcgaagggcgtgcccttctcgcgcaacagattgcgcagcggcttgccggcccgttcggccagccaagcgaccatggtccgcgacggcggggtcttcagatactgcacgacatgcggctcgatgccgacgtggcggatcagctcgagcgcgttgcgcgacgtcccgcaggcggggttgtgatagatgacgatgtccacgggatccttaggggcaacagggcgcgagttcagccagcaggggttcgcacaggtccgccctgcccccgcagcagtccttgagcaggaagaggaccaggtcgcgaagccgatccaggtcggcccggtagatgatcgaccggctgcgccgctccgacctgatcaaccccgcgcgcgtcaggacgccgagatgggacgacagggtgttggccgggatcaccagatggttggagatgtcaccggccggcagaccatcgggttcgtgacgcacgaggaggcgaaacgcctccagccgcgtcgattgcgccaaggcggcgagagcgagaatcgaaacttcggtttccatatttccaaattagtcgaaatatggaaatgttcaagcccgctcgtctgcgggtgcggcagttcaggcatcggtgacgacctgatctttgacgactgccgcctaaaagatcgcagagtagcgacagccgagtttaagggtcgctgggctatactctccgtcgagaccatggactttggccacgaggtcgacagttggccgatttcgcacgtctgtcggtccggacgcggtgcgctgatctcgcgatcaggcggcgggagccgccgacgctcccttctgggcgagccaggcgtcgatcagggtgatttcgcgctcctgcgccgtgatcacctcctgggccaggttccgcgcttgggcgtccttgccttgcgcgagctccacacgggccatcgagacggcggcgacgtggtgacctcgcatctgcttcatgagcttgatgtccgcgtccccggtgaaggcgggcatcgcctccatcatcgtgttcatcgaggccttgtagccttgggtggcgacggagtcgccgggcgcaggcgcagccatgccgccctccattccgccatgggcgtccgccgctgcgggggcctcaggcgcggctacggcgggctcttcggcttgcggggaacaggccgtagccaaggcgcaggcggcgaggacgaggctgatgcgtttcatgacggctccttgggatcccgacgttagcgaccaggagggcccattcgttccgccaactctaccgtccggcccgcgccaagagctcgatcagctcgccggcctttgccttgcgatcctcgggatcgtcgccggtcatagcgcccatgacgcagtggtcgaggtgatcccgtagcacttcggtctccacgcgatggagcgcggctcgaacggcctgaagttgggtcagcaagtcgacgcaataccggtcatcttcaaccatgcgggagattccccgcacctggccttcgatccggctgagcctgttgaggactttgggtttcgtgtcggtttgcatggggcctgttctcctgagcacccccatataccccagacgggtatcttgcgatataccccgcatgggtatatgttagctcttcggtcagccggagagagcgacatgtccacgcatcctcacaatcatgcctcgggtcacgcctgctacggggcgaaggcctcggatggcgcggcaacggtcaaggatcccgtctgcggcatgtcggtcgatccgacggccaccgctcaccgagccagtcatgacggtcaggactatttcttctgctcggcggggtgccggaccaaattcatcggcgatccgatgcgttacctgaaccctcccgtggaggccgagccggccgttcccggcgccatctacacctgcccgatgcaccccgagatccggcaggaaggcccaggctcctgcccgatctgcggcatggcgcttgagccggagacggtcacggcggaggccccgcccaaccacgagctgatcgacttcaccagacgcttctgggtcggtctggtcctgaccctgccggtcttcgccctggaaatgggcggacacctggccaatctccacatgttcatcccgggccagatgtcgaactggatccaattcgctttggcgacccccgtagttctctggtgcggctggcccttcttcgagcgcggctggacatcgctgcgcacccggcggctgaatatgttcaccctgatcgccatgggggtcggcgtggcatggctttacagcgtcgtggccgtcgtcgcgccaaccctgttcccgcccgccttcctgaaggccgacggcagtgcgccggtgtatttcgaggcggcggcggtcatcaccgtgctggtcctcgttgggcagattctggaactgcgcgcccgcgaacagacgtcgggcgcgatccgcgccctgctggacctcacgcccaagaccgcgcgccgaatccgggcggacggcatcgatgaagatgtctcgcttgaccagatcgccgtcagcgaccgcctgcgggtaaggcccggagagaagatcccggtcgatggcgaactcctggagggtcgggtcgctgtcgacgaatccatggtgaccggcgagtccatgccggtgaccaaggatgtcggcgaccgcgtcgtggccggcgcgctcaacaagaccggatccttcatcatgcgcgccgacaaggtgggcgccgacaccctgctggcgcagatcgtccagatggtggcccaggcccagcgcagtcgcgccccgatccagcggctggccgatacggtctccggatggttcgttcccacggtgatcgcgatcgccctgctcgccgccgtcgtctggggcctggtcggtcccgagccccgtttgtcctacgccctggtcgccgccgtttcggtgctcatcatcgcctgtccctgtgcgttgggtctggcgacgccgatctcgatcatggtcggggtgggacgtggcgcccacgccggcgtcctgatcaagaacgccgaggcgctcgaacgcttcgagaaggtcgacactctcgttctggacaagaccggcaccctgacggagggccgtccgtcggtgacggcgatcctgcccgccctcggcttcgtggaaacggacatcctgcgtctttcggccagcctcgagcggggcagcgaacatccgttggccgacgcaatcgtccgggcagccaaggaccgggacatcccccttaccgaggccgcggacttcgacagcccggtcggtcgcggcgttcgcgggacgattgagggccgccaggtcgccctgggcaacacccgttttctcggcgagctttcgatcgacgtcgccgcgctggagccgaaggcggaggcccttcgccacgacggcgccaccgccatattcgtggcgatcgacggaaaggcggccggggtcatcggcatcgccgatcccatcaaggccaccacgccggctgcgatcctcgcgctgaaagcggccggcctgcggctggtgatgatgaccggggacaaccggacgacggccgaagcggtcgcgcggcgcctcggcatcgacgaagtccaggcggaggttttgccgcaggataaggcgtctgtggttcaacagcttcgttcgcagggtcggatcgtcgccatggcgggggatggcgtcaacgatgcccctgccctcgccgcagccgatgtcggcgtcgccatgggggcgggttcggacgtcgccatcgaaagcgccggcgtcaccctgctgggcggagatctgcaaggcatcgtgcgcgcacggcgtctgtcccgcgcggtgatgggcaacatccgccaaaacctcgttttcgccttcggctacaacgcccttggcatccccgtggcggctggcctgctttatcccgtcttcggctggcttctctcgcctgcccttgcggcgctcgcaatggcgctctcctcggtcagcgtcatcggcaatgcgctgagactgcgcgcggtgaggctttagccaggataggcaatcaacagtccgcccacccacccaagggaggaaccggctgtgacgggccggattgattcagacgctgaccgcagtctccaggctttcgcagcggcaggcgaagacgaactgaaatttctgaagaggatacggacgatgtctcatcaacagatggaccacggcgggcaaggcaacgctcgtggactcggcccttatcggagcctgtacctcgagttggcgctcgatttcgtcatcatgtacctggtcatgtacacgatgatcgccacgctcggtcacttctatctcaatttgaacaacgtctacatgaccctgatgatggtcgcgccgatggcggtcctcatgctcgtcttcatgcggtccatgtacccgtcgcgcaaaacgaacctggtcattggagcggtcgccgtcgtgatcttcgtcggcagcttcgtcggcatgcgcacccaggcgttcgttggcgacgacgaattcctgcgatcgatgatcccgcaccattccggggctgtgttgatgtgcgagcaagcctccctgaccgatccggagatcatcgccctgtgcgacggcatcgtgcgtggtcaacaggaggagatcgcccagatgcaggcgctcctcgagaagcgtcgccgctgaccccggcgtgcgggggaaggcctcagccgccccccgcttcctcttcatgagggacgcggtcgtgtggcgcgtagagaagcagaaggccgggaccggccaaacgtctggagactgagtatgcgttacttcaaccccgcacccttcatcgccgtcgcggcggtcgtggccttcgccgccggaccggcggcggcccacgctcgcctggtcagcgccaccccggcgcccgactccaccgtggccgcgacccggacgctgaccctgaccttcagcgaacgcagcgttcccgccttttccggcttcgacgtcgtcaatgcggcggaggagaagatcgcgatccgcacctcggtcgccgaggacggcaggaccctcacgggcgcgctggctcgcccgctggccgccggcgcctaccgtgtcgactggcgtatcgcctcgagcgacggccaccgcatgacgggatcctacaccttcacggtgcgctgacgccgtgctggaagtcgcggtcatcgcgcttcgttggcttcaatacggcggcggcgtcgtccttctcggcgcgccgctgttccttctctacagctttaaatacgccgacgcgccgaacctggaatggtcgcgaccgacattgcgcctcgcggcgatcatcgtcgcgctcggctcgctcgccgccctggtggcccagactgccgtcatggcggggtcgctgagcgaagccgtgaaacccgcgtctctgtcctttatggtcaccggcacagccctgggcatggcgatggtcgtgcgggccgccgccgccttgcttgggcttgtcgccttggtcgccctgaaacccggtcgcgcgctctggagcgtgacggccgccttgggtctgatcgtggccgccagcttcgcatggacgggtcacggcgcggccaccgagggtccgggcgggcccatccatcttgtcgccaacatcattcacgcggtggcagcggccttgtggctgggcgccctggcggcgttgacggccctgcttctgcgccgagccggtccggacgactttgcaatccatcgcgccctgcatggcttcgccggccttggaacgctcgcggtcctgttgctggtgctgaccggtctcgtgaacagctggttcctgatcggtcccgagcgcgtggcgtcgatcgcgggcaacctctacggccagcttctggtcgccaagctcgtcctcttcggtttgatgcttgcgctggcggcgagcaaccggttccggctgacgccgacactgggctatgcgctggagacgggccaaccctccctcgccgccatgagcgcgctccggcgcagcctgttggtcgaaacgggtctgggactcgccctgatcggcgtcgtggcggtcatgggaaccctaccgcccccggcgtctctgtagccgcgatcgcgatgatctgaatgaggtcgtcgctccgccggccattgaagtatgatcagacgatgccgttcctgcgtcatgacctcgtccgactgacgaccgcgctgctagcggcgtttgccgtgctgttcgtgtccaccgcttcgatcgcctgcgaagctccggtcgatcaggatatggcgtccatgtcgatgagcggcgacggcgtcccttgcgagccgaagaccgtcaggatctcgtgccataaggcgtgtctggccatctgccagggcctggtccctcagggcggtgaacccacccccgcacgggtctatgcgtctgtcctctatccatcccttgatgcgcggcatgccgatttcaccgcggaggcggacgacccgcccccgcgacgctgatcctgttgaagaagaccgaactcattcaatcaaacagagatcaaaaccatgaaacgcacgctcaccctcgcagccctggtgctgctggcttccggttcagccgccttcgcggccgcgccgcacgccgtggcgcaggccgtatgcgcttgctgcgacgctatcgcagcctgcgcggaagcctgcacctgctgctgatcgtatgatcggggacgcccgcccgcgagggcgggcgtcttctcgatgttcctcaccgacgtcgcagggccggcgacccgctggcgcgggcctgagcgtcagccgggcgcgcgcgacgaccagtgaatgtggtggatgcgccagccgtcggcatggcgtttgaggaccatggtttcggtcgtcaggcggtctacggcgcggccgttgaattggcccgtggtgcggccttcgctggtgatccaggcgatgtccccgtcggcccatcccgatctgcgcgtcaccgtcgcttcagaggcggcggcgaaggcggcgtccgagcccaggtgatgggacgcatactcgtcgcgcgatcgctccgcgccaccctcctcgaagatcatcacatccggcgccatcagggccagggcgacggccgtgtcgccggccttcagggcgacgtgaaaggcgtcgacggccgccgccgcgtccgcagcttccgcggcgaccgagccggcggcttgggcatgcacgtgggcgtggtcctgggcgaaggcgggtgtcgccgaaagcacggcgagcgacaggacgagggcgagagaggtgcgggacatggcgaactccggattgtgggtgatctgaacgggctgagcgcgatctgcgtcaggccggcgggttgtggcgggcgaacacgcgggtcgcgcccgagcgaagcaccagcagagtgtcgtagggctccttgcgcccctgcggcgtctccatgccgggcgaaccgagcggcatgcccgggaccgcgacgcccaccgccgccggtcgctcggtcagcagtcgaatgacgtccggggccggcacatgaccctcgaccagatagccatcgatcagaccggtatgacaggaggcgagcgcgtccggcatgccccggctgctccggaccgattgaaggcttggaaggacggtgatggtggtggtgaagcccgcctggcgcatgtgcgcgatccaggcgtcgcagcaggcgcaggtgggcgtcttgaagaccgtgaggtttctggacggacgggtctgggcgcaggcggacccgcccatgccgatgaagacggccgcgcccatgagtagacgacggttcagattggcgggattcaaaagggttctccctgatcgctgtggacggatcgctgcgcctcgacagggtcggcgcgctgcggcgccagccgcgcccgcaaccaccgtcggccaggctgctcgacgaagacatggatggcggccgcggcggcgagcgtcaacacaagcatggcggccagttcgaccaggcccattcgatagtccgcaccccagccggagaacgcctgcgccgcattgcgccacaccatcaggatggggatgtggacgagatagagggcgaacgacgcttcgccggcgaacagaaggacggggtgagacaggaaggtccggaccggagccttggccaacagggcgagcgacaggatgaagggaccggccgccgccacgatgacccggtcgtcggcgcccatctgcatgagcgtcagcagcagggtcgtggcgaccagggcgcccatgagggacattcgcggcgaaggcgtccagcgctgaccgagatagtagaggccaatgccgtagaggaattcgggaatgatgcgcaggatcccgaggctgtcctcggcgcgaggcagcatccggccgaaccaggcgcggtagaaagcgtccaaagcgacgaaaaacagcatggcgagtgcaatcaggacccacggcctggcccgcagccggagcgcgagggcggcataggcggggaaggccagataggcgaaccactccgccgacagcgaccaggccggtccgttccagagcgccatgctctcgcgcgggaaccacgcctgtacgagcagaagggtgcccgcgaagtcgacgggattaaaccggccaggctccagcccgacgccgaacacaggcgcgatcagcaccagcccaagcatggccaggaggatgaacaggtgagccggatagatccgggccaggcgcgccgccaggagtcgaccgtagttcggggcccggtctccctgcaggtagacgtgggtcaggatgaagcccgacaggatgaagaagacatccacgcccaggcgcgcgcggttcaacaagcccgcgctctccgccgggagggtccagtagagctggaagtggaacagcacgacgccgagggcgagaaagaacctcacgcccgtgagcggatcgagcacgtcggggaatggaacccgcctgggccctgctctgtcgctcacgtcttttccccggacgacagggcgcgtcccggtcgtctctggtatctacgcgggcgacggctcgtcccctcgtgaggggaccggaaggccggcgcgtatggcaagtggggcgtgacgcgggtgcgcaatgactgacgacatgaatgagttgatcgcagcggtcgggccgggcgacgccggccggctggtcggcatggaagacgcggtctgggtgcggatcggcgaacgcagggagcgcgcccgcatgggtcaggtccgggtcgcggccgttgcactcgcgctggtgatcggcgttgcgaacggagggctgatgctcatggctccgcggccggagccgtccgagatgcggattttcaccgtctcggcgggcttgtcgcctctctccggcctggacgttcggggatgagggccgcctggaagtcgatcgttatcacggccatcctggccgcgctggccagcggcgcggcgacctgggcgagcgcgacatgggtcatgcgggagcggcagccgccaagcctgcacagcgtcgtccatgagaaactcgacctgagccctgagcaggatcgacggctcgacgtggtcgaagcccggttcgccgctcagcggccagcgctcgaagcggaagtccgcgcggccaatcgcgaactggcggccgccatcgccgccagtgacggcgacacgccccaggtccaggccgcggtcgatcatttccatgccgccatgggcgatctgcagaaggcgacgatcacccatgtgttcgagatgcgatccgtcctgaccccggcgcaggccgaggtgttcgacgccgcggtcgtcgaggccctgcacgacgacgccggctaagcggcgcgcgtgggtgccgagcagagcatcgaggcccgtgcggcgaccggagaccgggccgccttcaccgccttgatggtcgccacaaaggccgatctctaccggttcgtgcgccgctatgtcggcgacgagtccgaagcgcatgacgtgcttcaggaaagctatgcgtccgcttggctcgccctgcggcggtatgatccggcgcggccgttcgacgtctggctgcgctccatcgccctcaacaaatgtcgagactggggccggcggcgcgcggtgcgcagggtcgtgcgcggcgtcatgggcctggaggcgcccgaggcggcggcggtgggcgacgatgcgccctcacccgagacccggctggacgatcagcgcagggccgaagctctgcaacgcgccttgcgggaccttcccgacgccctgaaggggccgcttctgctcgccacgctcgagggacggtctcacgccgagatcgcctcgatcctcggcattacgcccaaggcggtcgagacccgcgtcgcccgcgcccgcaagaccttgacggcggctctgggccaggcatccggcggagacgcttgaccttgccatgatgggaaggtgcgcaagctgcgaacccgacgtttgtggcgtcctgacgcaaggggtacgccgcccggctgcgtatctgaacgaacggccgaatagcccgaccaaggaatttctcgcctatgtccacgccccgcctcgatcgccgaacgcttctccgtggcgcagccgccggcggcgggctgctgggcctgcagggtttgctccccgcctgggcgcaaacaggatcggcgggactgcgggcggatcttccgacgctgacgggaccgaacatcgacctgaccgtcggacacacgcccttcaccgtgggcggccgcaccggccatgcggtgaccatcaacggcgttctgccggcgccgctgctccgcctgcgggagggccagaacgtccggctgtcggtggccaacaccctggacgaggacacttcgatccactggcacggcttgctggtgccgttccagatggacggcgtgcccggcatcagcttccctggcatcaaggcgcgtgaaaccttcgtctacgagttcccgctccggcagtcggggacgttctggtaccacagccactccaacctccaggaggcgatgggccactatggaccgatcgtcatcgatccggcgggcgccgatccggtgggctacgaccgcgagcatgtgctggtcctgtcggactggagtttcatgcatccgcacgaaatcctcgacaagctgaagaaaagccccggctacttcaaccagcagcgcaccacgctcgcgggcctgctcgacggcagcgaccgcatgagcctcgaggagcgccgcatgtggggccagatgcggatggacccgcgcgacatcctcgacgtcaacggctcgacctacacctacctcatcaatggccacggaccgcaggagaattggaccggcctgttccggcccggcgagcgagtccggctgcggatcatcaacgcctcggccatgtcgatcttcaacattcgcatccccggcctgccgatgacggtggtccaagccgacggcgagaacgtgcgcccggtcgagaccgacgagttccagatttcagtcgccgagacctacgacgtcatcgtccagccgaccgaggaccgcgcctacaccatcgtctccgaagccatcgaccggtccggcatgggccgggcaaccctggcgccgcgcctgggcatgaccgccgaggtccctcccctgcgcgaggtcccgaacctcaccatgcgcgacatgggcatgggcggaatggatcacggcgcgatgggcgacatgtccggtatggaccatgacgcgatgtccggcatggaccacgccgctccgacccagaacgcgcccgcagccggcgagatggccgggatgtccatgtcgggcatgaacatgcgcgatcccgagaacgctccgcccgacatggcggtgggcgtcggcgtcgatgggatcgccatggaccccgccaaccgtctgggtgagcgtccgatcggtctcacgaccgtcgatcatcgcgtcctcgtctacaccgacctggtgtcgctccagccgaacaaggacccgcgccccccgtctcggacgatggagatccacctgaccggcaacatggagcggttcatgtggggcttcgacggccgaaagttcagcgaactggtcgaaccgatccgcttcgagcgcaacgagcgggtgcgggtgaccctggtcaacgacaccatgatggcccacccgatccatctgcatggtcatttctttgaactggtgaccggcggaccggccgggcaccagcccctcaagcacacggtcaacgtcgcgcccggcggcaaggtgaccttcgatctgaccgccgacgcgcccggtgattgggccttccactgccacatgctgatgcacatgcacgccggcatgttcaatgttgtgacggtgcggcccatggacggagctgcgtcatgaaccgcctcgccgtcgccctcgccccgctggtgctcgccgccagcgccttcagcgcccaggcccaggaccctcacgcgggccacacgatgccggcgaccgcggcgccgacgcgccccgcgccagcaccgcggcccccgccacaggcgccggcccgaccggcgcaggatccgcacgccggtcacgtcatgccgcccgcgcagacgccgcccgccgcggatccgcatgcaggccaccagatgccggcgcagcccgcgcccgtagacccgcacgcgggacaccagatgccggcggcgacgcccggccaggctgatccgcacgcgggccacgacatgtcggccatgtcgcccgcgcagaccgaccctcacgccgggcatgacatgtcgaccatgagcatggggccgcccgatgtggcgaccagctccgacaatcccggccgtcctccggaggacccgctcccggccgccgccctggccggccctgcccacgccgccgatctcgtcttcggcgccgaggccatggccgcctctcgccggaccctgattcacgaaaacggcgacgtccgcaccacggccgtcattctcgatcgcctcgaagccggcttcggcgacgacggcgagacctacctctgggacgtccagggctggacgggcggcgacatcaatcgcttctggtggaagtccgagggcgaaggcgacttcggcggcgagctcgaggaggctgaagtccaggcgctctacagccgcgcggtcacgcccttctgggacgttcaggccggcgtgcgtcaggacttccggcccgacggcgaggacaccacgcatctggtcctcggcctgcagggcctggcgccccattggtgggaagtcgacgccgccgccttcctgccgcccgacggcgacctgcccgcccgcgtcgaggccgaatacgaccagcgcatcccccagcgcctgatccttcagccccgcctcgaaatcgacgcttcagccagcgacattccggaactggagatcggttcgggcctgtcctcgatcgaggcgggcctgcgactgcgctacgaattccgcaaggagttcgccccctatgtcggcatcgagtggagccgcgcgttcggcgataccgccgattacatcgaggcccgaggcggcgagaccgacgacacccgcttcgtcgtcggcctcaaggcctggttctaaccgaaggagaccaccccatgatgatccgcactctcgttgtcaccgccgccctcgcgttcgccggcaccgccgccgcccaggacccgcatgcgggtcacgctatgccggcccaggccgcagcgccccaatccggcatcacgaccgttcctgcgaatggcgcgatgacccagggttcgcccgagcggttcagcgtcaccttcccccacgccatggtcctcaagaccgtcgccctctccgccgaggggcaggctccggtcgacgtcactgtccccgccgcgccggccgccgccaccgtcggcgtggctcttccgcgcctcgcgccgggcaactacacggccgcctggaccgccgaaggcccggacggccacaagatgtccggctccgtcagcttcatggttcactaggagaacgacgatgagggtttccaacctgctggccgccgccggcgcgatcctgaccctgagcgcgggcgcggctctggcggccgaaggctgcgattgttgcaaggacatggctgcggacgcggctatgacgtgctgcgacgagatgcaggatgatgcgtcttcggctcccgctcattcactggcacctgacagcgcgcctgcgaggccttcgtcagaggccgtgaaccacaatcagcagcgttcaccaacctaagcgacacttctacgatttcggcaggaactctccgcccaaccgccgacgaccatcggtcgagcgcgctaaggtcgaggctgcaatgccccagaacaaactttggctcacaccggaaagcggacgctcccggagtcgccaaagagtcagttccggtcatcggtcgtctaatccgctagcacttcgcggcgtcgggactacaggtaccctccccccgcgcgccacgcggccacggcgccattgagcggcgcgttggtgtcgcggatcatcatctgatcaggcagcgtgccgaccgcgaaggccgtgtgttcgttgagccagacgtcaacgtggccttcaacatagcctgggtactggtccgccagaccgcggatggcgtggtcgctaccgatgagagccaagccaagggcaaaccgcaggtcggacccgtcgctattcccttccagatgacatttcattgttccgggcagatcggccacgtgatgcgaatacagcgtgatacccggcgtcaggtccacccagccttggcccgggattttgaccgtcagcgttgactgcatgatcagtgcgatgtcgcccggacccggacgcaggaccgggccgctacggaagcagtgcgcgtgttgaaaaacgtagtcaggcaccatgtctattcatcttccgtggggtcgccgaactgtccgatgacgacgacgaaggcttccggagcgccaatgcggatcggcggcaacggcaggtgcatcgacgggatgggctcggcgaacgcgaggcgtttccactcttcgtcggagcgttcgatgtggttccagacatggcccgagcgcttcgggccgcacgagatgctccgaatttcgccagccctgtcgaggtagcggagtacattcaggacgcgtcgcgcgtgtgatccggccgggctatagtcgggctcccagtccgacgcgtagccctccgccttgacgatggcatcgatgatggaacggcgggtcaggggaacgtccgtgtcgtccaacatccgcgccaccaagggcaagtcggcgtaagtctgggcgtcaagtcggtcatcttccggaatgtaatcagtataatagcggaaccgcacagtcgcggggtcctgcactgttcccggatgtgaagaatgcaggatgacaccagcgtcgtccgccaggtcgaccagggccgagagcgggccttcgacggtgacgcgcacgggtccctggccgcgcttgtcgatgcgctccagctcgatgggggtcagggtgacgcgctcgatcaggccgcgcagggtgtcgcgggcgcggccggcttcgcggtcgtcgccggcgagggcggagcgcaggtcgtcgagcatggcgtccaggcgggcgatcacggcctcggcctccaggggcgcgggggcgggacgcggcttgaccttgatctggcgctcgaagcgctggcgctcggcctccagccggtccagctccttcatcatcagctcgcccgccaggccctggacgcggccgtcgcggaccgtgtccatgatattggcgatctggcgctccacctcctttagatgggtggccccggcctcggtgcgggcggccagttcggcgttggcgcgctcgatctcggcgcgatactcggcgaggtagggttcaatcagttcgggcttcagcagccgacccttgaggccccacagcaccaggtcctccaggtcctcgcgggccacgcggcggcggttgtcgcaggtcccctcgcgggccgagccgatgcagctcagcttgtcggagacgaccgcataggccttgccgcagacgccgcagcggatgagacccgagagcagatagtcggggcgacgccgtccccggaaacttgagggggccacgcggcgggcctcgatccgatcctggacggcctggaacaggtcgtcctcgacgatgcgcaggtggggcacggggatgaccaggcgttcgccctggggggtgaccttggccttggaggtgcccttgtggcggttgtgcttggtgacggtgcggccccattcgttgacgccgacatagagcctgttgcgcaggattccggtgccgacgtcgcggttgccgtagatggcgccgggcagccaaggtccgcctcggggaccgggcacgccctcggcgttgagggccttggcgatctccaggggggtcatgccggcgacgtagtcggtcatgatgcggcggacgacggcggcctggacgggatcgggctcgcgctggccgttcttgccgttcagcgccaggaccatgcgatagccgtaggcgggctgcccggagatgcggccgtccttgacggtgccctcctggcctcggcgggtcttctcggcctgccccttcacatagcgggcgttctgggcggccttgaaggcgacctccatgtcgctgaccacgccggaggagacggtgcagacgacgatgtccagggcctccatctcctccagcatcccgtgggtgcccgaggcgctgcggctgaggcggtccaggtcctcgacgaggatgacggtgaactctccccggtcggcggcggccagcatggcgaacaggccggagcgcccgatcaccgtggtgccgctgcgctcggcgtcgtgataggcgccggcctcgacccagccctggcgctcggcgtaggcgcggcagagggtcaactggtcctcgatcgacttgaacgtctggtggccggtcgaatagcgggcgtagacggcgtagcgggtgcccgacggcggcagggcgctcaagacccggcctcctcgaccccgtcgtcatcgaagatgctgtcagggaagacctcgatgacgatgtccatctcctccatggcctccatcgcctccatcgcctccagcaacgcctgggcgcccaaggcaccgtgggcgtgccggtccaggtcctcgaccccgccatcctgctcggcacaggcccggcaccggggctgccggtcggtggagtagcgggcgtagagggcgacgcgtgcgcggggcggcggcggggcgctcacgacttgaccttccggcgcttcgcctcagcgtggccgtaacgcgccctgagcgaacgctcctggcggagagactcggtcatgacgctcctgaacgccacgtccagatcggtgacgacgccgccgacgacggtgtggacggcgacgcccagggtcttcagctccgccagcagacgaaggacctgcgaggcgtcgcggctcaggcgggacacgtcctcgaccagcacgacgtcgaaggcgccacgtccggcctccgcgatcatcgcatcgaggctcgggcgggaccccgtcatgccgctgacggcgttgtccttgtagaccgtgaccgtctcccagccccgctcggccgcataggcctcgcaggcgttccactggtcggcgagcggatagggcgtcgcccgggaggcgctggcgcagcgcagatagatcgcgcagcggtgagccgggctgggggccggaacgggggcggcggcgggaacatcttcttgcggcccgtcatcttgcgggacggcggcgatggtgacgacgcggccggcgccggcgtcggcgacgatgacctcgaactccccgtcgccgaggcgatcgaccaggccgttcaatcgggctcccgccagcccgacaccggggcgatcctcgtcgatcatggtcacgacccgcagaccggcgcgctcggcgtgccgggcgcaggtcgtcagggtcgatcctccggccatgtagagcgcggcccgcgccggggccgtcactggacgcctcccaggacctcggcgcgggccgtaatccgcgccagcgacagcatcaggggcagcagttcggccgtctcatcatcgaggccgttgctcaggcggtgttcggcctgggcctggcgctgatggctgagcaggcagccgaacgaggcgtcgccgtggatcggccggggttgaaaggccgatgcgccgtccggttcgaacggcgcatcatggatgggatcggcatagaacatcaggcggctccttcattgtgagtggagcgcctattaggtctacggtctattgtgagtcaaggtctttatgaggtggactcgggcggcggcaggtcgttgacggccgcgtggagcgccagaagggtgggcaggccgacctcgatggtgatcagacagtcggtctgcgcggatgcgtcaccggccttggaaggttccgaccaggccacggcgggggcgtaatgttcgtggaaggcctcgacctcctccagccgcttccaggggcggcccagatgaatctccgccgcgaggccgggcacatagctgacgacgcgcagggcgcgggcgtaaccggggcggaacgaaccgccggcggcggccgacttgaccaccatccactgcatcgagaactccgcctcggatacgccgctcgtcggttgttcccagtccgtcatataggcctcgtgccactcggcgatcgccggagcgttggcgatcagccgttcgacggcgtcggcgaacccgaccttctcgcgcaggaaatccatccaggccggcatgtcctcgcgctgcatgtcccggttcgaatcgtcggggtgcggaaccagggatcgcaggttatggacggcggcgacggtgccttggggactgctgtcgccacaggtcgccagcagcagggtcgcggcgtccttgacggtcatgatcgccgcgccgacgccccgcttcgaggaccggatcaatccctcgtcgcgcacctgccgggcgatatgagcgatggtcgcctggccccgacggtcatgccgagcgatggcttcgatgagagcgggaaggcgcgccaaacgtgatgtctcctgacgtggaactatctccccttagcgcattgtgctctcaactccaaaagagcctttgcgtgccggtcttatcatccacggcttgaatcgcgaccgccacacgcatccggccgatgaggatagtgtcctcgacatcgaggtgggaacggcattcgtagtcagtttcccttgcgatgacgccggatgtaagtggccaaccagcccgcgttcgcgggggccggtccggtccaaggttgctcgtctaccggatagtttgagagggtcgtttccactcgctccgccaaggccggagcgtccaaatctggaaacaccgcttgcgtgaacgccagtccatcgaagcgcatgatgaccttcccattgttgtcgaacaggcaggctaagacacctcccggcaggaacaggccgatctgacgtccatcgccgggatcgacgctgcacacgaccttgcagcccagtccgacgatcgcattgtggacgcgcagccgcgccgcctggcgggtcgccggatcggggtcgtcaagagcgtcgcgaacgtcccggacccgctccaggtgctcggccgggctcacagctcccttcgccgcttccagcgccttggcggcgtcgtcacgttgcgccatcagattgcggagggatcgttcggcatcgaccagcttcgcttcgatcgcctccgaggcgccaatccggccaagggcctcgacccaccgatcgacctgctccttctggttggagatcgccttctcaaggtcggcgagaaccgccgccgaggaagcggtctggtccggctcggcgaagtagcgatcatcgagcgcgaggtggaggatttcatccaacgcggcgcgctcgaatgggtcgtaacggaacatggccttctgcgagcatccgcgccggcgcgccgcgaagttgcactgccaatagcggttggcattaggctgtccgctggaccgaagatgcatccggttgccgcaggactcgcacacgacaacgccggcgaacaaattggcgacgcttcgggtgtggcgcccccctttccgggggccggtctttcgcgattccacctgagcccgagctcgcgccacaaggtccgcatcgacgatccgggggtagtagccgacgatgcgttggtcgaacttggtccgcttggcgctagtgttggagaagccaggcacatagtcgccttcgaccgaaggctggctgaggatcagcttgaccgagccgatttcccacgtcggagtcgactctggcttgcgccatttgccccacgcggggatgccccgctcattcagctccttcgcgatccaacgcgcacccttgccctgggccgccatctcatagacgtcgcggaccatctgcgcgcgatcctcgataatctcgaaaccgctccggtcggccttggcgatcaaccaaccgggcgcctttgcggtgatgatctgccccgtggtccgagcccgttccatgttgcggcctatgcggtcgagcacacgttccgacttctgctggctctcgtcgttcgccagcttggctcgcatcagaatttcgaacacgcccatgaggtcggcgcgaagccccgcatcgtcaaagaccttgccgccatcgacagtggcgatggtcagccccgccgcgcacaggtcctccatccagcggagggtcgtccgggtctcctgacgagacagccgatccagcttctcgacaaccaggaccgttccagctccgacgccgccgtcacgcacgcggttggcaaagaggccgagttctccggccgacaggtgcgcccctgtccatgccgaccgtcccaagtcctcaatcacctcatcgacaggccatccccgctgctcacagaattgttggcagagctccagttgccggtcgcgactggctcccctctcctggttgggcgtcgaaaagcgtatgtagataacagcacgcatgggcggagtttaagctgtgtgcccctgtgcgtgcaataggatcgtagggctgcatctactgctacgcccgtccgtcccatgcctggatgggcctatccccgggcctggatttcgagagccggatcttcttcaagccccacgccgcacgtctcctggaacaggagctgctcgccccgcgataccggtgcaaacgcatccacataggtggaaacaccgacccatatcagcccgtggagcgcgagacccggtcgacgcgcggcgtgctggaggtgctgcagcggttcaatcatccgttcagcatcatcaccaagtccgtgctgatcgcgcgcgacgtcgacatcctggggcccatggggcgcgacaagcttgcgtccgcctttgtgtcgatcaccaccctggaccggggtctcgcccgcgccatggagccccgcgcctccacgcccgccaaacggctggaggccatctctcgcctggcggatgcgggcgtaccggtgggcgtgggcttcgctcccgtcatccccggcctcaacgaccatgagttggaggccgtgctggaggccgcagccaaggccggggccgtcaccgccatgtatgtgacgctgcgcctgccgctggagatcaaggacctgttccgcgagtggctggcgaacgcccggcccgatcgcgccgcccgcgtcatgtcgctgatccgccagacgcgcggcggcaaggactatgacgccgactggtctcagcgcatgaagggtacgggtccggtcgccgaactgatcgccgcccgcttcaaggcggcggtgaagcgctatggactggacgccccgcgccaccagctggacgaaacccgcttccgcgtgcccgccagcgcccgctcccagctggacctgttcgacgttccctagtcgcgggccgcatccgggtcgatggcgttcgtcaccaggtcacgccaggtcggatcgccggcgtccaccagatcgacatcctccatcagggccacggctgcgccgccgtcgggcaggatcaggcccagcacctccatcgattcaccttcggcgttcaggtgcgtctcggcctgcacgatgaccgccgcctgctcgccgtcctcgtcccaccagatcaccggctgcggcatctccatggacagcggacgcggatcgtcggtgtcgcccagcgcgaagaccgcccgtttcgcctgcacgtcgtccagggtcgcgaccgcccccgcaaacggcgtcagccgcgtccagtcctccgcgtcgaagccgccgccgtcctcgtcgaagctctcgtccatcgtctcgccctatcgccggaacacgccgaccagctccacatgcgccgaccacaggaactggtccaccggcgtcacccgctccagccggaatccggcgtcgatcagcacccgcgcgtctcgagcgaacgtctgcggattgcatgacacgccgaccaccacctgcgccttggtcgaggcgatctgcgcggtctgctcgatcgcgccggcacgcggcggatcgaacaccaccgcatcgcatcccttcaggtcgaacggcgtcatcggccggcggaacaggtcgcgcgcctcggccacgatggccttcatgcccctggcggtcttcaccccggccttcagcgccgcaatgcccgcctccgacgcatcggccgcgatcaccggcgccacggtcgccagcggaaaggtgaaggtcccggccccgcagaacaggtccgcgatcttcttcgccccccgcacagccgccacagcccgcgcgaccatagccgcttccgcctccggtacggcttgcagaaagccgccggccggtagggccacggtggcaggcccgaacatcccctgcggcgcacgcgccatcatcagcgtctcgcccgcgaggctgaggcgcgccagatccgcccgccccgccgccgccaccgcacgcgtgcgggcgtccgccgacaacccgccggagcgccgctccacgccggtcacatcgacgtccagccccgtcagcgtccaggtgacgtgcagcgtcggcgcagacttcgggtgctccagaaacgcgtccgccacctccgccagcgccggaaacgcccgcaccagtcggggatcggcgatcgggcattcacgcacctcgaccagcctccatgaccgccgcgccttgaagcccagcacgacctcgccatcgactccgcgccgcgcatgcagcgccagccgtcgccgcgtgccgggcggggtcgccaccgtcggctctatctccgtctcgatccgctcccgcgccagcgccagccgcacctgctcgcgcttccactccaggtacgggccgctcgcccaatgctgcaacgagcatccgccgcagtcgccgtactgaggcgagaccggcgcgacgcgctcggggctcggcgagacgatctcgatctcttcggcgcggccgtcgatcacccgcgcccgcaccacctcgcccggcagggtgagactggcgaacacgggcccggcgggcgtctgcgccacgccgtcgccctgcccgccgacgcgctcgatgctcaaggtctccatcgccgggcttctagccgctcgcggacccgttacaaaggccgccggcttggcgatgaacaaagatgaacggcgggctcacccaccgttcagcttgccgacgccagtatgcaacacagacggaccgagaccgttaacggaccagcgttcaggtctcgatcacaggaaacacaccgatgccgctgcatctctcccgcaaatccctcgccgcctcggccgccgtcctggccggcctcgtggagctgcccgccgtcgcctcggcccaatcctacggctatggccagaactatggcaccggcgcctacggccgcacctacgactacgaccgcgactatcggtatgatcgcgactatcgcgatgcgcgctgcgatcgcgagcgctccggccgcaccggcgcgggcgcggtgatcggcggcggcgccggcgctgtgatcggctcccagctcaccggccgcagcagcaagaccgaaggcgcgctgatcggcggcgccctgggcgcggtgatcggctcccgggtcggacgcggcagttcggacgcctgctacgaccgcgccggcggctacgactacgactaccgctacgaccagccgcgctattacgatgaccgctacaccggcgatcagggctattacgacgaccgccgcgactacggctacgaccgcggcggctactacaaccagtacccggcccagtacggcgggggctactacaaccagtatccggctcagtacggcggctacagcggctacagcgggtacgccggcggctacagcagctacagcggctacggccagtcctattcgtccggctatggctatcagtgccgcagcgtcagcaccacgacgcgggaccgctggggccggctggtgaccagcacgcgcgaggtctgctgacccgccacgccatcgcggcgtcgatcattttcagcccccctgtcgatcgacgacgtgctgggagccgccggaggagccatcccccggcggtttctcattgtgcggcccgcgtcgcccacagcaggaactcgacattgccgtcgccgccggtgatcggactctcggccgtggcctgaaccgtccatcccgaccccgtcagccaatcgaccacgcgggccagcgccgcctcgcgctgttccgcgtccttgaccaacccgcccttgccgatccggtccggcccctcggcctcgaactgcggcttgaccagcgtcacgaggtcggcgtcgggcgcggcgagcgacagggcggcgggcagcaccttggccaagccgatgaagctggcgtcgcagacgatcagctggggcggttcagggatcaggtcgggcgtcaggtcgcgcgcgtcggtccgctccaggctggtgacgcgcgcatcggcggcgagccgggggtgcagttgaccggaaccgacgtccacggcgaacacccgacgcgcgccgcgttcaagacagacctcggtgaagccgccggtcgaggcgcccacgtccagcaccacccgcccctccaccaccaccggccacagcgtcagcgcgtgatccagcttcagcgcgccgcgcccgacgaaccggtgcgccgcctccgcctcgatcgcggcgtcctcggcgacctgctccgaaggcttggccacggcgcgcccgccgactcgcacccgccccgcctcgatggcggctcgcgcccgggcccgggtgtcaaacagcccgcgcgccaccagaagctgatcgatgcgcaccttcacgcccttctccccttgcgggagaaggtggctcgcggagcgagacggatgagggggccgctcgatccggatgcgacgtctgccagaggtgcaggctgattcagccccctcatccggccccccgggccaccttctccctcaaggggagaaggatcacagcgcctccagccgcgtcagcgccgcctgcagcttggtcttgccggcctcggcctcggccagtttggcgcgctgctcctcgaccacctcgggcgcggcgcgggagacgaagttggggttgccgagcttcttgttcacgtggccgatgtcgctgtcgaaggcggcgatctccttctccagccgcccgcgctcggcggccaggtcgatgatgccggccagcgacagggcgaccgtggtcccgcccgccaccatcgtcaccgcacccgcaggcgccgcatcggcggtgtcgagactggcgacgcgcgccagggtcaggatcaggtcgcggtggcgggcgatgcgctcggcgcccgccgcgtccggcgacacgaacgtcaacggcggcttggccgacggcggcacgttcatctcgccgcgcagggcgcgcacatcggtgaccagatcgaccagccagccgatctcggcctccgcctccgcgtcgatgaagctgtcgggagacaccggccattcggccccgatcagcaggctgtcgcgcaccggacccgccttgccgagctcggcccacaactcctcggtgatgtagggcatgaccgggtgcagcagcttcagcgtctgatccagcgcccaggccgtcgtggcgcgggtctcggccttggcggcctcatccgatccttggaacaccggcttggccagctccagataccagtcgcagaagacgttccagatgaagcggtagagcgcgcccgccgcatcgtcgaaccggccgccttcgatggcgtccgacaccgcacgctcggccttggtcagttctccgcgaatccagcggttgatcgtgccgcccacattcgcggggtcgaagccgtcgacgcgggcgcagccgttcatctggctgaaccgcgcggcgttccacagcttggtgccgaagttgcggtagccctcgatccgctgcttcgacagcttgatgtcgcgcgtgcccgagaggatcgccatggtgaagcgcaagggatcggcgcccagttcgtcgatgatgccaagggggtcgatgacgttccccttggacttgctcatcttctggcccttctcgtcgcggaccagaccgttgatgatgacccgcctgaacgggacctcgcccatgaagtgctggcccatcatcatcatccgggcgacccagaagaagatgatgtccgccgccgtgaccaggtcgctggtcggatagaaccgctggaggtcctcggtcttctccggccagcccatggtcgaaaagggccacagggccgaggagaaccaggtgtcgagaacgtcctcgtcgcggcgcagcgtctttccgccggacgcggcgatcgcctcgtcctcggtttcggcgacatagaccgcgccgtcctcgtcataccaggcggggatctgatggccccaccacagctggcgcgagatgcaccacggctcgatgttgcgcagccattcgaaatagatcttttcgtaggacttcggctcgaacaccgtgtcgccctgctccaccgccttcagcgccggctgagcaagagtgtgggcgtcgacgtaccactggtccgtcagccacggctcgatgaccacgcccgagcgatcgccgtgtggcacaacgtgcttggtcttctcgatctcgcgcagccagccctcttcctcggcgcgggcgacgatggccttgcgcgcggcgaagcggtccatgccgacatagtcgcctggcacatccggcgtgtcgccgtcggtgatgcggccgaaggcgtccatgacgttcagcgcctccagcccggcccgcttgccgacgccgaagtcgttgaagtcgtgcgccggggtgatcttcaccgcgcccgaacccttggtcggatcggcgtattcgtcggccacgatcgggatgcgacggccggtgatcggcagggtcacgaacttgccgaccagcccggcgtagcgcgcgtcgtccggatgcaccgccacgccggtgtcgcccagcatggtctccggtcgagtggtcgccacaacgatgaagtcgcgcatctcccactcggtcgcctcgccctcttcgccgaaggcgatcggatgctgatacgtcacgccgtcggccagcggataggcgaaatgccagtaggcgccgtcgacctcgcgctgctcgacctccaggtccgagatggcggtctggaagtgcgggtcccagttcaccagccgcttgtcgcggtagatcagcccttccttgtgcagttgcacgaaccccttgcgaacggcggcgttcagcccctcgtccagggtgaagcgttcgcgcgaccagtcgcagggggcgcccagacggcgcagctgctggacgatggtcccgccgctctcggccttccattcccagaccttctgcacgaaagcgtcccggcccatgtcgcgccggccgatgtttccatccgccgccagcttgcgctcgaccaccatctgggtggcgatgccggcgtgatccgtgccgggcagccacagcaccgccttgccccgcatccggtgatagcgggccaggatgtcctgcagcgtgttgttcagcgcatgcccgatgtgcagcgaacccgtcacattcggcggcgggatgacgatcgaataggcgtcggccgcgccgtcggtcgcctgcgcggcgcgcggcgcgaacaggccgctttcctcccattgcgcatagagacgcggctcggcggcctggggatcgaaggttttttcaagcatgacggtgtgtcttcggaaatgcgaaggggcggccccttcaggagccgcccctcggattagtctcggctgaagcgaagggctaggcgctgcgcgcgatgcgttcgacttccttgcgtacctgggcctcgacgatggccggcaggtgggcgtccagccactccttcagcatgggacgcagcagctggcgcgccagctcctcgacggtgacgcccccgatgcccgatccctcttcggaagccggctcgggcttcttgaacgaggcggcgagacccgcaaaggccgaggcggcgctggcggcggcgctgtcgccgaccagggtgtcataggcgggagcggcggcctgcggcgcatcctcggccgacgtcggctgcggcgcggccgggaagggctgatcggccgggtccatcacgtccagatcgccgatgctttccgtaggcgcctcgtagcggtcggtcagttccagcacgtcgtcctcgccggccggcggctcgggctcggcgggcggagcgaagctggtcggcgcctctgccggcgtgtcttcctcggcggacgcggtggcggccggcggcgtcgttccggcggtgtccgccggcgcgtcgtcctcggagatgatccggcgaatcgacgccaggatctcttccatggtcggttcctgggactggtcggtcatggcgaaaccccgagagaagatcgaaagaatggcggcgggcgaagcggcgtcgccatgcctggacgccctgtcgtcgcatcaacgcccgtcggaatcaacgggccttgacgctgaaggcgatcaggacgccggggcggtctggacgacctggcgcttcagctggccgtcgatgggcgcatcggccgtgtccggggtctcgaccaccaccggcgcgccgatccggtccagcgtctcgaccacgccgtcccagggcaggcccccgcgacccttgacctgctcgtagttggcggccggatcgtaggcgggcagcgtcggatcgaggtccggtccgcccagtcggcccatggcggccagcagcgaggccttggcgacgtattcgttggcgcgggccgaggccagggtcacctgcgacgagcgcagcgtcagctcctgctgcagcacgtccagcgtggtgcgcaggccgacctgcgcctcctgccgcacgccctcggccgcgaccgatgcggcgcgcaccgcctcctcgcccgccgccagcgtcgattgcgccgacagcacctgggcgtaggccgagctgacgctttgcagcacgctgcggcgctcaccctcgacaccgatctgggcggcgttggcgcgctccaacgcctgggccacgcgcgagcggttcagcccgccggtgaacagcggcaccgacaccgacgccgtggcgctgaacgcctggcggtcggccagctcgcccaggtcgccgaggttggaggtcgaggcgccgtaggacgccgccagccgcgcggacggcagatattcggcgcgggcctgggccaccgccgcctcagccgcctgctggttgtaggtcgccgccaggatgccgggattggccgccagcgccgcatccagcgccgcctcgaactcggtcgggatgggcggcagcagcggcgcggcctccaggtcggccggggcctggcccacgacggcgacgtagttggcgcggctgatcgacagctgcgcctgggcgttggcgaggtccgcctgcgactgggccaggctggcctcggcctgcgccacgtccgtgcgggtgatctcgcccacttcgaaccgcgcgctggtctcctccagctggcgttgcagcaccgtcaggttctcctggcggatgcgcaggatctccaggtcgcgcgtgacgttgacgtaggcctggatggccgagaccatcacctgctgctcgatgtcgcgcaggttctctcgcccggccagcacattggccagggccgcgtcgatcgccagcgaggtgcgcccgccggtccagatgttttgcgacaggctgacgcccacatcagcggtgtcgctctcagagtctccgcggatcacggtggtgtcgggaaagccgtccccgtccagatcggtcgtgccggttacggaggtgtttggcgcccagacgcgcgaatagccgacgctgccggaggcgctgacctgggggcgcagtccagcacgcgcttgaaccacgctctcgtccagggcgcgttgatttgcgcgctgcgccaggaggttggggttggtctgataggccagcgcaatcgcctcgcgcagcgtttccgccgaggcgggctgcgccagagcgaccgacagggcgaccaccgccaccgacgtcaggccaagcttgcgtttcaacatagtccgtcctcgttgacgccggccgtcggcgtcgaattcccgtagcagcctaactggcgtctagcctgacgccgcgccagttaagttttcttcacgctggccgtcgctcagagtacgaactgcggcgccggcgtcatcgtttcgagcaccgccggcgacgaatcaaacagcggccgacgggacaggccctcacgcccccgcacgtacagcaccgccttgccgaccggcccctgccgttccaccacggccaggcggccgccgacccgcagcttttcgatccaggcgtccggccgcacggccaccgcaccttcgctgacgatgatgtcccagccctcgccgtgcggctgatccagcggcgcgaccaccgtctgcacgccctcgtcggccagcgcgggagcgaccacgtccatgaccgcctgatcggcttcctgcgccgtgaccaccgccttcatgcgctgcagcacggcggcggcgtagggggcggcgatggccagcgcacgctcgccctcgcgcacatccagcgcctgcagcagcttggccacgtcgcgcgcctccatcagccgtcggtcgccggcgatctggaccggcgcctcggcataggcggcgaacgcccgctccggatcacagaagcgttcgcgcgggacgaccagcagggcggcctgcagggcgcggtcggtgacgtcgttcacccgcacctgcgaatcgaccatgaccttgcgcgcggcggtgaaatccatcggaacagccttggggaagaagcgatcagcgtaaaacttggcgcgcttataggtccgcgcgttgcggcggacaatccgatctgatagcgaacgcccctcgcgatggaccgcccccctccaaggggcagcggcctgatggcggagtggtgacgcagaggactgcaaatccttgcacccgggttcgattcccggtcaggcctccatcgcgatcgtccccctacccgcagctccgtcccggcccgctcagcgccgggctggtcaggtgatgcagggcgatggcgcttgtcgccgccacgttcagcgaatcgaatccgccgtgcatcggaacgccgaccgcgcggcagcgggcgatcacatccgtcgacaggcctggcccctccgagcccagcacgatcgcgacaggacctccgcggcgataggcggccagagtctccgatgcgcttggcgtcggggccagcacctcgaacccgcgggcgatcagccgccgcaccaggtcgccggccgatccgccgacggcgaagggcgtcctcagcaccgccccgaccgacacccggatggccttgcggtagaagggatcgcagcatcgctcgtccagcagcaccgcgtgcgcgccgaacgccgccgcgttgcggaacagcccgcccatgttgtcgtgattgccgatggcggaggcgaccaccaccgccgtctcgcccgcgccggccaagagatcatccacgcccgtcgaccggggtttctcgcccagcgccgggatgccccggtgcagcggaaagccggcgatccggtccagcaccgcctgcggcgcgacataggtcggcgcctccacgctgcgggccacatccgccatcgcctcggccctggcgtccgccagcagcagggcgcgcgtccgacaccgggaggcggtcgaggccagcacccgcaccaccacctccccttccgcgatgaacaggccctggcggccggtcaggtctcgctcgcggatgtcgcgaaaggcgctgatgcgagggtcttcggggtcgtcgatgcggatcatgcggttttcttacacttagccgttgcgcaatccgaaaaggcgctgctataggcccgcctcccgagcagctgttccgcggtagctcagtggtagagcagccgactgttaatcggctggtcgtaggttcgaatcctacccgcggagccactcggcgtttgatcccctgctggcgaaatcggtcttgcgacgcggtcctttgtaggacagcgcggtcgatttgggtcaagcagacgtcgaacacgcgccgcagcgcctcaggcggcggacgccgtcagcccccgtccgccatagtcgctttcggagaatgcgaccgcctcctggatctgctccgcgagccacagcgtggcttcgtcggcgagagatcgctcgtgccagaccacatggtagtcgaacgtgggcagcgtcatcggaagctcgaaagtctgcaggtcatagatgcgggcgaagtgacgggccgctctggccggcaggatcgcaagggcgtccgtttcggcgaccatgaagggcacgctggagaagctgggcgcggccatcagcagcttgcgacgacgcgccttttcatgcgcgtgcttaagcggatcggcgaagccctcgcccaccaatgctgcgatgtgaggccaggcgaacagggtctccagcgtcatggcggctcctgcggcgggatgggctcgccgcatcagccccagtcggctctcggtgaaaagcctgcgaccgcagacgccggcgccctccggcgggtagccgatgatcacgaggtccagccgaccctccgccagcctgttcaggctgccggcggacagcgcctcgacctccaggcacgcgccgggcgccgctttggccaggaccggcgccaccggcctgatgacggtgaggatgccgaagtccgtggacgcgacgcggaaggtgcgatccagactggaggggtcgaagcactccggccgcagcagagcttcgccttgcctcagccagccctgcagcggtgcggcgagggcctcggcacgcggagtcagcaccatgccgcgacgtccgcgcaccagcaggggatcgttcagttggtcccgaaggcgcgccaggatgcggctcatcgccggttggctgacccccagtcgatcggcggtgcgcgacacgctccgtgtctcgagcagggtctccaggctggtcagcaggcgcaaatccaggtgacgcgaggggtgcaagatgatcgcctccggtatgtcgcgcacgcatgatgatcatgcgcaggtcgtcatcgccctaaatgcgaatgactattagatgcgcggtgcctcgcctgaaacggcggagcctgtgtcgcgctagcggcggatcgacgcatgtcgagcccgtcgtgcgtcttcgtctggggagcttcatgcctgtcttcacgtcccgctcgcacgtcttgagcgccgtccttctcgccaccaccgccctttacgccgcaggcgcgcaagcccagagccgggtgcagagcccgcccatggcggagctggacgaggtggtggtgaccgcagcagggcgcgagcagcaggtcaaggacgcccccgcatcggtcagcgtcattacgcgcgagacgcttgagcaggcgccctatcgccaaatcacggacgccttgctggacatccccggcgtcaccatcacacctggggaaggcaacagccgcgacatctccatccgaggtctcggcagcgcctacaccctgatcctggtggacggaaagcgactgaactcgcgcgaatcccgcaccaacggcggcaacatcgccgaaagcggcctgctgcctccggtcgagatgatcgagcgcatcgaggtcgtgcgcggcccgatgtcctccctttacggctcggacgccatgggcggcgtcatcaacgtcatcacccgccgcatcggcgatgagtggaccggcagcttccgcgtcaatgggacggcgcagacggacggggactacggcgactacttcgacgcgggcgtctacgccagcggaccgctgatcgcggacaccctgggcctgcagttggcggcctcgatgaaccgccgcgccgaggacgacattctcaccggctcgcccgagcggaaggacgacagcctgtccgccaaactgggctggagtctgagtccagaccacgatctgctgttcgaagccgcctactacgatcaggagtcccttcagacggcggggcgcaccgcggccgtctcggcgactgcgccggaagggaccgagtcgatccagagccaggaacgcttcgtctactccatcaaccattccggcatgtgggggcgcgcgacctcgcagtccttcatccagttcgaggacgccacccgcaaggaaacaaacgtcaacatcaagaacaccgtcgcccagacggcctggatcgtgccgatcggcgcgcacatcctgaacatcggcgcctactacaacttcgccgacctttatgcgccgagcggcaacggcctgacggtcgacggcagggtccgtgacgccgcggatcggacgcagtgggccctgttcgccgaggacgagtggagcctgacctccaacttcgccctgaccgccggcgcgcgcctcgacgaccacgatctgtatggctcgcggatttcgccacgcctgtacggcgtctggaagcccgccgccggcctgatcgtgacgggcggcgtgtccaccggcttccgtgcccccgacattcgccagaccctggccgactggggccagaccagccggggcggcaacgtctatggcaatccggatctagaggccgagacctccctgacctatgaggccagcgtgatctacgaggtcggccgcgacctcgagatcggtctcaccgcctatcagaccgacttcgaagacaagatcctgcgcgtcacctgcgtggaggccggcgcctggtgcgtcagcgaaccggccaacagctccggccgcttcggcaccacctacatcaacgtcgacgaggtccgcatccgcggcctggaggcgacgcttgacgcgcggctgaccgacagcatcaccttcaaggcgaccggaaccctgaacgactccgagcagctgaccgggaccaacgccggcgccgccctgaacgagacgccggaggcgcaggccagcgcggccctgaccttccgtcctcggaacttccgggtcagcggctatgtccgcgccatctactatggcgaggaacagcaggcggcgctcgccatcagcgcctccaacatcatcgccccggactacgtcacggttgatgtcggcggctcttacatcgtcaatgacaaggtgacgctgcgcgccggcgtccagaacctcttcaaccacgagatgacctatgaagactacggctacgtcaacgacaaggcccgcgtctgggctggtctgaccgcccgcttctgatccagccgaggaaccctgagcatgatccgcacccccttagccaccgccgccgttctggcgcttctcggcgccgccctgcccgcttcgtccgccttgacgcaatccgccttgatcttccccgcgccggccaagacgttcgaggggcgcgtcagcttcgcctccgccagccagggccagccgatcctgccggggaccgaggtcgtggcgaccggccagggtttcgcgcccggccagaccgtccagctgctgcacggaaccacctccgtcctcggcgatgtgacggccgacgcagagggcggcttcgaggcccgcttccgcctgcccgccgatgcggccgtgggcgtccatccgctgatcgtcgtctcgcccgcgccctacgcagcggtggtggcggaactgaaggtctcgccagccatcccggcctcgggcgaggaccactacgacatccttcgcggcgcggcgacgcgcggactttatcagtcggcctacagcgccaagaacgacgccatcttcgtcgcttccgcggtgggtcgtccgccggttcggcagtccgagcttctgcgcatggacgccgacaccctggagatcgaggcgcggatgacgccggcggcggctccggcccgcgttggacgtgacggcgcgccggctgatggcggcctctacgccgtctacggggtcggggtcgacgatgttcacgacaccgtctgggtgacccaaagccgccagaacactgtggcggtgtatcgccagtcggacctgtcgctggtgcgccagttcgatccgggtacggtcaatcacgcccgcgacgtcgtcgtggatccggcgctggacaaggcctacgccagcgccacctttgaaccggaagtggtcgtcttcgacaccgcccggcccgaggtcgccagccgcatcgccatcgcgtccggccgacgcggggaacgcttctccgccgccagcctgtcgctgaacgccgccgctcatcgcctgtatgtggtgagcaacagcaccaacgaggtcgccgtcatcgacacccagaccgacgcggtggtgaaggtcctgcccgtgccgggcgcccgcagcgccatcggcgtgtcgcacgatccgcagaccggccgcatcttcgtggcggcgcaggggtcggacaatgtggtgatcctggacggtgaaagcggcgccgtgatcgccgacacgccggtgggcgccggcgccctgaacgtcgtcttcgatccggtcagccgccaggcctttgtcgccaatcgcggctccagctccatcgccgtcatcgacgcggacggcaggctgctggccaatctggacggcgcgccccaggccaatcacgtcgcgacggacggccagggcgtgatctacgccgtgaccaagggcggagaccaggacgacgccaacaccgtgtggcgcatccagccgaagcgctgatccgtctcgaactctcgcacccgtccagccccaagcgggcgggtgcgtcagccgtcgctggcgtgacgcagcgcgtcgggcagcagggcgaagggggccgagccatggtccgctccaggcgcaaggtggaagcgggcctgccggccgggcgtgctggtcgcccaatcctcgatcctgccccgcatgttccggcgcgtctcggcctcgccgcaaccgaccatcaacgccggtccgccgatcgcgggatcgggcgttcgccaccacagggacgggctgatgctgatccacctggcgaacaggtcgggcgcagcctccagcgtctccagaacaaaaaggcccgccagcgaatggccgaacagggtcaaccgtctgctgtcgatcgccgccgtctcgagaatgcacggcagcacctcgtcgaccagtcgatcgagaaagccggcgccgccgcccccttcgcggctcacgtccggttcggcgcagggatatcgcgtgaaatcccgtgcgcgccggtcctccatcgcgccgccgctccgtcgcgtgaccgccgccacggccatcgacgccacaccggtcttttccgatcgacgcgaaagggccgccacccccgccgccgccgcgccgaagaagcgatcgccgtccagcaccaacaaacagggccgaccatcctcgggagctgcgtcgtcaggttcgtacagcatgagctccagcgcgccgcccggcccatccaacatgagggttcgatgtccgggcgggctccagggcgtccagttcatgaggccggattgagtcatgcgccctttctagcccaaggccggcgggtgatgtactgcgacgcagtctcggtatgaaaacagccctccccctctccgcagccgctgaaaaggttctggctcagcaccagagccagcgcctgcgtcgccgcaccgtgctgctggtcctcgccttggcgtgcgcactggcgctggcgcttgatgccgcgacgggcccgtcggcgatgccggcgtggcgcgtcgttaccgggatcgtccgcccggacctgctgagcccggccgaggcggccattgtctggcagatacgtctgccccacgccctcacggccattctggtcggcgcggcgctggccctctcgggcgccgagatgcagaccgttctgaacaatccgctggccagccccttcaccctgggcgtctcgtccgccgcttcctttggcgcctcgctggcgatcgtgctgggtttgggcctgccctttgtgcccgccgacgccgtcgtggccctgaacgccttcgtgttcgccttcggctcggtgctgctgctccaggccatggcgagggcgcggcgtggcggcgtgcagagcatcgtcctgttcggcatcgccctggtgttcgccttcaacgccctgacagccctggtgcagttcgtcgcctcgcaggaggcgctgcagcagctggtgttctggaccatgggatcgctgtcgcgggccagctggcgttcggtggcggccatggccttggtgctggccgtcgccgcgcccttctcctgggcggccgcgcgcaccttgaccgccctgcggctgggcgaggatcgtgcggccagcgcgggcgtcgatgtggcgcgccttcgcttcttgtcgctgctgcgggccagcgtcttgtcggcggcggccgtggcctttgtcggcgtggtgggattcatcggcctggtcgggccgcacatcgcccggctgctggtcggcgaggatcaccgtctctacctgccggccagcgtgctgagcggcgccctgctgatgtccctggcctcggccttgtccaagaccttggttcccggggcgctgctgccggtcggggtggtcacggcggtgatcggcgtcccggcctttctgatcctgatcttccgcagcggggcgcgcggatgagcctggtcgtcgaatccgtcggcgcccgctacggcgagcggacgatcctgtccgacctgtcgctgcagccgttggccgccggccatgtgaccgccctggtcggtccgaacggggcgggaaagagcaccctgctgcgcgccatcgccgggctgctaccggcctcgggacaggtgcggctggacgacatcgccttgtctcggctgtccgtcgccgagcgcgcccgccacgtcgcctacatgccccagaccctgccgcaggacgtggccctcacggttctggagacggtgatcgcggctctggaggcttcgcctctcgccgccggcccctctcaggcggaagctcgggcgctggctgcgctggaacgggtcggggccatggacctggcgctcaaacggctggaccagctgtccggcggccaacgccagatcgccggcctcgcccaggccatcgtgcgggagccgcgcgtgctgctgctggacgagcctaccagcgccctggacctgcgccatcagctggaagtccttcgcctagcccaggattatgcgcgcgaccaggctgcggtggtggtgatcgtgctgcacgacctccaggccgccgcgcgggtctcggaccacatcgtggtgctggccgacggccgggtccacgtggaaggcccgccccgcgacgccctcacctcaacccccctggccgacgtctggcatgtccgcgcacgcgtcgaaccgtgcgcgcgcggacagatccaggtgatggtggacgacgtcctctaggcccgccgttcagggacggatccggacaaccgtgtcgcccgccggatcgtccgggaccggtgtgcccgccggggcgtcgcgcggcaggccgcgggccctgttggccaaatagacggcgtgcgtctcgggatcgatggcgatcgtctgcgggaaggtgcccgtccgcagttgggccatcaccgcatagtctgcgccgttgacgaccgtgaccgtccccgccaggcgattggcgacgtagatacggtcattccccgcgtcatgggccacgctcagcgcgccgtctccggttggcaccttgcggatgatcgaaccgtcgttcgcgttcatcaccgtcaggtctcccgatccctggctggcgacgaacaggcggccgcgttgcgcgtcgtaggcgacgttggtgggacgctcgctctgcgtcggccagcgcgctgttgtccggccggtctgaaggtcgatgacgccgatgtccgccgaagtcatgcccgtgacgaacaggcgagcgcccgcggagtccagcgcggcgccggtcaaaccgccgacctccgcgtcgatcttgcgttccagcctgtgtgtcgcgccgtcgatgacccagatccggttcggccggctggtgtctccggcgtatccgccgacgatggtgacgtagaccttgttgcgcgcctcatcgacgacgacctcgcggacgtgggcggagtcgtcgtcgccgtcggtgatgtgggcgaccacctggccggtgcggacgtcaacggcgtccaccgcgcccgagcggaaggcgccgccgtagaggatctgggtgcggctgttgaagcccaggccgtagagcggactagccgagacgtcgatcaatccggccggcgtcaggtcggcgttgagacgggcgatcacgctgcgggtctcgtcacgcgggccgacggccgcgaccagaacggtgtcgtccgccggattgaagacgagctggtagaggctgccgggctcgaccttgaccgtggtctcaatggtctgggcctgtgcggcggcggcgatcgccaaggcggccacgccaccgccgatcaggctgcgaaaagcggtcatcggggtctccgttcgagaaggcgtcacgcggcggcgaggtcggcccagtaggcgccctgatagggcacggcgaggaagcggctgttgatctcgtccagggtggcgcggggatccaggtcgccgaacagctccggatggatccatttcgccagcacctccacggccacgacgtcgatgggcgagttgatgagctgatgggacaggccgtgagcccgcccctggcgcaccgccttcagggtcgcgatgccgggccgcgccgcgacccgcctcagcccggcctgcgactgctcggcggagaagcccgccccgaccacaaagccgcccgccctggccaggtgcggcccgccggtggcgatatagacgtccgggtcgcgctggatgacgtactccaggttcagcttgcccgtgggctggttcagcacgtccgcgccgatgtttcgtccgcccacgaaggcgatgtagtcgccgatgttgcccttgcccggagaggcgcagcagtccggcgtgatcatcgcgtggggttcgagaaagaccgtggggcgccggtcctgcggcacgccggccacgcgcgaggagatgcggtccagccgcgcctgcttgaaggcgacgaaggcctgcgcttgctccgatcgcccgatcagcccgcccagaagcgcaaggctgcgcgaagcgttctcgaacgggtgggaaaagaagtcgataaaggccaccgagacgccggcggcctcgagttgcgccgcctgctcgtcggacgggccggagtccaaagacaccaccgccgtggcgggccgcgccgccagcaccgcctcggcgttgaaggcgtggccggactgggcgatcttgggcagctgggccagcgccgggaacctggcgacgaaggccgcatgcatctccgggctgatgcggttcacgtccccgccccaggccgcaagcagcgacaccggatccggatggatcagcgacagggcgatcagatagcggccgtcgtcgatgctcagcttcccgcccggcgggagcgcccgcaccgggcgatcgcgcagatccttgagagcgccttcgccgcccgtctcctcgcccgcccgcccgcaggccgcgagaagggccaggccgcccagacccagcagcgcggaccgccgcgacagcgccacctcagaactcatagttcacgcccacccagtagcgacggccgtcgccctgctggtcataggtcgccacgtccagcaccttgtcggtcacattgtagacgccgaacttgatggccacgtcgtctcgcacacgccagttcgcgccgaggtcgaccaaggtgtagtcgggatacagacgccccacctggcgcggtccgtccagcaccggctggccgttggtgccgacgcgcaggccggcgttgacctcctcgccgcgataggtcaccgcgctccacaggttcagccgatcggtcgccgcataatcgaagcgggcgttgaccatgtgctcgggcgtgcgccccagcggctgcccgtcgtagagcccgcccttctgctcggagtcggtgaaggtgtagttcgccttcagcgtcagggcgtcggtcgcagcccacgtcccgcccagttccacgccctgaatgcgggcgtcgctgatgttgtaccagtagtacagctggtacagcgggtcctcgtcccagcgcagcacctcgcccggcacgtcgcagacgccgttgccgttggcgtccgggccgcacacgcgatcgtcggcgatcttgtcggtgaagtcggtgcggaacaccgtcgcattcagcgacaggtcgcgcgacggccgccacagggcgttgatctcatagttggtgctggtctcgggcttgaggttcggatcgccgatgatgacgccgcacaggcccgcgccgtagttgcagttggcgccgcccgtctcataggcgtagccctccgccaccgcgcgcacttccggcgccttgaaccccgtcgagacgccgcccttcagcgtcagcacctcgctgggtgtccagaccagataggcgcgcgggctccagtggtcgccgtatcgcttgtgatcgtcccagcgcaggcccagcgtcagcgccaggtcgtcggtcaggccgatctcgtcctcggcgaacagggcgcgctgccagacgtcgaaggtggcggcgacgttgtcgcgggcgcccgggttcacgtcgaccagcttgttctcgatcacctggccgccgaagaccaggttgtggtcgcccagcgtcgtacccgccagcgggacgttgaacagggcgtcccacaccgtgttggtgatctccggcgcacgaccgccccggatcagggttccggtggcgtcggccgtagaggtttcccgctgcgcctcctcgcgcagcaccgaaagggcgctggtcccccagctccagtcaccgttccaggcgagcgaggcgctgtcgcggctatgctcgttgcgaacgctgcgtccggtcggcgccacggtcaggccggcggtgctgaagcggtctatgcgcgcggtgtccagttgcagcatcacctcgtggtcaggcgtcggcgtccaggcgatccggcccgccagattgtactcctccgaccccatgccgcccgtgctgcttgggccgttgtagatgtcgtcctcgtcgcgttcgagcgtgcggccccagaactgcagccccagcgtttcggccacgaccggcccggccaggtagaactggccctgataccagtcgccgctgtcgccgttctcctgggcgatatagtccgccccgaccgaaccgccccaccgcggcggcaccttcttggtgatgatgttgatcacgccgcccagggcgtccgagccataaagcgacgacatcggtccccgcaccacctcgatccgttcgatggcgccgaccggcggcgtgaagctctgctccagtcccccgttgccgttgccccgcgcctcgcgtgtggactgccgccgcccatcgaccagcgtcagcgtataggcgcccggcaggccccggatcaggatgtcctgaaagttcgccccgccgctgaccgacacgccctccacgtcgcggacggcgtcgaacaggtcgacgtacgccttgttctcaagctgctcgctcgtaacgatcgaaatggaggccggcgcctccgccacgctttgcgctcgggtgctggcggtcacgacgatgtcgtccaccgctgcgggctccgccgactgggcgaaggcgaagccgggggccgccaacgtggtgaaggcgagcaaggcgaaacgattgcacatggggggttccttgatccaagagccgcgtactgcgattggttatcaggatcaagaagcatccggtgcggcgctttctccggaccgacttggcggggtctgtccgccgagcccttctttccttggatcatgggcgtccgagctgatccttaccgccgcgctcaccacgccgctcgaccgtgcgttaagccggatcggcctatgcctcggcccttcacaggggcgggccgatgctggaagcgatcgcgatactgttgctgcaggccggcgggccgaacgtcgtggcccatgcgccgcggcccctcacgcccatgtccgaccaagccctggcggctgagcggtccggtccgttcgcgggcgcgccgacgtccacggcctcggcgcccgctcgcatgacgtcttccgagtgggccgcccgcttcgactccagcgtcatgcccgttcgactgaccacccagatcattgaaacgatgatgcagccggatcgtggcgacctcggcttctactcgggctttctcctgacgcccggcaccacgatcagcgtcgcggccaccatcaacggccgggacttccagctgcgttgatccggctgcggcgcgtcaccgcggctcctgggattgtaatcccgtcgcaccccgactaatgcgaagcactcgcaacacagggtgtcatggtgcttctttcgtctcgtctgctttcctgctcggctgtctggctgctcgcctgcgtcgccgcccccgccctggcgcaggaatctgacgccgcccagctggacgacatcgtggtcaccggcagccaggtgggcctgccgccggcctatgccgggggccaggtggcgaccggcggccggattggcctgctcggcgcgctggacgtcatggacacgcccttctcgaccacaaactacaccgaaagcctgatccgcgatcagcaggcgcgcagcgtctccgacgtgctgcagaacgatccgaccatccgcgtcagcaagggcttcggcaacttccaggagctgtacgtcctgcgcggcttccctatctattcggacgacatgacctataacggcctctacggcgtcctgccgcgccagttcgtggccgccgaactgctggagcgggtcgaggtgttccgcggcgccagcgcctttctgaacggcgcggcgcccggcggcagcggcgtcggcggagcgatcaacctggtgcccaagcgcgcgcctgaagccccgctgaaccggctgaccgccacctgggacggaggcgacgagatcggcgcgtccgccgatctggctcgacgcttcgacgacggcgcatacggcgcgcgcctgaacctggtcagccgttccggcgagggcgagatcgaggatcaggacagcgaactgaacgtcgtgggtctcggcgtcgatcaccgtggtgcgcgcgcccgcttctcggcggacctgggctttcaggatcaccgcatcgacgcccctcgcccgcaggtgacgccggcgggcgcggtccccgccccgccttcggccgaccgcaacttcgcccagccctggacttacaccgacgagacccagctgttcggcgccgcgcgcggcgagttcgacctcgccgacgacgtcacggcctgggccgccgtcggcggtcgccggggcaaggagcgcaactccctggccaatccgacagcacagcccgacggaacgctcagcgccaatcgcttcgacaatggccgtcgcgacgaggtgttctcggcggacgtcggcatccgcgcggacctcgagaccggacccgtcgatcaccgactgattgcgtcggccgcacgaatccagagccgggagagcaactcctacgccttttcggactttgcgggcttcgccagcgacctgtacgatcccgtcgccgtccccgcgccgtctcccaccgccctgaccgccggctccctcagcgacccgacggtcgtcagccgggttcggatgaccagcgtcgccgtcgccgacattctgtccttcctggatgatcggctgctcgcgaccatcggcgtccgttaccaagaggtggagaaccgcgcctacgactacgacacctccgcgcagaccggcggctattcgagcgacgccacgaccccggtcttcgccctcgtgtacaagccgtcggagcgcgtctccatctacgccaactacgccgaagccctgcagcccggctcgaccgcgcccgctcaaagcggcggcctgcccgtcgccaacgccggcgaggtgctggcccccttccgatccgagcagatggaagccggcgtgaagtacgacgccggcgccttcggcggcgtgctcagcgtctttcgcaccacccagccgtccgccctgttcgacacgacgagccgcgtcttcagctcggacggcgagcaggagaaccgcggcgtcgagctcagcctgttcggagagccgatgcagggcctgcgcctgtgatcctccctcggtttggtggacacccatgctagcttttcggagctggagaggagtgtctgatgagtgttcaacgccggaactttccggattctttcaagcgcgaggccgttgaccgcgtcgccaacggcggcctgagcgtcggggcggtggcccgcgagcttgggctgcacgagacggtgcttcgtcgatggatgacgcagttcggggtgcaggcgacgggggcgtcgcggcgccccacaacgcaggcgtcgtccccgtcgccgtcggatctggcggcggaggtggcccggttgcggcgagagaacggtcagctgcggatggagcgggacatcctaaaaaaagccgcgctcatcttcggagcggcctcccgatgaagttcgggttcgtcgatgagcatcgtcaggtctggccggttcgcgtgatgtgcgcggtcctgggcttgtcggccagcggttactacgcctggcgcggtcgccccgagagccagcggtctgtcgccaatcgcgagctgaccgaggatatccggctgatccatgcggagagcagcggctgttacggctcgccgcgcgttcacgccaccctgcggcggcatgggcgtcgggtcggtcgatcccgcgtggagcggctgatgcgccgcgccggcctgcggggcttggcggccttgccgcgtcgcgcccggacgacgaacagccgccacggttatcccatcgcgcccaacaggctggcccggaacttcgaggcggcggcgcccaaccaggtctggctcgccgacctcacctacatcccgaccggcgaaggctggctctatctcgccgccatcctcgacctgcacacccgcaagatcgtgggctggtccatgcgccagaccctgcacaccgagatcgccctcgacgccctcaacatggccgtcgaacgtcagcgccccgcgcccggcctgatccatcattcggaccggggcatccaatacgcagccgaagcctatcgatcagccctggcccgatccggcatcaccccgtcgatgagccgaaagggcgactgctgggacaatgccccgatggagagcttcttccacaccctcaagaccgaacgcgttcatcaccgcgtctacgccacccgagaccaggcgcggcgagacctgttcggatacatcgagggcttctacaatccccatcgcctgcactcagcactgggctatatcagccccgctgaggccgagcgcaaagcggcttaaccccgtccacttttacgggggaagatcatgactgacttgccgcgcccgctggccacggcctgcaagcccgcttcgcgtccctccgcgtcgcgggcctccagagtctcgcgcatgaaaagtcgtttctgcgccaccaactccgcgagcaagccgaggtcggccatctgcgacggctgatcggcgtatagacggcgtagctgcgccagatgaggatcaagttgcgtcagcgcgtcggaatagggctgaaggaagcttgtctcgcccgcgatgacgtagccccggtggccggtctccgcatcttgcatcaaggaaaacgtctgctgcagcgcatggcgcgcttggtgcgattgctccacctccgcccgcaccgcccgcgctcggctgaactcgcgcctgagctcctccccagcaaacgcgagagcaaaggcaagcaggcccgtcagcgcccaaagcgcccacgaccgtaacagcgctcgcctcatcatcacggaactccaaagcccacgcggaacagccatcaccgcacacgccggccgccacttcaaggcccgctcctgggtgcatgcccggctcgatggtctgcgccacggggtgacggaccgccagcaccgcccttgctctgatcacagacccgcttgggcggacttcctgttgcctgacgtaggcggtcaatgccggtgcggccggcgggcagcagtgctgatcaaatcggcggacgccaaggtctaggctcgctgatggaacaagcatccgatagttcagacgcacgaaagccccgctttttggggcggggctttcatgtttgtcgagtttgggtgcgggagcaggatttgaacctgcgaccttcaggttatgagcctgacgagctaccgggctgctccatcccgcggcgaacggaggggcgtgagggaagaacggttcgagcgggtcccgccctcaagcaggccgaaggccgatagggcaaggattgtgtttgtcatattcggctgtccgccttgtagacccggcggcgacctactctcccgcgccttgagacgaagtaccattggctctggagggcttaacgaccgagttcggaatgggatcgggtggggaacctccgacatagccaccgggtcaacgaggcggacagcggaatatgagaagacattgtctgcgatcgttctggtctgaacgatcatcgaatgagttttgctgagaaacgatcaaaccgatcggattattagtaccagtaagcttcacgcgtcgccgcgcttccacacctggcctatcaacgtggtagtcttccacgatcctcagcgaagccttgttttgaggttagtttcccgcttagatgctttcagcggttatctattccatacttagctaccctgctgcacagctggcgccatgacaggtccaccagaggtatgtccatcccggtcctctcgtactagggacagatcctctcaagcttcgaacacccacggcagatagggaccaaactgtctcacgacgttctgaacccagctcacgtaccactttaaatggcgaacagccatacccttgggacctgctccagccccaggatgtgatgagccgacatcgaggtgccaaactttgccgtcgatatggactcttgggcaaaatcagcctgttatccctagagtaccttttatccgttgagcgatggcccttccacgcgggaccaccggatcactatggccgactttcgtctctgctcgacttgtcagtctcgcagtcaggcgagcttatgccattgcactcgacgagcgatttccgaccgctctgagctcaccatcgcgcgcctccgttacactttgggaggcgaccgccccagtcaaactacccaccacgccatgtcccgggaccggataacggccctcggttagacgtcaacgacagtaagggtggtatttcaaggatgactccaccagagctggcgccccggcttcatagtctcccacctatcctacacatacggtcgctaacgccaaggcgaagctatagtaaaggttcatagggtctttccgtctgaccgcgggaaccccgcatcttcacggggaattcaatttcactgagcctatgctggagacagtggggaagtcgttacgccattcgtgcaggtcggaacttacccgacaaggaatttcgctaccttaggaccgttatagttacggccgccgtttacctgggcttcagttcgacgctttcacatctccctttaaccttcaggcaccgggcaggcgtcagaccctatacgtcgcattgctgcttcgcagagccctgtgtttttgctaaacagtcgctaccccctggcttgtgccactcagtcctgcttgcgcagggtgagtcacgcttattccgaagttacgcgtgcaatttgccgagttccttcagcatagttctctcaaacgccttggtatgctctacctgaccacctgtgtcggtttcgggtacggtctctgctggagttatttccagggacaacgcccccgcacgcacaatccaataagtgcgtacgagttatgccatccgtcacttccagctggtgcaggaatatttacctgcttcccatcgactacgcttttcagcctcgccttaggggccgactaaccctgcgcagattagctttacgcaggaacccttggtctttcggcgggagtgtctctcacactcctatcgttactcatgtcagcattctcacttccgatacctccagccaggctcacgcctgaccttcactggcttacggaacgctccgctaccgcttgcagtaaactgcaaacccatatcttcggcgcacggcttgagccccgttacattttccgcgcaggatcgcttgatcagtgagctgttacgctttctttaaaggatggctgcttctaagccaacctcctgattgtcaaagcaatcccacatcgtttcccacttagccgtgacttgggggccttagatgatggttagggttgtttcccttttcacgacggacgttagcacccgccgtgtgtctgcccgatagttctcttgggtattcggagtttggttagtattggtaccgctcgcgcagcccgcaaccatccagtgctctaccccccaaggaattcgtcggacgctctacctaaatagatttcgcggagaaccagctatgtccaggtttgattggcctttcacccctatccacaagtcatccgaggctttttcaacagtcaccggttcggacctccagttggtgttacccaaccttcatcctgctcatggatagatcacctggtttcgggtcgtcatacgtcgaacttagcgccctattcagactcgctttcgctgcgcctacacctaacggcttaagcttgctcgacacatgaagtcgctgacccattatacaaaaggtacgccgtcaccgcgcttggcggctccgactgcttgtaggcttccgatttcaggatctgtttcactccccttgtcggggtgcttttcacctttccctcacggtacttgttcactatcggtcgtagaggagtacttaggcttggagggtggtccccccatgttcagacaggatttcacgtgtcccgccctactcgagtcttctgctgtttgacggctacggggctgtcacccgctatggccgacctttccaggtcgttcgcctttatgtcacagaagcactggcctggtcccggttcgctcgccactactacgggagtctcggttgatgtcctttcctccgggtactgagatgtttcagttccccgggttcgcttaatgatgcctatgtattcagctcattatacctttcaacaatccgccaatcgccgtccccgaaggaacagagttggaagactgtaaaggtgggtttccccattcggaaataaccggatcaaagggtgctagcgcctccccggttcttatcgcagcttgccacgtccttcatcgcctctctacgccaaggcatccgtcagaagcccttcaacgtttgatcgtttctcagcaaaactcatgcgtggtttattccacccgactggaaagatgccgggggaccacgcctgattttgtcagacaatgtcttcttctcgaacagtgacctagaagctcaggggagccggtcgcgttcttccttcacgatttcaatgccggtcggcgagcgccgacaggcaatccttgatgcgatctgcgagccttggcggggtgcgccaccgctttcaaagcggggcctcgggtctattccccggccgcgggcgcggcctggtggagccagacggagtcgaaccgacgacatcctgcttgcaaagcaggcgctctaccaactgagctatggccccgttccagccggaacagtgcgaagcccaggagagctgtcggacgatctgcttaaaggctgaagtccagcccccggcttgccagaggtcctggtaggcccgggcagactcgaactgccgaccttacgcttatcaggcgtacgctctaaccacctgagctacgggcctatggcagcgacagccgggtgcgaaacccaggctcgcgatcgcgtcaccgtcgatcacaacccgtatggctgcgtcgatgatgacgaaagtggaaagagaaacggagacggcggcgttccgcatgatgtgctcggcgctgtgaagcgcttcgctatgcggagcgtcaatagaacctcgtgagaggcgctggagacgcatccttagaaaggaggtgatccagccgcaggttcccctacggctaccttgttacgacttcaccccagtcgctgaccctaccgtggtcgcctgcctccttgcggtcagcgcagcgccttcgggtagaaccaactcccatggtgtgacgggcggtgtgtacaaggcccgggaacgtattcaccgcggcatgctgatccgcgattactagcgattccaacttcatgccctcgagttgcagaggacaatccgaactgagacgacttttaaggattaaccctctgtagtcgccattgtagcacgtgtgtagcccaccctgtaagggccatgaggacttgacgtcatccccaccttcctccggcttagcaccggcagtcccattagagttcccaactgaatgatggcaactaatggcgagggttgcgctcgttgcgggacttaacccaacatctcacgacacgagctgacgacagccatgcagcacctgtgtcccagtccccgaagggaaagccagatctctctggcggtccgggcatgtcaaaaggtggtaaggttctgcgcgttgcttcgaattaaaccacatgctccaccgcttgtgcgggcccccgtcaattcctttgagttttaatcttgcgaccgtactccccaggcggattgcttaatgcgttagctgcgtcaccgaaatgcatgcatcccgacaactagcaatcatcgtttacggcgtggactaccagggtatctaatcctgtttgctccccacgctttcgagcctcagcgtcagtaatgagccagtgtgtcgccttcgccactggtgttcttccgaatatctacgaatttcacctctacactcggagttccacacacctctctcatactcaagacacccagtatcaaaggcaattccgaggttgagccccgggatttcacccctgacttaaatgtccgcctacgctccctttacgcccagtaattccgagcaacgctagcccccttcgtattaccgcggctgctggcacgaagttagccggggcttcttctccgggtaccgtcattatcgtccccggtgaaagaattttacaatcctaagaccttcatcattcacgcggcatggctgcgtcaggctttcgcccattgcgcaagattccccactgctgcctcccgtaggagtttgggccgtgtctcagtcccaatgtggctgatcatcctctcagaccagctactgatcgtcgccttggtgagccattacctcaaccaactagctaatcagacgcgggccgctctaaaggcgataaatctttcccccgaagggcacattcggtattagcacaagtttccctgagttattccgaacctaaaggcacgttcccacgtgttactcacccgtccgccactaaccccgaaaggttcgttcgacttgcatgtgttaggcctgccgccagcgttcgctctgagccaggatcaaactctcaggttgagttgacttctgacctaagcttaagaccaccaaaatggccttggcattagttctacgtattcttgacgagttcccacgtcatcgatcccaaaaaggaaccgacgcatggtatcttcaaaaagaccgcagatgtcagtgtcgattgacgttccgaagaacgtcgctagaacaccgccgcctgcgtttctctttccagatcaacgatttcaaagacccaggaaccgatctctcagtcccgccgtttatcgcccggctgcggcggaggcggcgatttagtcgcctcggtgatccgtgtcaagcggttctttttgcgaagaacctctttcaccaaccgacccgggaaactcccgaaaccggcggaggcggcgatctaccgaccctccaactccccgtcaagctgttctttttacaaaagaacctctctccgaagacccggcccgaagaccggaagaggcggcgatctagcgacccccgaacccctcgtcaaccggcttttccaaaccgccgcaaaccgcgaaacctaagcctcacaacccgcagaaaaccgcccccgaaacccagccaaaaggccaagccccagacaaaacaaacaatagcgattccgtcgaagcgcggaagatggcgccgaccgctggaaaccgcaagagcgaactctccgatttcctgtgggcgggtcggtgtctccaccgcgtcccggccctccggccagcccgtttccgagcgaggcggctctataggcaggcctctcgggcgcctcaagcgaaatctcacggaacgtgggaatagttcgcgggcgtcaaggctggcgcacctgccgcccccttccctatcttccccccatgaccgacgccgtccccctctccctgcctgtccgatcgcctgaactgctggcgcgcctgcgcacgcggcgctcagcgcccgcccaggcgctggaggcgcccggcccctcggacgccgaactgacgcagatcctggagatcggcgcccgcacgcccgatcacggaaagctcgcgccgtggcgcttcgtggtcatgggaccgcaggtccgggcccggatcgccgcggaactcgtcgtactcgcggagcgcaagcgcctgccccccaaggcccaggccgtgttggccaagctcacggccgccccgctgacggtgctggtgatctcctcccccgttgccgacgacaaggtgccgatctgggagcaggagctgtcggccggcgccgtgtgcatgaaccttgagcacgccgccggcgcccttggctattcggccagctggatcaccgactggtacagcttcgatgcggaggcgaccgctctgttcggcgtgcgcgcgggcgagcggatcgccggcttcatccacatggggacgctggcccagccgccgctggagcgcccgcgtccggacctgtccgccatcgtcacccgcctggcctagccggctccggctcgggccggtgcaccagcgacaccagcacgatcgacacgatcatgagcaggaaccagctgcccagcttggccagcgacaccatctcccaccccgattcctgccccggataggcccaggcccgcgcgaaggtgcccaggttctcggcgaaccagatgaagatcgcgaccaggccgaatcccagcagcagcggcatcgatcgtctgcgccggtcggcggtgaagaagaaacacccgcgcccgaacagcacggcggtcgccatgaacagcacgatccgcacgtccggcagccagtggtgggcgaagaagttgacgtagatcgccgccgccagcagccacgtcgtccacaagggcggatagcgccgcacgcggatatgaaagatgcgctgcacccgcgcgatgtagctgccgaccgccgcatacatgaagccggagaacagcggcaccgcgccgatcctcagcagcgagtcttccggatagatccacgatccatgcgccgtcttgaacagctccatgaccgtgccggcgacgtggaacaggaagatgacccgcgcctcttcccagctctccagccggaacagcagcatcgccgcctggatcagaagcgcgccgatgaccaaaaagtcgtagcgcgacagggccgcgtcctccggccacagcagataggtgccgaaaatcagcgccagcatcagcgcgccgaacaggcacgcccacccctgcttcagtccgaaccacaggaattccagcccataccggctccacgcgcgacggtctccccacgcctgcagccggacgagccgggcgcgcccccacgcctcgagcggaagtcggggcgcccccgccactgcggatcagccgcggccgcgataggtcggcacgccctgatcgggcagccacaggccctcaggcgccgcgcccgtctgccagaagacgtcgatcggaatacccccacgcggataccagtagccgccgatccgcagccacttgggctgcagcaggtccgccagccgccgtccgatcgagacggtgcagtcctcgtgaaaggcgccgtggttgcgaaagctggtcagatagagcttcagcgacttggactcgaccagccagtcgcccggcgcatagtcgatcaccaggtgggcgaagtccggctgtcccgtcaccggacacagggaggtgaactccggcgccgtgaaccgagccagatacagggtgtcggcatgcggattgggcacgcgctccaacaccgccgtttcgggatcggcgggcgcggcgggccgcgcgccccggtggctgagggcggggacggccgtgggctgtctcttttaaacaacccccagcccacgagaatcctgagcaacccgcatgccgtcttcttctttaaaaaaaaaaaaatatcattactcattctaatacatactaaaaccatcttattactcatactgtgatt

SEQ ID NO: 9 - DNA, 56815 bp, brevundimonas massiliensis
  source 1..56815: mol_type = genomic DNA
atttactctatttttttttttttttttcaacaaaaaagcggccaaccgatttgccagggattctgggggccggggagttgtttaaaagagccactccctgcaccgatcgagtatcccccccgaccctctcgatcctgagccatccccaggaccggcgcgacgggcatgaccccgccgctcccgctccatccgctcccgccgctcgcaaggtcgcaggccaagcgagccctccagtgcgacgagacccatgcaggatggcacgggcgggagctcgggcgaggaagtcgaggtggggtttggctaaggggctgttcaggcgcgggtttgtcccggctgatgcgttggccgcgcttcttttctcgtcatcctcgcccttgtggcgaggatccagacgcccagtcttcgccgtgaagcaccgggagtctggaccctcgggacaggcccgagggtgatggggagagaggtggaaaaaaagggggacgcgaggcggcgttctccctccccgggtggtcgcgtcagcgaccgggtggggcggctcggcagggtcgcacggatcgaagcacgtcaggtcgtcgatgggtcgcctggccgcccctacccggcttcgcctgcggctcagccaccctccccgttcgggaagggagaatgccggtctcctctcctcccccatcggcgatggggaggtggatcggcggcggagccggcgagacggaggggtcctaagccctcgccgcccgtgaggcgtcgacgccgagcgcctgaagggaggcggcggcgatgtggtcggcgttaagaccggcggcggcgtacatggcggcgggcaggtcctggtcctggaagacgtcgggcaggtgcagggtgcgaatcttcagccccgcgtccagcgccccctgttcggcaaggaactgcagcacgaaggcgccgaagccgcccatggccccctcctccaccgtgatcagggcctcgtgctcacgcgccaggcgcaggatcagctcgccgtccagcggcttggcgaagcgggcgtcggcgacggtggccgagacgccgcgcgcggacaggaggtccgccgccttcagcgattcctgcaggcgcgtgccgaacgacaggatggcgacggaggtcccttcgcgcacgatgcggccgcgcccgacctcgagcggggcggccatctcgggtatctcgacgcccacgccgtcgccgcgcggatagcggaaggcgctggggcggtcgtcgacagccagagaggtcgagatcatggcggcgaggtccgcctcgtcggcggcggccatcagcaccatgccgggcagcgcgcccatgtagccgatgtcgaacgagccggcgtgggtcgcgccgtcggcgcccaccagccccgcccgatccatggcgaagcgcaccggcagcgactggatcgccacatcgtgcaccacctggtcgtagccgcgctgaagaaaggtcgaatagatggcgcacaccggcttcatgccgtcggcggcgaggccggcggcgaaggtgacggcgtgctgctcggcgatgccgacgtcataggtgcggtcgggaaacgcctggccgaacaggtccagcccggtgccggacggcatggccgcggtgatggcgaccaccgacggatcggccttggcgtgcttgatcagctcggtcccgaacaccttggtgtagctgggggcgttggagacggacttggactgcttgcccgagaccacgtcgaacttgaccacggcgtgcagcttgtcggcgctgctttcggccggggcgtagcccttgcccttttgcgtcaccacgtggaccagcaccggccggtcgtcgatggcggcggcgttcttcaggatggggaccaggttctccatgtcgtgaccgtcgatcggcccgatgtagtagaagcccagctcctcgaagaaggtgccgccggtgaccatgccgcgcgcatactcctcggccttgcgggcgacgtcgcggaaggggcgcggcagatgctcggccactgacttcccgaggcggcgcacgttctgataagcgccgcccgacaccaggcccgccagataggcgctcatgccgccgaccggcggcgcgatcgacatgtcgttgtcgttcaggatgaccaccagctgcttggtggtctcggcggcgttgttcatcgcctcataggccatgcccgccgacatggagccgtcgccgatgacggccacgaccttgttggtctcgcccttctggtcgcgggcggcgcagaagccgagggccgccgagatggaggtcgaggcgtgggccgcgccgaacggatcgtattcgctttcggcccgcttggtgaagccggacaggccgcctggctggcgcagggtgcggatgcggtctctgcggccggtcaggatcttgtgcggatagcactggtggccgacgtcccagatcaggacatcgcgcggcgtctcgaacacatggtgcagggcgaccgacagctcgaccacgcccaggcccgcgcccagatggccgccggtgacggacacggcgtcgatggtctcggcccgcacctcctcggccagctgctgcagttgcttgacggagaagtcgcgcgtgtccgcagggatgcggacggtgtcgagaagcggggtgtcgggcatcaggcgccttggctggtcgtgtcgaggccgccttagaatggcggacgtttccttatcaggacctgcgttttagcacgaagtccacgctggccttgaggatttcggcgtcgcggccgaacggatcaaggtgggcgcgcgcctggtcggccaggtgtgcgaccctctgacgcgccgcatcgagcccgagaagcgtgacgaagttggtcttgcccagagccgcgtccttgccgccggccgccttgcccagctcctccgtcgtgccctcgacgtccagcaggtcgtcgacgatctgataggccaggccgatgtcgtgggcgaagcccagcagcgcatggcgatgcgcctcgccggcccgcgccaggatcagcgggatctcgaaggcgtaggcgaacagggcgccggtcttcagccgctgcatgcgggcgaccccgcccagatcgtcgcgcacgcccagcagatcgatcatctggccgccggccatgccgcgcgcgccggacgccagcgacaggcgcgcggccagttcgcagcggatttcggcgtcctcgtgcgtgtcctcgtgcaggatgatgtcaaaggcggcggtctgaagcgcatcgccggccaggacggcggtggcctcgtcataggcgcggtgcagggtgggccggccgcgacgcaggtcgtcgtcgtccatgcacggcaggtcgtcgtgcaccaggctgtaggcgtggacgcactccagcgcgcaggcggcgcgcagcaccggacgctcctcgatgtcgaacagccgcgaggcctcgatggcgaaaaagggccgcagccgcttgcccggacccagcgccgcataccgcatggcctcggtcagacgcgattccggaccgtctgcgcgcggcagaagctcgtccagcgccacggtcaccaggtcggcaacctccgacacgcggtccagcacggcctgttcgggcgagttggcggcgagcacggcgctcatcagaacagccttccgccgagcggcgcgtcacgatcgacgccgaccagcaccacttccccatccgcatcgggaaagcccagggtcagcacttcgctcatgaacggaccgatctggcgcggggcgaagttgaccaccgccgccaccttgcggccgaccagttggtcgggcgtgtagtgccgtgtgatctgggccgaggagcgccgcgtgccgatctcggggccgaagtcgatcgtcagcttgtaggccggcttgcgcgcctcggggaacgggtcggcggccgtgacctggccgattcggatgtcgaccttctggaagtcgtcgaatgcgatgcggtcggcgaccggggctgcggccatcagccgaactccgccggctgcacgcccttgggctggccgtcggggccgaccacgatcttctccacgcgaagctgcgccgccttcagccggttctcgcaatgcgctttcagccgggcgccctcttcatacagggtgatggactcctccagcggagcctggccggattccaggcgcgagacgatggtctccaggcgctgcaacgcctcctcgaaggacaggtcggtcggagtggaaggcgcggcgtcggtcatcggtcgggaccctagagggggcgcgccgtcgcttcaacggctaagcggctcagcccttttcgtagcgacgttgtgaccagtatttgaagccttgatcgtgcaccagccgccagccggcggccttcaggcagcggccgaccatgtggttgaaatagccgtgggcgaagaccagcacgctttgcccgccctcggcccggcggatcagcacggccgcggcctgacgcgcgcgcgcctcggcctccagccgcgtctcctgcccgccgtggtggttgaacacgtgccaccagaagcgcgacaccccgccccaggtgcgcggcgacagacgaatccagtccgggaacggcggcggcggcagcggcgcctcgatgaacagggcgtcactcatgacctcgcgcccggcggcgacggcgcttgcggtctcctgcgcgcgctggcgggtggaggcgtagatggcgcccgccccttcggccgcggccagcagggcggcgggcggcgtctggccggcgcgcaggccgccgacttcatagcggccccaccattcgccgtattcgcgcgcgctgaggcggcacttgcgcgaaagcgccggctcgccgtggcgggtcaggatgatggcgcccgtgcggggcttggacgggctcagcacggccggagacgccgccggctgggcggacggctccgaagactgcagggacagaacggtgctgggcatggcgaacggacgaaacctgaaaagatcaggatcttggtcgtcctttagtcctcccccagcgcctctagatgggcgacagccgaacggctgagtccctcaaggtcgtagccgccctcgagagaggagacaaccatgccgcggcaggcgcgtcgagccacttccagcaccgcccgcgtggcccaggcgaaatcctccggctccagcgactgatgggccagcggatcgcggcgatgggcgtcgaagccggccgagatcaggatcaggtcgggaccgaacgtctccagcggcgccatcagcccgccggcgaaggtcgctctccacgattcgcgcgcggcgtggggcggcacgggcgcattgacgatgttgccgacgccggtctcgtccggcgctcccgtgcccggataaagcggcatctggtggatggaggccaggaacaggctgtcgtccgcctcgaacgccgcctgcgtgccgttgccgtggtgcacgtcgaagtcgaccacggcgacgcgggcgaagccttcggcctgggccacacgcgcggcgaccgcgaccgaggagaacaggcagaaccccatggcgcggtccggctcggcgtgatggccgggcgggcggacggcggcgaaggcgcgcgtcatctcgccccgagcgacggcgcgcaccgcgtcgacggcggccccggcggccagacgccccgcccgaacgctgccgggcgacagcagggtgtcggcgtccaactgggcgacgccgtgatcgggagaggcccgcagcaggcgcgcgacataggcggacggatgcacccgctccaggtccgcgacggacgcctcgcccgccaggcggcgatcggcgccgagccccgcgtcatcgatggcgtcaaaaacggccttcagccggcccggcttctcggggtgtccttcgccggtcaggtgcgccagcatgtcgggatgggtgaacaggggcacggacatggcgatgatcatagtggcggcccggcggcttgtcgcgcaccgccggcggccgtagaggcgcgaccatgacagacgccgacatccgctccgcccgccccgaagacgccgaagcgctgggcgtgatcggccgccagacctttatcgacaccttcgtcagaggcttccgcatcccctatcccgagccggatctcgagaactttctccgggacagcttcagtcccaagaccatcgccgccaagctggccgaaccgggcgccgcctggtgggtggccgagcgcgagggcgaactcctcgccttcgcaaacgcgggtcccaacaccctgccccatccggacgcgcgtccgacgcagatggagctgcgccgcctgtatgtgtcgcgtgccgctcagggactggggctcggcacgaggctgctgaccctgtcgctggactggatggaggcgcacacggacgggcctttgtggatcggcgtctggagcggcaacctgaaggcgcagaagctctacgccgcccatggattcgaaaaggtcggcgagtaccagtacccggtcggacgctggctggacgatgagttcatcctgcggcgcggatagactatgttgcggtcatgacccgcgccgaactgctggaaaagctgcgcgaactgaaaccctggctcgaggagcagggcatcgtcaacgtgcgcctgttcggctcctacgcccgcgacgaggccggaccggacagcgacgtggacctgctggtggagatgaccaagccgctgggtttcgacttcttcggcattgaggacgccctcaccgacgcccttggggtgcgcgtggagatgggcacggagcgttcgatgcacaggttgctgcgcgagcgggtgctgcctgacgccgtccatgtctgacttcaaggaccgtcttcacttggtggagatgctcgacgcgatcggcgagatcgagatggacactggcggcctgagcgaagacgcttgggttgaggtcggatcgcttgtgcgcgctgtttcgatgagcctcatcacgcttggagaaggcgcggcgcaactgagcgacgccctgaaggagtccgcgccggacgttccgtggaggcggatgatcggccttcgcaatcgcctggcgcacgcctacttccgcgccgaccgacatatcatctggcaggcggccacccagcatacccccatcatcaaagagcagcttctacggttgctcgccgctctgccggacagctgatgctgctgcccttcttcttcgccctgcgcgaggcgcgtgtgccggtgtcgaccaaggagtggctgcatctgatgcaggccatggaccaagatctggcgggacgtcgggtggaggccttctatcacctgtcgcgcgcggtgctgatcaaggacgagaagcactatgaccggttcgaccaggtgttcgggcgcgtgttcaagggggtggagacggtcgggggcgaggacctcgcgaccgagttgcccgaggactggctgaggctgctgacgcagaagcatctgtcagaggaggacaaggcgcgcatcgaggcgctgggcggcttcgacaagctgatggagacgctgaagcagcggctggaggaacagaaggaacgtcacgccggcggctccaaatggatcggcacgggcggaaccagcccgttcggccacggcggctacaatcccgagggcgtgcgcatcggcggaccgggtcggcacggacgcgccgcaaaggtctgggaaaggcgcgagttcaggaacctggacgacacggtcgagctgggcacgcgcaacatcaaggtcgccctgcgccgcctgcgtcgctttgcgcgagagggcgcggcggaagagctggacatggacggcaccatcgacggcacggcgcgccagggctggctggacgtgcggatgcggcccgagcggcgcaacacggtgaaggtgctgctgtttctggacgtcggcggatccatggacgcccacatccgcatgacggaggagctgttctcggccgcgcgcgccgagttccggaaccttgagttcttctacttccacaactgcctgtacgaaggtgtgtggaaggacaaccgccgccgcaacgccgaacgtattcccacatgggatctgctgcatcgctacaacggcgactggcgggcggtgttcgtcggcgacgcgaccatgagcccctatgaggtgtcggtgcccgggggctcggtcgagcactggaacgaggaagcgggcgaggtctggctgcgccgggcgcgcgagcagtggggccgctgcgtgtggctgaaccccacggctgagcggcactggagctatgccgcatccgtcgggatgatccgtcagattatggacgaccgcatgttcccgctgacgttggatgggctggaccgcgcgatgcgggcgctgacgcgctgaatgtggtagggcttggcgacacacagtgctggggagcctgtcatgatcgccgccgtcttcgccgttctgctgatgcagcagcccgccgcgtcttccgccggtccgttgccggagtgggccaaggccgatcccttcgcgttcgagcgcgcgcggtgcagcgccctggtccggggagagacgccgctgaacgtatgccaggccgaggtgcgccgcctgctggccgacagtctgggagacgaccttccgtcgacgatgcgcgtggccgggtcggtggacgactgccagcggctgagggatgcggccggcggctcgacctatgcggtgcaatgcggcccgcgccccgcgacgctcgcggcgtcaaaccttccggtcgaacgcgagtgccgcagccggccggatcgcaacggcggggtcacgagcgaatgccgccccatcggttcgaccgaggaagagggagggctgaagctgcgcctgttcggcgaccgggactgatcagcatgcaaaaacgccgcccgatcgctcggacggcgtttgttcagcaggcaaaccggatcaggtgcgatcgtcgcgcagcgtgtccttcacgccaccaaccgcattctggaccttgccgcccatctggtcggcgcggccctcggccttcagcttttcgtcgccggtgaccttgccggcggcttccttgaccttgccgcccatgttcttggcggcgccttcgacacgatcgtgatcagccatgagaagctcccttcgctgacgtcgccagaacagcgccgccttgtgcaaagaaaacggccgcgctgctcaagagttccccgggtcggacggctgcgacctgatccagaccagcacggcccaggcgtgcgcctcatggcgaagactggcggcggcctcatttggatcgatccagaccagcgtatgatccggctcggatttggcggcggggtcttccttgacgacggacgcggtccagaagcccgcgaggttgttgatcgcctctcccgttgtcttgacgaaatactgcgacgcttccgcgattcgctcggccggcgtgatcgtcaggccggtttcctcgacgaactcgcgcgccagcgcctgctgttcggtctcgtcgccgtccagcgcgccgccgggcaggtcaaagtaggggccctcgccgcgatcaatgcgcacgcaggccaacttgccgccgcgctccaccaggccaaaggccgtaggacggtcgcggtattcgtggtcgggttgcttttcgccgaactggagcatccgctcctaacgcgcgaacggcctaaaggtcgaaggcgaggcgcgcacgcacgcccttgtgcgctggatcgaactccaccgccgagcgcagaccggaggccatggccgagacgatcttggagcccaggcccgtgcccttgggcgcgccgtcgccgaggcccggcccgtcgtcctcgaccgtcaggatcgcgcgcgtttcgccgtcgggatgcaggtggatgcggatctcgcccatcctgccgggctcataggcgtacttcaccgcattggtgaccagttccgtaaccaccacgcccagcgacacggcttgatcggtggtgacgttcatcggccgggcgtccagcaccagacgcggcgcctcgccgtcgcggcccagcgacctggacagttcgtccatcagcccgtcgaggtattcgtccatggccaccgtcgacatgtcgcctgaggcatagagacggcggtgaacatgggcgaccgcctcgatccgcgcctgggactcgcgcagcgccgcacgggcgccgtcatccgacaggtggcgcatctgcagcgacatgaacgacgacaccagttgcagcgagttgccgacgcggtggttgacctcgcgcagcatggcttcggcgcgatcacgggcccggcggatttcttcgtgcgcggtctcgttctcgcgctgcagtcggcggcgcagcagggcgtcctcgagcgccgcgcgaagcagggcggtgaaatcctcggacacgtccttgatgacgtagtcggcggccccggcgcgaagcgcggccacggcgatgcggccctcctgcgccccggtgacatagaccaccggcggcggcgccggcagcgccatgatatcgggcaaaacatccagaccgtcgcgacccggcatgtagtgatccagggcgcagatgtcgtactcacccgccaccaaggcatgaagccccgcatcgccgtcgggcgcgcaggtcacggcgtatccgtggcgtccgagctccttttcaacgagacgcgacagtccgcgatcatcgtcgatgtagagcaggcgtatgggcgaaggcgcgtccaagggctgttcgttcgtccttattcgatcaccggcgcctgcatcaccgacaggaacaggcccagctgacggatggcgtcggcaaaggactcatagtccaccggcttggtgatgtagacgttgcagcccagatcgtagcaccgctggatctccaccttgtcgtcggtggtggtcagcaccaccacgggcgcgcggcgcaggcgctcgtcgcccttgacccgttccagaatgtcggtgcccgacatgtccggcaggttcaggtccaacaggatcagcagcggcccgttggtcaggatttcctggctgaacaaatagtccagcgcggcgccgccctcgtcgaagtgcgcgatctcgttggagatgttggcgcggcggatgtttttttcgatcagcttggcgtggccatggtcgtcttcgaccatgatgatcttcacgggttgcgtcacagggcggctccagaatccggcaggacgaggcgtttggggaatttcagcagaaaagtcgagcccttgccaagctcggactccagatcgatctgtccgccgagccgtcgcacgctgttgcgcacaaaggccaggccgaggccctcgcccgtccgatcctgacgtccggcgcggcggaacagctcaaagatgcgctcatggtcacgcggcgcgacgccgcgcccgttgtcggcgatgcgatagacgatccagccgccggggacgtcttcgccgctgatctcgatgcgaccgggccggctggcctccagatacttcaccgcattgtcgatcagattgccgaagatctgctccatcgacagccggtcgctgtcgatcatcggcaggtcgcgcaccacgatttcggcgtcggccgtctcagtctggtgacgcacgctgtcggctatgccttgcgccatggccgtcatgtccagcgtctcgatcgcgagattgcgacggccttcgcgcgacagcttcagaatggcgttgatcagccggtccatcttggtggtggaggcgcggatgaagccgatggcctcgggcacgtcctcgcgcaccgcctgcaccacctcgggatcgacctcgcgctcggcctcggcgcgggcgagcgccttgtcgatggtgcgaccggcctgctcaagctcggaggtgtagcccatgacattgaccaagggagcgcgcagatcgtggctgacgatataggcgaagcgctggatttcctcgttggcgcgggtcagttcgccggtgcgttcccgaaccttgtcctctaggctggcgttggcggcgtccagcgcttctcgggccgactgcatctccagcacatagcgccgcaccagccaggccgagattgcggccatgaccagcaccagcaccgccgccagcgtgttgatgacgacggtgatcagcccgaaccgctctgacgtctggatccgcttagcgatgcgggccgacttgatcccgtcgaactcgctgatgtcgttgcggatggcgtccatgagcctgcggccctcgtcgctgcgcacgatctggatcgcctggccgatgcggccttgccgcgccagcgcgagtgtcgaatccatctccgccatcttggcgtccaccgcttcgtgcagccgatcaacgggcgcacgcagttccgcatcggtgtcgccgcggtgcaaagtctccagcgcaggcgccagcgactggcgggcctcctcgaacggctgaaggtactgcggtcggccggtcagaagaaagccgcgctgcgccgtctcggcgtcggtgaccgcgatcagcagcgtacgggcggcgcgacgcatctgctgggcgtcctcgatcgagtcattcacctgcgcggtccgcccgatcatcacaaaggtggcgatgttgaccagaagcagcagcaggaacgcccccgccagcaaccccgccacggcgcgccccacgctcggggtgcgcaggaagtcgccgacgagatgcagggccttgcgggagcgagggatcatgaaggttgctttagccgccgcaagcgtcgccgcatagcgccatgcgtcacacctgtcccagagtcctcaggcgggccttggggtggacctcgttctggctcatcaccaccgtctggccgcggaagcgttcgatgatggagcggacgtaggggcggatcatggggccggtcagcaggaccgcattctcgcccgacatggcgatgcgctcaaaggtgtcgcgggtcgagcggatgaaatcctgaaggcgcgacggcgccatggccagctgcctgtcctcgccctgcccgaccagcgcctcggcgaaggcggcctcccagtcgggcgacagggtgacgatgggcaaggcgccgtcgtggccctggtgctgccagcacagctggcgcgccaggcgtccacgcacgtgctcgaccagggtggagacggaggtggtgtgcggcgcggcctcggccaggccctccaggatcgccggcagatcgcggatcgacacccgttcgcgcagcaggctctgcagaacacgttgcaaggtggtcaccgtgacgacagaggggatcagctcctcgaccagcttcttctcctcggacccgacctccttcagcagcttctgcacctcggcgtaggagagcaggtcggccatgttctccttgaggatctcggtcaggtgggtggtcaggaccgtggacggatcgacgatggtgtagccgcggaaggtcgcctcctcgcgcagggactcctcgatccaggtcgccggcaggccgaaggccggctccttcatgtgctcgcccggcagttcgacctggcggccggccggatccatggtcatgagacagcccagacgcacctcgcccgccccggcctccatctccttgatgcggatggcgtagccctgggtcggcaggcgcatgttgtcgaggatgcggacctgcggcatcacgaaaccgtactcctgcgccagcgagcggcgcagggcgcggatctggtcggtcaggcgccgaccctccaggtcgttgatcagcgccagcagcgaatagccgagttcgatcttgacctcgtcgatcgagagcgcggcggagatgggctcctccacatcctccctgggcttggcctgggcggcggcgatctcggcctcggtcggctcaggcttcagccgggcacggccaagccgccaagccatgaagccggagcccagcgccagcgccgcgaacggcaggatgggcatgccggggatcaggccgatcaagccggccgcgcccgacaccacgcccagcgacaccgggttggtggccagctgggacaccagggccttgtcggccgtgccctccacgcccgccttggacaccagaaagcccgcggcgatggagacgatgatggccgggatctgggtcaccaggccgtcgccgatggtcagctgggtgtaggtgttggccgcatcgccgatcggcatgccgtgctgcatcaccccgatcaggatgccgccgatgacgttgatgaaggtgatgatcaggccggcgaccgcatcgccgcgcacgaacttggaggcgccgtccatggccccgaagaaggtcgattcctgctccagctccttgcggcgcaacttggccgtcgcctcgtcgatcaggccggcggagaggtcggcgtcgatggccatctgcttgcccggcatggagtccagggtgaagcgggccgagacctcggcgatgcgggtcgagcccttggtgatgaccacgaagttcaccaccaggacaatggcgaagatgatcaccccgatgatgaagttgccgcccatcatcagctcgccgaaggcgttgatgacctgaccggccgcgtcatggccttcctggccgtgggtcaggatcagacgggtggacgcaagattcagccccagccggtacagggtcgtgaccagcagcacggtcgggaagatggcgaagtccagcggccgcttcatcatcacggccgtcatcaggatcagcacgctggagacgatcgaaatcgccaggagcagatccagcagcagcttggggaccggcacgatcagcagcatgatcacgccgatcacgccgaccgccatcatcacctcgccgcgcatcagccagccggtgacgtcctggcgcgtcggccgggcgtagccgtccttcatcaggatcggggcgtcggtcacgtggcggcccttgcggcggcgggcgcgtcgtcgggccgtccgtggcccagcgccgccagggcgcgccgcgacgcctcggccaccaccgcctcgcgccgctcgagcggcaggctttcgggcgcgtcatagtagacggcgatcctgaccggcagttcggcggcggcgtaggcgtagccgatgtcgttggtctggccggttccgccggtgccggtcttgtgggctacggtccagccgttcggcacgccggcccggatgcgccctcgccccgtcgggctgtcgatcagccagtcccacagcggccggtgcggcgactggaaggtgaaggggcggtaggtctcctccatccagttcaggttctggaccgtctggttcgcggtggtggtgtcctttgtgccgtccgcgacgttgagcgcgggctccagccggtcgatggaggtcgtctcgtcgcccatggcgcgataccaggcgcgcagcacgtcaaggccgccgatctcgcggatcaggatgttggcggcggcgttgtccgacagttcaaccgtcgcctgcgccagttcggaaatggtcagggtccggccgacggccccttcggtcgtcggccagtggggcaggatgtcgccggccgtgatagggatggggcgatccagggtttcctgctcgcgcgaggcccgctccagcacgcaggcggccaggaacagcttgaaggtcgagcaatagttgaaccgctcgtcgccgcgccaggcgacggcgcgccgctcggccgcggccagtccgatgcggccgccgtgtgtgcgctccaggtccgacaggtcgagcacggcaggggcctggggcggctccacagacgattcccgccgctcgggcgcacgacggcaggcgcccagaccaaggagggccagcccccccaacacgtgtctgcgatccgcctccgccattacgatcaggcggcgtagccggcggcgacgccggattgcggcgcagggatcggcgtgccctcgtcggcgtattcgttcagcttgttgcgcagggtgcggatcgagatgcccaggatgttggcggcgtgggtgcggttgcccaggcagtggctgagggtgtccaggatcagggtcttctccatggccgccaccgtctggccgacaaaggagcgggtcacggcgtccgccgcctgggccgcgcggccggccggcccggcgtcataggtcgaggcgacgggctgcgaagcgggcgcagcgccgggcgtcgtgtgcagcgggcggccgtccggcaggcggatggcgtcggcgtcgatctcgggtccgaccgccagcagcaccgcgcggtgcatggcgttttccagctcgcgcacattgcccggccagcggtgggcgacgatggcgcggcgggcgtccggcgacaggggacgcggggctacgccattggcggcggcgtatttcttgacgaagtgctcggccagcacggcgatgtcgcccggccgctcgcgcaagctcggcagacgcaggttgaccacgttcagccggtacagcaggtcctcgcggaacacgccttcggagacggcccgattcagatcgcggttggaggtggcgatgatgcggatattgaccgacacgggcctggagccgcccacgcggtcgatcacccgctcctgaatggcgcggagcagcttggcctggagccgcgcgtccatctcggtgacttcgtccagcagcagggtgccgccgtcggcctcctcgaacttgccgatgcggcgcgccacggcgcccgtgaaggcgcccttctcgtgcccgaacagctcggattccagcaggttgtcgggaatggcggcgcagttgacgctgatgaacggcttttccgcgcggcgcgagttctggtgcaggtagcgggccatcacctccttgccgacgccgctttcgccggtgatcaggatggaggcttccgagcgcgcgacctggtcggccaggccgatcaccgccttcatcgacggatcggccgagatcatcggcttttcgtcgtcggccaccgccgacagcaccgccgcgatcaggtcggcgtccggcggcagcggaatgaactccttggcgccggccttgatggcggcggcggcctcgcgcgcgtcggcgtcgacgccgaacgccaccaccggcacggtgatgcgctcgttctcgttggccgagatcagggaggcgatgtcgaggcggtagtcgaccatcagcaggtccgccccctgcccgcgccgcagctgctcggtcgcctgatccgcgcgctcgacatggttgacctgggcgccatgcgccatggccatcttcaccgccgtcgccagctggcccgagagcctgcccaccaccagaagccgcatcggtcttcctccttgagttcagtagaggtggtcgcccgtcaggcgcccgtttcctcggtcttgatgatttccgtcatggtgacgcccagacggtcgtcgatcacgaccacctcgccgcgcgccaccaggcggttgttgacgaagatgtcgatggcctcgccgaccttgcggtccagctccagcaccgagcccttgttgagcttcagcagttgggcgaccgacatgtgcgacttgcccagcaccgccgagatgttgaccggcacgtcgaacacgggggccagatcggcggcggtcttgtcgcccggtgcgtcggtggtggccagggcggtcgagtcgccgaattcctccagcgaaaaggtgtcggacatcagaaggcgctccgtgcggaggaaagcggttcggcgtggccggcttcggccgccagggccgaagtcagcgcctcggccacgcgggcggcggaggcgtcggggtcgtgttcggcgcggccgtcggcccattccagctgaaaggcggcggcgggcaggcccggctcctcgcgaaaggcgacggcgccggtgaagccgccggatgcggccgcatcggcgatggtctcgcgggcggcctcgtccaggcccgaggcgcggatcaccaggcggggcgaggcgtcgatctcctgcgccagcatctccagcgcggctttcagcggcgccagcgggtagcggtccagggccgagccggcgatggcgcgcgcggccgccagcgccagatcggccgactgctcgcggtgcgcttgcgccgccgactgtagcgacggcatggcctgagccacgctctgggccactgcgttcagggccatggcgcgaaggttctcgacctcgtccagcgcctgctgccgcgcctcgagccgggcttgagcgaccagggcgtcgacttcggccggcagataggtgcgcttggccggcttccatgcggagggcgtgacgacctcgcctgaggcgtcgaactcggtgtcgaagatgaaggggcgcggggtcatgtcagtagatcagctcgtcgtcggacccttgcccggccagcatgatgtcgccgcgcgcggcgaggtccttggcgacctgcaccatggccatctgggcgccgtcgacgtccttgaggcgcaccggacccatcgactccatgtcctcgcgcatgatcttggaggcgcgctcgctcatgtttgagaagaacatctcgcgcagcgactccgaggcgcccttcagcgccaggcccagctggtccttctccaccgcgcgcagcagcgtctgcacgccgccgggatcgagcttggagaggtcctcgaacacgaacatcagggcgcggatgcgctcggccgcgtcgcggttgcgctcttccagcgcgccgatgaagcgggcctcggtctggcggtcgaagctgttgaagatgtcggccatcatctcatggctgtcgcgcttggaggtgcgggccaggttggacatgaactcggtgcgcagcgtctgctcgatcttgtccaggatttcgcgctgcaccggcgccatgcgcagcatgcgctggacgcattccagggcgaagtcctcaggcagggcggtcagcacgcgcgcggcgtggtcggagcgcaccttggacagcaccacggcgacggtctgcggatattcgttcttcagatagttggcgagaacggcctcgttcacattgccgagcttgtcccacatggtgcgaccggcgggaccccgaatctcctccatgaggccggcgacgcgatcctcgggcaggaaggcggcaagaagcttctgcgtctgctcgtacgagcccatcaccgcgcccgagccggccaggccggagacgaactcaatcatcagggcctcgacggcctcggccgtgacggtgcccagcgtggccatggcctgggagatctccttgacctcctcatcgtccagccgctcccacagctgggtgtggtcctcgccgagcgccagcaggatcacggccgccttttccgggccggtcagcttgttggcgtcctcgaccgctgccttcttggtgaccagcttggccatcagccttccgccacccaggtgcgcaggatgcccgcggcgtcatcggggttggactggacgaagtcggcgaccttcttgacggaggaggccttcacctgaccctcgatgcgggcgatgtcgatgcgctgctccatttccgacgcggggccggtcagttgcgccaattgcggctggccgtcgggaccgatcaccgtggtctggagctgggtaaccggaatgccgccggcgtttgccagggccgggacgttcgcgccgccacccgacgccgtcttcagcagcggacgcagcacaaagaagatcagcagcaggccggtgacgaacagcaccagcagctccaccgcccgcatgatgtcgttcttgccgaagtcgaacatcttgttggcgcccgccaggtcgccctcgatgccggcgtcgcggttgaagcggacgttgacgacctcgatcttgtcgccgcgcccctcgtcgatgccgacggcggcggcgaccagcgacttgatctggccgatctcctccggggtgcgcgcggcgtaggtcggctcgcccttgccatcggcggccggggtccacttgccgtccacggccacggccacggccagcttcttgacctcgcccggctcgcgcgtcgtcgtggtggtggtgttggagatctcgtagttggtggtctcggtgttctccgagttggtggagccgatcggcgtctgggccggcgcctggccgcccggaatgttgttggccgcggtcacgccgccgtcggcctgaccggtcgtgtcctgggactgggagccgttggcggaggtggagcgcaccacctgaccgtccgggtcgaatttctgctcctgggtggtggagcggctgtggtcgatgtcggccgtgacctggacgcgggcggcgccgacgccgacgacgccctcgacgatgtccttgatgcgggcctgcatctgggcctcggtgttgcccttggcctcttccgccgacttgccgccgaagccctggtcctcgctgccggcggcgagcgtcctgttggtctcgtcggcgacggtgacccggtccggcttcaggttcggcacggaggaggccaccaggttgcggatcgcccgcacctgatcggccgacaggtcgcgcccgcccaaccccaccagcacggcggcggtgggatcggcggcggcggtggagaacatctcgcggcgcggcatggtgatgtggacgcgggcggcggtgatgccgcgcatggacatgatggtgcgcgacagctcgccctggagggcgcgctgctcgttcagctgctgctggaactcggtctggccgagcaccgactggttgtcgaagatctcgtagcccaccgagccggaggtcacgagacccttgcccgccagcatcaggcgggcttcgcccacctgatcgcggttgaccatgatggtggagccgtcgcccttggacgagtatttgatgctggcctgatccagggccgaggtgatctcgcccgcttccttcaagtccaggttggaatagagcaaggcgtccggcgcctggccgacgcgcagcatcacggcgaccagcacggccgcgacgccggcggcgacgcccagcaccgcggcgaggcggccgatcccgaacttctgcaacgccgccgtgaagccgcccacgccaccctcgaaaagactggcgggccgttcaagcgccccgctaggcagaaactgccgcccgggtggtaaatggcgcgttaaggctgtttacctttgtggcgatcggcgtcctgcagatgcggcaggacgggctcggcgccggacggcagcggcgcatcgggtgcgcgcaggaaagccagaacgtcgcgatagacgacctcggcctgaaggtcgcggttcagcaggtgccagccgtccggataccaggcggtgcgtagggtcgcagagttcggcaggcgctccagcgcgcgcttcatcggtccgggcttcacgatctggtcgtgcgcgccgtacatcaggatcgccggcgcccggatgtcgcccagccgccgggacgccgtctccatcaggtcgacaaggccgaacacggcgtcgaggcgcgtggccaggatgctgtcgggatcgcggccgttgcggatcagttccagctcattgtcggaggcgcggatgcgccgggcgataaagtccggcgccgtggccgcatagccgccggccatgcgtgcggcgacggagagggccgcgctgttaagccacccctgcgacgaccagccccagacgccgggcgccagcagcaccacccggtcggcgtccggcggccggtccgagccgaaggcggcggtcgccacagagccgcccatgctctcgccgaccacagcgatgacggcgtgcgggtgcgcagcgcgggccaacgccacggcggtgcgcaggtcctcggtcatccggtcctcgcccgcccagcggccgcgacccggcgcccggccgaagccccgctggtcataggcccaggtctccaccccctgttcggcccaccacggcccggcgaggcgaaaggaggcgtcgtgatcgttcatgccgtgcagggcgacgatcacggcccagggttcgccctgcgccggcgcccagcgcaggaacggcaggcgcgcgccgtcgtccatgacgagaaagcggttctccacggccggccccgcgaagcctgcgtgcggggtcatcggcggctgcacatagggggtggcgcaggccgaaagggtcagacccagcgctagagccgcaaggatcggcactctccttctccgctcatccccgcgaaggcggggacccagcgctttgggcgcaagacggctgcgggtcggcccgcgcatcaaaccaaggctccgtgctcggcccggtctggatccccgccttcgcggggatgagcgggagagaggatgtcccgaacgcgcgcttggagatagggcagcacctcggcttcgaaccagggattgcggctgagccaggcggtgttgcgccacgacggatgcggcaggggcaggatgtcgggaccgtagtcgcgccaggcccgcaccgtctcggtcatgttcgccttcgcccgcgcgcccagcgcccaggcctgggcatagccgccgaccagaagcgtcagctccattcggggcagtgcggccagtaggcgaggccgccaaagggcggcgcagcgcggcggtggcggatggtcgccgcccttcgccgcggtgcccggatagcaaaaggcctgggccgcgaccccgatgcgcggatcgtcgtaaaaggtccggtagtcgacgcccatccaatcgcgcagccgatcgccggacggatcggtgaagggcacgccgctttcatgcacccgccgcccgggcgcctggccacagatcaagagtcgcgtctcgggcgagaccatcaccaccggacgcggcgtgtgcggcaggacgcccgcgcaggcgcggcaggcgcggatgtccgacaggacggcctgaaggtcagaggaggtcggcatcgtccccggcggccaccggacggcgggcctgcgcctcggccgcctcctgctcggtcggcaggcgcaggcggatcacgcccttgaagctttccggatcgaccgccttgcccttcttggtgatggtcagccgaccctgccgcatcaggcccaacgcgacggtgcgcaccttgggcatcatccgctgccactgttcgggctgcagatccttggccacctcggaggggcagatgctcttgcccggctcgcgcgtggacagtttttcgaagattgcggtttcgatcgggtcgctcattcggcctatatgctgcaccgcgagagcaagaagaaggcgcgacggctcatggcccggaaaattaccgttcaggaaggcgagttcgccggctggcagacctatgacctgaaggacaccttcgacgtggtggtgggtccgttctatggacgtcccgatccggacgggcggatgcgctgcgcctttcgcgccgagcagaagcacatgaacgccggcgggcgcatgcatggcggctgcctgatgaccttcgccgacatcgccctgttccagatcgcctatcaggaaatggagggcgcttcgggggtgacggtgcagctggactccacctttatcgacggcgcctacgtcggcgagttgatcgaggcgaccggcgaggtgaccaaggccggcaagagcctgatcttcgcgcgtggccagatcaccacgggcgaccgcatgctgatgagcttttccggcgtgatccggaagttcacgccgcgcggctaggcgaagggcgtgaacgccagccgctcccacggtccgccgagatagcgccacagcaacaggccctcggctccgaacgaccagggtgcgaacccggccgcgagttggtcgtgcagggccgcggcgtccttcggatcaaccttgttctggaccgtgacgtgagcacggaagccttgccggtcctgcggcgtcaggtgttcggcgaaacgggcggcgagccggccgcgcagcgcgtccagaggcggggcgtgcagcccgtaggccacgccacgcccgagcttgcgcaggccgacgacctcgacggagaagcgcggttggttcttcgcctccgcctccagcgcgtccatcaccgcctccagccggtcgccgggcaggtggtggaacagggtcaggtgggccgggatttggttcaggcgcgaggggaagtgcgcgcggcgaagcgcgtcgaaatggtcgaaagcggcgggctcgaacgccaggctcaggatcagcggcgccgcgcctccgctcacgcgccggctttcgccgccggccgggcgcggcaggcctcgagccagcgggaaaggttctcgaactcggccggcgggcggtagcggaccagccgcgcgaaatcgagcccgaccacagccacgatgtcggcgatggtgaagcggtcagcggcgatgaagtcgcgcccttcgagatgccggtccagcgtcttcatgaagcgctcggccgagacccggttgtagtcggccacgtgcggcgactgcaccgcctccagcgccgccagcgcaggatggctgtggcgcacgttcagcatcagcggattggcgaggtagaactcgcagcggcgggtccacatctcgatgatggcctgctcgcgcgcgtcgcggccgaacagattgggctcggggtgcacagcctccagatagcggcagatggctatggactccgagatgcaggtcccgtcgtccagctccagcgccggcaggtgcggcacgccgaccctgtcacgataggcgggctgcctgtgttcgccggtcaggatgtcgacctcgaccagttcgacgtccgcaacgcccttctccgccatgacccagcggacgcggcggggattgggcgcgcggttggaagtgtagagcttcatggcggcggtctctcgtgatccgaggtgacgctactgcccgaacacggcggcgggcaaggcgccgaccaccgcggcggtcatcagggtggccaagaatccggcgaacagcgccttccacaccaggcccagcacctcctcgcggcgctcggggatcagcaccgacaggccggtcacggtgatgccgacggagccgatattggcgaagccgcacagcgcataggtcatcagcatgcgggtgcgctcgttcatggcctcggccggcacctggcccaagttgatgaaggccacgaactcggtcagcgtcagcttgacgcccagcagccagccggcgacgcccgcctgcggccactccaccccgatcagccaggcgaccggcgcgaacacgaagcccaggatgcgctccaccgtcagggcctcgccgccgaccacgaagccgcccagcatgacattgaccaaggccacaaaggccacgaacacgatcagcaccgccgagatgttcagcaccaccatcaggccgtcggccgtgcccttgacgatggcgtcgatggcgctgtcgtacttcagcgccgagttgtagtcggccaccgccccgcccatgccgggcgtctccgggatgatgatgcgggccagaagcccccccgccggcgccgagacgatggaggcgaccagcacatgcccagcggcgttcggcagcaccggcgccaggatcgaggcgtaggccaccatggtcgagcccgccaccgtcgccagccccaccaccatcatcagaaagatctcggaccgcgtcagcttgtccagataggcgcggatcacgatggggctctcgatcatgcccagaaagatgttggccgcgacggcgagcgccgaggcgccgcccaggcccatggtcttctggaacagaaagccgaacgccagcgtcagccacttcaggatgcgccagtgccacaacagcgccgacagcgccgagatcaccaggatcagcggcaggacgttgaaggcgaaggtgaacagcgcgccctggttctgcaccggatagggttggtcgccgccggcgagatagccgaacacgaactgcgttccctccgccgtcgccttcgccaggccgtccaccgccccggtcaccgccgccagcacgccctgcgatcccggaatggcgaacagagccaggatcagcgccgcctgcaccccgatcgcgcccagcgccagccgccagggaaacgccttgcggttctccgagatcgcccagcacacggcgacgatgacgaccaggccgagcaggctctggaggttcaggaggttgaacatgaacggcaatccctcgaccggcgctgaggcgtcgcttgaagggcaatgcagcccccgtggcaaggggtcgcagaggctccggcctcggcctctcctcctcgtcgcgcagcgatggggaggtggcgcgatgcgcagcatcgtgacggaggggttctatccgccgctgccccctccgtcccgtcggctgcgccgccggtccacctccccatcgctgcgcgacagggaggagagggatcacagctggcggcggaccagcttgccgtagtgctccatcagctccagcgacagggcgccgggggtgaaggtgtagtcgccgacctcgcggaccggcgtgacctcgaccgccgtgccggtcaggaagcattctctgaaggtggacagttcttccggcagaatgtcgcgcacctggacctcgatgcccttctctgcggcgatctccagcaccgtctggcgggtaatgccgtccaggatgaagtccacgcgcggggtgtggatcacgccgtcgcgcacgaagaagacgttggcgccggtcgcctcggccacatagccgcgccagtccagcatcagggcgtcggcgaagccgcgcttctccgccgcgttcttggacatggtgcagatcatgtagagacccgccgccttggcggtggtgggagccgtcgccgggtcggggcggcgccatttggcccactccagccggatgccttgcgccttgaccgccgggtcgaaatagctgggccagtcccacaccgcgatggccaggtgcggcttgttgttcagggccgagacgctggtctgttccgggcccagataggccacggggcgcacatagcagtcgctgaggcccatcttggcgcaggtcgcgttgcaggcggcgtcgatttcggccacgctgtagggaatatcgaagtcgagcaggttggcggaccgcttcagccgctccgtatggggcgtcagcttgaagatttcgccgccgtacatacgctcgccctcgaacaccgacgaaccgtagtggaggccatgggtcagaatgtgcgtcttcgcgtcccgccagggcacgaaatcgccgtcgaaccagatccagccgtcacggtcgtcgaaaggaacgaaggccattgaagaacatctcccggaaaccttcaggggttagagccccgggcgccgccgaggtcaacgcctcatgtgaaggacccgcccgatgagcatgaccgattcgcgcccccacggacgctcgggtcccgtcgccggcccgggcgtcggccgccacctgctgatcgtcgacgacgacgaccgcatccgcgaactgctgaaggagttcctggcgcgcgaaggctatcgcgtgacgggcgcggcgcacgctgcggcggcgcgccggctgatggagctgatcgagttcgacctggtggtgctggacatcatgatgcccggcgagagcgggttggacctgaccagctgggtccggagcaaggccgagctgtcgcgcacccccgtgctgctgctgaccgcgcgcggtgacgccaacgaccgcatcgaggggctgtcgcgcggcgccgacgactacatgtccaagccgttcgagccgcgcgagctggcgctgaggatcgacgcgatcctgaggcgcaccggcggcaagccgatagggcccaaggaggtccggctgggcgccgccaccttcgacatggagcggctggagctgacgcgcgacggcgcgccgcagcggctgaccgaggccgaggcgcagcttctgaagaccctggccctccatgcgcacgcgccggtcgagcggatgagcctgtcgccggacaccgccgacatcaccgggcgcgccgtggacgtgcaggtgacgcgcctgcgccgcaagctggaggccgacccgaagaacccgcgctatctgcagaccgtacgcggcgtcggctacatgctggcgcccgactgagatgcggctgcgccggcggctgaacctgtggccgcgctttctgaagcggcggctgccgacctcgctgtggggccggtcgctgctgatcatcgtcctgccggtgctggcgatgcagatcgcggtgacctgggtgttcttcgacgcccactggcagaccgtgaccgcgcgcctgtccgagggtctggccggcgacatcgcctgggcggtccagtcctatgaggacgatccgacgcccgccaacatggccgtgatcgccgaccgcgccgagcgcgccatgcagctgtcggtcgcctttcaggaggaccgcaccctgccgacggagacgcggcgcggcgcgatcggcgtggtggaccgggtgatggagcgggcgctgcagggacggctggacaggccgtactggttcgacaccacccgataccccgcctacatcgacatccaggtgcaggagccgggcggtgtgctgcgcttcatcgcgccgcgcgagcgggcggtggcgactcaggcccacatcttcgtgctgtggctggcggtggcgaccatcctgctgatgggggtggcgatcctgttcatccgcaaccaggtgcgctccatcgagcggctggccgatgcggcggaggcgttcgggcggggtgaaagcgtgccgcgcttcaagccgcacggcgcgcgcgaggtgcgccaggcggcgacggcgttcatggccatgcgcgaccgcatccagcgccacatcgaccagcgcacggccatgctggcctcggtgagccacgacctgcgcacgccgctgacccgcctgcggctggagctcgcgctggcgccgcccttcaagcgtcaggacgccatgcgcggcgacctggacgagatggagcacatgatcgacgaatacctagcctttgcgcgcggcgaggcgggcgaggacacccagaccgtggcgctggcggatctgctcggcgccgtggccgaggatgcgcgccgggccggagccgaggtcgaggtggaggtctcgccggggctgacagcctccttgcggccgctggcgttcaagcgcgccctgaccaacctggccggcaatgcggcggcgcacggtgagcatgtgcggctgtcggcgcggcccctgccctccggcgggctggaaatcgaggtcgaggacgatgggccgggcataccggaggcgatgtacgaggacgctttccggcccttctcgcgcctggacgaaagccgcaaccagaaccgcaagggcgtgggcctaggcctggccatcgcgcgcgacgtggcgcgcggccatggcggggacgtcaccctggggcgcagcgatctgggcgggctgaaggcggatatccgcctaccgggctgacgcggcggggactggcgaaaggccctttgaaggcgcatcttttcgacagacagggctttgtcggagatccatcatgagacccctcgcctttttcgccccggccgccgccgtgatcgcgctcgcgagcgccgcccaggcccaggctccggttcaggcgccaaatgtcaccgtcaccgtgggagccaagctgcaggagcaggtcgaagaactgggtccgcgcgaggtgcgggatcaggccgatcgactggccgaacgcgtgcgcgaggcgctggcgcgtcgcaatgacctgaacgggacggccgtcaatctggtcctgacggacctgaagccgaaccggccgacgctgcagcagctgacggacaggcccggtctggaccgcatccgcagcgtcagcatcggcggcgccgccgtggagggcgagatcgtcaccgcggacggccgcagcctgccgttcgaatatgaccgcttcaactcaagcctggccgacgtttacggcttcagcacctggtgggaggcggaccgcgttttcgaccgcgtggcgcgcaagatcgccgaaggcgacctctagctctggcctcgtccgggcctagttccggcccatcttgcggttgcgccgaacggcggcggccacgacctcggccatcaggcggtcgatgcggccgccctccgccatgacgtcgagaccggcgcgggtggagccgccgggagaggcgatgcggccgatcaactgatccagcggctcgtcgcctgcgctttcggccgccgcgacaaaggtcgcgcgcgcgagggtgcgggcggtgtcggccggcaggcccgccgcctccccgccccgcgccagcgcttcggtcatcgcatagaaataggccgcgcccgatccggccacggcggtggccgcgtccatcgccgcctcgtccggcagatccaccgtgacggccatcggctcgaacagggcccgaccgagcgcccgcgcggccgcatcgccggcgtagacggtggccacgccgcgcccgcgcgcgacgcccgtggtgggcatcacccgcacgatcggccagggaccgaccccctccgccagggacggcgccgtgacgcccgccatcaccgacaggatcaccgcctgctcgccgaggtgcggcaggagcggcgcaagcgcttcgcgccagaccgcaggcttcaccgccaccacgacgcagcgcgcgtcacgcagcgtctccagcggcgggttgatccgcgcgccttccgccctcgccgtctcggccgcaggcttctcggagggcgtcaggatgatcaggtccgaaggccggacggtttccgtcagcagccagccttccagaatggccgaccccagtcggccgcagcccagcaggacgaccaggccgctcgccgccatcaggcggtgcccacggtctcgaacaggcaggcgtcgatggcctcctgcggcttcttggatccgcggatcatgaagtcgaaggcgggataatagcggtccgccgcctccatcgccgcatcgatcatcgaagccgcctgcgccagcgtcggccgctcgccgtgcggcaccgacagcgagtggcggaagacgatctcaccgtcctcggcccagacctcgaaatggcccatccaggtgcgctgattgatcatgccgaccagttcataggcggcggtgcggcggctcttggtcgcgcgcaggtccagggcgcagcacagctgcaggcagtcgccctcgggccgccaggcgaaccacagctcatagtccttccagtcgccggccatggcgaaggcgagatcgccctcttcggtgcggtcgaacggcaggttctcggccgtcagcacatattcgaccacatccagcggatcgaagggaacatcgacctcttgcggcccggcgacatccatgcggcgaactcgtcctttgaacggcgaagtgaatggtgaatcacctcttaaccggacgctagacgtgttcggggtcgcggctcaaccggctgcgtcgaccgggggagttccgtctgtggagtttcccgcctcaggcttgtcggccagcttggcggcgaaggcggcgcgcatcaccaccatttccgcgcgaagcgccgcgacctcgcccttcagggcgtcaagctcgtcgcggcgcaccaggtccatgtcggcggccaggcgatcggtctgggcgcgccaggcggacttggcctcctcgcccgccgcctgggccaggcccatggcgccggtggtcagcttggcgaactcgtccaggatggggttgcgggtctgcatgggcgtgctccgcccggcgcgccgggctgttgaagggtctgaagtggatataggccctgcttcggccacggcgaagggccagtgtccggcaaaagcgtcgcagccgccgcaacaaaccggcgacgacgacggcgacgcttgctaaaccacgccgaaccgaagcgctcgaggaccgcccttgccctttcccgaattcgatccggttctgatcagcatcggtccctttccgatccgctggtacgccctggcctatgtggcgggcatcgtgctgggctggtggtacgcgtccaagctgatcaagaccgaacgcttgtgggcgccggcgcgcccgccgctgacgccgaaccagctggacgacctggtgctgtggatcgtgctgggcatcatcctgggaggacggctgggctacgccctgttctacgatccggccatgtacggccagctgttcaccggccagagctgggccgagcggctggagctgttccagctgtggacgggcggcatgagcttccacggcggcttcctgggcgtctgcctggcgatcgtgctgttcgcgcgcggccagaaggtcgacatgctgcggctgggcgacatggtggcgccggtggtgcccatcggcctgttcttcggtcgggtcgccaacttcatcaacggcgagctgtggggccgcgagacgaccgtgccgtgggcggtccgcttctgcaacgacagcatccagcggatgtacggcttctgcccggcgggcgacgcgccgcgccaccccagccagctgtacgaggcgggcctggagggcctgctgctgctgggcctcttgtcgctcggcatctggaagatcggcatgctgaagaagccgggatacatcaccggcctgtttctgctgttctacggcctgtcgcgggcggcgctggagaatgtgcgccagcccgacgtcggcatgcctgacttcccgctgggcctgaccatggggatgatgctgtcgatcccgatgatcctggtcggcggctggctggtgtggcgggcctggagccgtccgcccgtccggggatgacggccgacacgctcaaggcgcggctggcgcgcgaaatcgccctgtcgggcccgatgacggtcgccgactacgtcacccgctgcctgcacgatccggccggcggctattatgcggcgcatccggcgctgggcgcgggcggcgacttcatcaccgcgcccctggtcagccagatgttcggcgagctgatcggcctgtgggcggccgagacctggaaccggctgggcgcgcccgaacgggtgcggctggtggaggtcgggcccggcgacgggaccctgatcggcgacgctctgcgggcggcgcggctcgcgcccggttttctggaggcctgcgatctcgtgctgatcgagcctagcggccccttgcgtgcgcaacaggcgcgggccctggccggtgcggacctgcagccccgctgggtgcgcggcctccacggcgttgaaacggatgcaccggtgatcctgatcgccaatgaggtgctggactgcatgccggcgcgccagttcgtgcgcaccgagggcggctgggccgagcggcgcgtgggcgtcactgaccacggcggcctgttcttcggcctgaccggcgtgacggcgggcttcagcaagccggacttcaacatggcgcccggcgaggtgctggagatttcggaccagcaggcggcgttcggacgcgacctgggcgccctcatgaagcaggcgtcaggcgcggccctgatgatcgactacggccgggcgcggcccgaggccggcgacaccctgcaggcgttgaagcgccacctaaaggtcgatccgctggaggcgcccggccaggccgacctgacgcaatgggcggacttccccctggtgctggaggcggcggtgcgcgcgggggccgacgtgaccggctgtctcggccagggcgagttcctgcgtcgtctcgggatcgaagcgcgcgccgaggccttgaagactgggcgccccgacgccgcaccggtgatcgaccgccagctgaaccgcctgaccgcggaggaccagatgggaatcctgttcaaggccgccgcgatcttttcgccccgctcgctggtcgtgccggggtgggacgcatgagcgcgccggagccgatcacccatccgctgctggacggcgtgcgccacggtttcttcacgcgggcgggcggcgtctcgacgggcctctacgccgggctgaacacggggatcggctcgcgggacgatcccgccgccgtggccgagaaccgcagccgcatcgcccaggccatgggcggaaccgccgccgacctcgccaactgttatcagatccactcggcggtgacgcgcgtggccgaagggccgtggaacggcgaacggcccgagggcgacgcggtggtgacggcgacgcccggcgtgatctgcgcggtgctgaccgccgattgcgcacccgtgctgctggcggaccgggaggccggcgtggtgggcgccgcccacgcgggctggaagggggcgctgggcggcgtgatccattcggcggtggcggccatggaggcgctgggcgcgcggccggagcggatcagcgccgtcgtcggcccgtgcatcgcgtccgaaagctatgaagtcggcgctgatttcctcgaccgcttcgctcatcatgatccgggcagcgagcggttctttcacgctgcttccgccccggacaagcgactgttcgacctgccaggctttgtgctgtggcggctggagcaggccggcgttggtcaggccgcgtggaccggcgacgacacctgcgtggacgaggcccgcttcttctccaaccgtcgggcgcaccagcggggcgagccggactttgggcggatgatgagcgtcgtcaccctttagcggcgaccgaccttcagcccgcccgcgccagctccggcacccgaaccgtctcacgccaggcgtgcggctgggccagcagggcgcgcaccagcttgttgttcacggcgtgcccagccttgtagccgtcgtaccggcccagcagcggcgcgcccagcacatacaggtcgccgatcgcgtccaacgccttgtgccgcacgaactcgcgttccatgcgcaggccgccggggttcagtatctggtcgccgtcgatcacgaccgcattctccagcgagccgccgcgcgccagaccggcccgacgcagcgcctcgacctcgtgggcgaagccaaaggtccgggcggccatgatctcacgccggaaggtcgcctcgtccaccacgaagtcgatcacctgattgccgatgacgggcgtcgggaagtcgatctcgaaccgcatctcgtaacgatcgcaaggcgtcagggccgcgtgcttgtcgccctcggtgacgtggacaggctccaggatctcgatgtagcgcaccggcgtcggctggcgacggaagcccgcccggtccagcagttgcacgaagcccagggccgagccgtcaaggatcggcagctccggcccatccacctcgaccgtcacattggcgatgccgagtgcggcgaaggcggccatcagatgctcgatggtcgacaggcgcacgccggccgcgttctcgatcatggtgttcaggcgcgcgtcgaccaccgcctcgcccgacacgcggatgcggttctcgcggtccttgacgtccgtgcgcacgaagacgatccccgcgcccgccggggcgggacgcaccaccagacgcacgcggcggccggtgtgcacgcccacgccggcgcagatggccggcgccaggatggtgcgttggtgatggtcgtggctgaccgacaaggcagaactcgcttcttcgcatcggcgccggttgaaccgctcgcggttcgcgcctcatgagtcctctagaacgaggactgcaatgccgaaagcaaagtccggtttccgattgtttcgtaacgggacggcgacggaaacgtaaaacgccccggagcgagctccggggcgcttcaggtcaggcgcggcctcgatcagttggcgaggcggcgtagaaacgaggggatttcgagatcgtcatcgctggacgaggcctgcggctcgggcgcggcggccgtctgtgtcgcctggcgcatctgcggctgcggacgcgggctgtaggaggcttgcggctgcggacgcttgccccgaccgaacaggctccagccgctgcggcggtgatcccggtcgtagtcgtcctcctccatcaccggctcaggccgcgcggcgggcgcctcgcggcgcggctcggcgcgcgcgggctgggccggctgggcggtctgggccggcgtgcggtgggtctcgtactcctcgacccagggatcgacgatgggatcaaggctgcgcgtctccggcgcggcgtggatcaccggctcggggcgggcctccatgcgaggctcagggcgcggttcgggcgagcgcgcaggctcggccgcacgggccgtgggcgcggcttggaaggtcggctgcaccggcgccgcctcgatacgcggctcgggcgcccgcggagcctctgtgcgaaccggttcgcgatatggcgcgcggctgggctcgggcgcgcgggcggatgcgccatacaggccgccggccgcgcgacgggcgtcgtggttggccaggggcgaggcggtctcgggcgccgtgcggccagccgtctggccgccgcctggtccgccctgggcgcgcgccagctgctcctcgtccatgcccgtggcgaccacggacacgcggatcttgccgtccagcgccggatcaaaagccgcgccgaagatgatgttggcgtcgccgtccacctcggccgagatggcgttggcggcttcgtccacctccagcagagtcatgtccaggccgccggtgatgttcaccagcacggccttggcgcccttcagcgaggtctcgtccagcagcgggttggcgatggcgttctgggccgccagcagggcgcggtcgtcgcccgtggcctcgcccgtgcccatcatcgccttgcccatttcggacatgacggcgcgcacgtcggcgaagtcgaggttgatcaggcccggcaggatcatcaggtcggtgatcgaacgcacgcccgagtgcagcacctggtcggccatgccgaaggcgtcggcgaaggtggtgcgctcgttggcgacgcggaacaggttctggttcgggatgacgatcagggtgtcgacgtagcgctgcagctcggcgatgccgctgtcggccaggcgcatgcggtggcggccttcaaaggtgaagggcttggtcaccacgcccaccgtcaggatgccgcggtcgcgcgcgcatttggcgatgatgggggccgcacccgtgcccgtgccgccgcccatgccggcggtgatgaacaccatgtgcgcgccttccaggtgcgcgtgaatctcgtcggcgctctcctcggcggcgttcatgccgacctcggggtgggcgccggcgccgagcccttgcgtgatcgtctcgcccagctggatgcggcggtcggtcttggcgaacgacagatgctgagcgtcggtgttggcgaccacgaactcgacgccctccagcccggcgtcgatcatgttgttcacggcgttgccgcccgccccgcccacgccgaacacgacgatgcgaggcttcagttccgtgttctgcggcttaaccaacgagagcgacatgactttaccgaccttccgacctgcctgcgacgccgatgcgagcccgccgattcgcatcgttacacgtccgttaatgaatcaacgcgcgaggtaaaggaagggttaagttgctcttccgccgctttgccgaagagagcgaaaggcaaaggttccagccatccggaacgaaaaaggcccgaggacatccccgggcctttgccgactttaagcagaggtcagaacttcagcgaaaccgacgccgtccagcgacggccgagattgtcgatgtaagccccattgtagtaaccgtttcggcctaaagtatcctcatcggtgacgttgtcgatcacgatctgggctctggcgttgtcagtcacgtcgtaccccagcgacagggtgtgcagagtgtagccatcgtagcggatgatcggttggaactcgaggccgatcggtgtgccgcccgacttgatgcgagtggcgtcttgtatttcggtcgtccaacgcgcgttgaacttgccgatgttgtacaacgccgtgagttgcgtcgaccaaaccgggttcgccagcgtatcctcgccggacaccgagtcatcgaactcgcccgttccagacgtggtgtactccagcagatagtagatgttcccgcggaagccgaagcggccaagatcgcggtttgcagtaaatacgtctgcgagatcaaccgaatagctgaagttcgagttgatcgccttaacccgggtgccgcccaggttgaagaacggcagctcgaagccgttggtgaagttgaagttggtgtcccgacgaatgccagcgcagctgttgacgccgatatcgccgctgttgtccgggaagttcgcgctgtcgtagcagaactcggcagccggttgggccagcaagggcccaagcgcgcccgtgacggtgatctccaggtaatcggcagcgaagatgaagttcgggatgaaccggggcgtcgccacgaagccgtaggtgaaggagtcgccctcttccgggacgagatcttgggtgccggagatcaagcctgtgaacgaggcgcccgagggcgtgaagttgcggttaaggaagtcctccgccgtcgcgcggtccgtgatggacacggggcctgacgtgcccgtcaacgtgccgccattgtccgtggcgcggttgaggacatcggtgatgcagttggcgcgacgtgcggttgggttaggaccgacgctgatgttagcggtcgagcacgggtccgccgaagaggtgaagaagggctgaccgcctaggaacaattccacgatgctgggctggcgcacggacttcgacacattgccgcggaacaggatgtcttcgctcggctgccaagtggccgccagagtatagatctcctgggtctcgccttcgtagctcggcgacctcagcgtgccggtcgtatcgcggaacgaaggcgcggaaccgtccagtttactgtaacggaccgacgggttcagttcgagcgaccgaacaaacgggagcgtgaagtcgccgccgaagatcgggatgcgaagctccaagccgccttccttggtctcgacctctgcaaaggtggtcgctgacggcgcggaacgcgtagcgccgatgcgcgagatttcgtccaccgtgtagccgagttcctccttgcgcaactcgcccgacaaggcgaactgcaccataccggcgggcagattgaagaggtccccagacaggatcgcctgggtgaagttctgagtcgactcgttgttgaagaagttgcgtacgctgatgtaatccttcgcggcctgcgacgcgcgcccttcaccaaagatgttcaacggctgacaggcgtccacgagcgcttgcgtggcgttggtttggaacacgatctgttcgcgcaccccgtcggcgccaatctggctgatgacgttgggttgcgtgccgggaatctggccgccgtagctagccaggtaggccgagaggccgtcgcgttgagcccggcattggacggcgccgccgacgttgaccgcatcgatggctagagcaaaggcgacatcgttgatcgcactgaattcgacgttcgtttccgcacgaccataggtgtgggacaattcccactggaagtcgcgatcaaacagcgagaagtcgccgttgaagccgttgacggtgcggaaggtctcgtttgtcgagatttgcgataggtcgttgacgatgtcttcgttgtagcgcgagacggtgaagtttccggtgatacccgccgccgccaaagctgtgcggttttgagccgtcagatacgggtgattgacgttcaccaggatcgccgcgttctccgtcgagctcgacgaaacgccgttgaacaggccgccattgctgaaggggttgcgaaccgtgacatccgagtacaggttttcagtgaagaagcggatgttgtcggtgacctgatagttggcgatcaggttgccaacgttgcgctcttgctcgacccgcaggacgttggagtcggtgcgattggccccgtcgccgccggctcccgtggcgaaggtgccgggcgtgtcgggtccgccggatcccaagctgtaggtctcgagatcgccgttccggttgaagcggagcggcgcagccaggcgcggcagaacgcccgcgccgattcccgtgttcgcgatgtccggcaggccggcgaggaagctgcccgcgaaggcgttgagaggcgtattcggattggctgcgtaatattcacgcgccgtgggattgcgctgctgcaggatttgcaaggcggccgtacgcaactgcgcggccgtcgcgcccgcgggcggggtgacgccgtaaaaggcgaacacacgcgcggcggttgcatcctgcgcagccggcgtcgcgccgggcagggccgagggcgcgaaattacagatgcgcgggttagccgcggcggcggtggccgcctgagccgcggagaaggcgcccgcgttacagaggttcggagcacccggaacttgctgcagggtgcccgagataaacgagaatcctggggtcgccacccgcgcgaagccgggctgcgtgacggcggcctcggccgttccgctaccagagacggtgttgaacacgacgccgccaaaccactgattgatctggcggaaacggtcgccgtagatagtcgacggcacgccatctacgccaccggcgaggaatgcggtcgaaccgaccaagccaggggtgaacgccggattgcggaagccgccattggcgaagttggagatgctggtgatattatccggacggaaggacgcccgatcgctcgccagcaggctgtcgatcttgctgtactcgcccgaaattgcgacgttcagacgatcgtcgaggaagttatcgccccaagtcgcgttgaccgacacccggccagcgtcggcatactcgaaggtttgaccgccgataatgttgatttcggcgccttcgaaatcgtccttcaggatgtagttgaccacccccgacacagcgtccgcgccgtaggcggcggctccgcccacggtcaggatgtcgacccgatcgatgagggctaccgggatggtcgatgcatcgacctgagatccggtttcgttacccgaaacaaagatggtggcggagttgtttgaaacaaagcggcgaccgttgaccagcgtcagggtacgtgcagtacccaagttcagcaaatcgatgtacgtcacgcccaaagacgcggtttgagcgccgttcgttccattgaggttggcgccgccgccgaccagcgggatgtcgttcagcacatcgcctgcgttggtgaacagacgctcttcgatatcctgctctccaacctgtacgccggggatcacgccttcatactgcggacgagggatacgagatcccgtgacgacgatctcgtcaacgacagcagcctcttgttcgccagcctgagcaggttggctctgcgtgttcgacgaagccgcaggcggtgatgacggttgtatctgagcccacgtcggcgcggctgcagtgagcaagccggcaaggaccgtggtcccgaatagatggtgacgcttcaacatcgacgatccctcaaggtggccctctccccatgagccgaccaccgttcacgaccaccattcacaaggaccgggcccgcatcaaccagcccgtccggaaatcggcgagatcgtgtcaatacagcgacattttcgccacatccgccagcaaaccgttggtgaactaaaggttttcccgcagccagcccgccacgcggccgacgacattgcctctgtagacgcggggagcgtcggctgcggtgatctggcgggccatgagcttgcgggcggagacggcttcgcgggggccgtaggcggcgcggagcaggacgccggcggaggcgcagaaggcggggccggaggcggcgtcggccaggtgcggcgcgcgttggggctttccgagacggacagggcggtcgaacacacgcacggccagttcgcgcacgccgttcagctggctggcgccgccggtgagaacgaggccggcgccgggctcgagccccacgccggcgttgcgcaggcggtcgcgcagcagttccagcgtttcctcgacgcgcggggcgatcacggtcttcagcatggcgcgcggcacgatcacgggaccggcggaggcgtcctcgccgcgcggcggggcctccagcatctcgcggtcctcgttggcgctggccatggccgaaccgtgcagggtcttgagccgctcggcgcccgccttggaggtcgagaggccccgcgcgatgtcggaggtgacgtggtcgccgccgacgttcagcgattcgatgtgcagtaagctgcgcccgccccagacggcggcgctggtcgagccgccgcccatgtcgatgcagacggcgccaaggtccatctcgtcctcctccagcgcggccagagaggagacgacgggggcggcggcgacgccctggaggtccaggtgcgccagctccaggcagtggctgagggtggtgaagacgttctcggccatggacacgaccaggaggtcgagacccagcgagccgccgcgcatcgagcgtggatcgtgcacgccgcgcgcgccgtccaccgaccaggcgatcggcaggacgtggatgggccggcgattcggcagacggatctgagccagggccatgccgatggcgcgcgccaggtcggcgtcgcccaccggattggcgcccagcgaaacacgggcctgcacccggtggcttgccatctggccgatggcggtggtgacgatgacgccggacacggggctggaggcggcgcgctcggcccgctcgaccgcgtggccgatggcctgggcggcctcgtccatgttgatgatggccccgcccctgacgccgcgcgactggacgtgactggcgccggcgacgcggatggtgcggtcggcgtgtcgcacgccctcgggcttcatgatgaagcaggagaccttggactggccgatgtccagcgcggcccccaccggcgcgcggcccgtacgcgggtccccgcccctgccgtgatcgttggctgcgccgccgcgttccttgccgcccatgacggttggtgtccttcttcttgtcaggcgccggagggccgcaccgcgacctcttcgggggttcggagatcgacgcgggcgaagcccaggtcgagcaggcgttcgcgctgatccagcgcgtcgagacggatcagggccgcctcctggtcgatggccggaagctggatcaggctgccgtccttgaggcgcaggtcccagcggcgctcgtccacgcgcaccagggcgtcgacgcggcccatcaagcgggggcgctgggccagcagcggcagcacctcggcggccgcctggtcggcgcccttgcccaccaccagcggcaggccgggatagcgaccagcctcggcgtcggggatgacctggccctggccgtcgatgacctgggcgcggccggcggactgccacacggccaggcggtcgtgctcgacgacctcgacgatcagggtgtcgggcaggagccgcaccacgcgcgcctccttgacccagccgaccgcctggacccgcgcgcgcaccgcatccagatcaaggccgaccagcggctggccggcgtggaggcccagcgcctgacggacggccggctcggcctcgcccgaggcgccggcgatgtgaacgcgcttcagcgaaaagcccatgccgacggtgacggtgtcgatcccgtgcgagatcgaggcgccgatgcgctcggcccgcgcgcctgtcgccagcacaacggccagcgccagaactccggcggagaggcagacaacaacggcgcggggggacaggtccaagcggccgatggccgccatctggccggggatggccccggcgctgcgtgaagagccgccgcgcgccgaccccctccccccggaagaggcgccgcgcggggagccctgaacaccttgtcgccgaccgccgcgaactaccgcgggcatgaggcgtcctccaccatccaacgcaccagatcttcgtaactcatgcccacataggccgcctgctcgggcacgagcgaggtcgaggtcatgccgggctgggtgttgacctccagaagaacgagatcgtcgttaacatcgtcataacggaagtcggatcgcgacacgccgcgacaccccatggcggcgtgcgcccgttcggcttcgcgcagcgccgcctcgaacacatgggcgggcagcgccgccggcaggacgtggaccgagccgccgggcgtgtatttggcttcgtagtcgtagaaacccttggtcggggtgatgtcggtcacggtcagggcgcgcgggcccgtggcctcgcccagcacggccacgcacagctccttgccggcgatatagggttcgaccacaacctgctcgccgtaggtccagccgtcggcgcccacggccgcgaccggcgactcgtcggcggagcggaccagatagacccctacggaggagccttcggcgttcggcttgatgacgtaaggcggcgtgatgacgtgaccgcgcgcgacctcgcgccggtcgaacaggcccccgcccggcacccgcacgccggcggcgcgcagcacggacttggacttctccttgtccatggccagggccgaggccagcacgccggagtgggtgtaggggatgcgcagcgtctccagcacgccctggacgcagccgtcctcgccccaggcgccgtgcaggcagttgagcaccacgtccggacggatcagaccgcccagcacattggcgagatctcggccggcgtcgatgcgcgacacgcgcgcgccctgcgcctccagcgcccgtgcgcagccctcgcccgagttcagcgacacctcgcgctcggccgagaggccgcccatcaggacggcgacatgcaggtcggaaagagggcggttcatgcgcggctccgggaagcccacctccatgccgccgacgcggttaacagcccgtcaaccaaaggggcgacgattgcgcaggttcgtcccttggctgagccgggatagcggtggcggcgggatgaaggcggcgtgctttcaaccgttagcccaagctctatctcgggcaggactgtccgcctgtcggccgaacgccgacgccagcagccgacccgttgcggacggtcgctcactagacgatggtgaaatccgagatggaacttcatcaaacccccttcatcgccttaacgatgagcgcccttatcgttcacgtcgtgagcggcatcgtcgcagtttcgacggggcgaagctggatgcgcgagttgtccagactcgctcagaccgtccggttactcagtgttcgacggcgagaggttctttcgccgctgtcgttgaagatggtggtcgtatcccgaacagccttgaccatagcggtgttttcgcttggactagacttggtcatcaacgcttagcgagcagcaaaaccatgtccgcttccacgccgaggcgtagttcgggtcacgaccgataccgttgaaaaagtcggcaattgccacgggcggcgagtgctgattcactctggtcattgaggctggaggcagcgcgatgatgggcgagcggcgggtcgatcaggcggccctgttctatactttctcgctggaagaccacgtccctgcgaaccatctgctgaggtcgatcgaccggttcgtggagttggaaggtctgagagggcatctggcgccgttctacagcgccatgggtcgcccctcgatcgaccccgagctgctgatccggatgctgctggtcggcttttgcttcggcattcgctgggagcgtcggctgtgcgaagaggttcacctgacccgggcctcccgcgggttctgccggctaggcctggaaggtgccgggccggatcattcgaccttctccaagaaccgccacggccgctttcgcgacagcgatctgctgcgccagttgttcgacacggtgctgcgccgctgcatggctgaaagcctggtcggcggcgaaggctttgccgtggacgccagcctgatcaaggccgaggcgaaccgggaacgcagcgtgcctggcgatccgggccttccgcccgaggcgtcgagccgggccatcgacgagtatctggcggtgctggacgacgcggcgttcggtgcggctactccggtgacgcccaagttcatctcgccggtggatccggcagcgcgctggaccgccgccaacaaggggccggccttcttcgcctatgccaccaactacctgatcgacctgaagcacgccgtcatcgtcgatgtcgaggcgtccaccgccgtgcggccggctgagctgacggcggcccgcaccatgatcgagcgggttcaggataggcatgatctccaccccgaccgccttgccgctgacaccgcctatggctcggccgagatgctggaatggctggtcaacgaccaggggatcgcaccccacatcccgatcatcgacaagtctggccggacggacgggaccttctctcgagccgacttcacctatgatcccaccgccgacctttatcgctgtccgggcggcaaggcgctgaagcagtatcggcgtgccttccgagccgatcatcccgagacgccgccggatgacacctatcgctatcgcgcctccaagatagactgcgacgcctgcgctctgaagccgcgctgctgtcccaacacgcccgcccggaaggtcacgcgctcaatccacgaaggtgcgcgggacttcgctcgcgccatcgccaggaccgacgcctacgtcgtttcaccgcgcgagcggcagaaggtcgaaatgctgttcgcccacctgaagcgcatcctcaggctggaccgactgcgtcttcgtggtccctgcggcgcccgagacgagttcctcctcgccgccaccgcccagaacctgcgcaaaatggctcgactgatcccgcaaccgaccgctcccacgcccgcctgaaggcctgaagcgtcacgatcccatcacagcctgaccacgcagccgtgctgtcccgtcagccatccgactttttcaacggtatcgacctttagcggacattgtaattgtggacccgcaccgtaaagtgagcttgataacggagggttcattgcacaagctcgtctcgtcagtcgttctgctcctaggtcttgcatcgtccgccgccgctcagagtgtcccggagggggtgcaccgcctcgccgacggtccatcggcgatgtgcgggattgtcgggatgaacgctaccgaactcgtagaaaccgcgcggcagtcgccagacctgaggccggtgaccatctcctctgaccggttcgaactgttcgaagggggcgatcctgtcagatttcagctggtagctacgctacctgctgagccggcgtttccggcggtttcttgccgtgagctatacgagacgggaggggcgcttcggatgaagcgatccatgcgatgcgacgccgatcgcgccgactgcgatgcactcttccaagagttccaggcactagacgccgagttcaagagattgatgcaaggcgaaggtcgctgatgagtgttgccgccaatctcggcggcccggaaaaggtgttttagcttcaccatggcattcgcgcgcacaagcctgatggcgtttagcttgctgctcacttcttgctccggggtcgaagctgaaggtgagctgcgtcacttcgcaggagtctggctgtacgagttggagggttcgaccttcattgaaggtgcaactgacataccttcagagcgcccaccctatgacgaaaccgactggctggattggttagaagaaccacggctagaagctctcatagaggatcatgttggcgatccagactgtcatgaagtgcagccgttcctgatcacgtttattggtcgccggacgcgcaatccagatcgcggtgcgggtcatatggcgctgtggcgttctgaggtcacgatcgacagaacaatctcggccaagaggctcagcccgtcattctgctatgacggctaaccagccttagctgacttcagagacgtctgcttcgcgacgtcagccgctgcgccccaaccgcctgatctcccaatccagctgcacaccggtcttcgccagcacatccgcgcggacggcttcgcccaggccttcgatgtcggccgcggtggcgtcgccggggttgatcatgaagttggagtgcagttcgctgaacttggcgccgccgccggtctcggcgtgcagccggccgcgccagccggcgtcgtccaccagcttccatgaggaatggccgggcgggttcttgaaggttgagccgccggtcttctcgcggatcggctgggtggtctcgcggcgggcggtgatctcgtcgatgcgcgcctggacggcggcgggatcgtcgtgggcgccgcggtaggtcgcctcgatccagatgatgtcggccggcgcctgcgagtgacgataggcatagccgaaatcggccagcgcatagtccacccgctcgccgccgcgcgtcaggccccaggcggagaccagcacgtccttggtctccgagccgtagcagcccgcgttcatggtcagggcgccgccgaccgtgccggggatgccggcgtagaactccagccccgcgatgcccgccttggccgaagcgcgggcgaccatggcgtccagcgcgcccgcgccggccgtgatcctgtcgccgtcggccgccacgcccgcgaacgatcggccggccagccggatcaccacgccctcgaccccgccgtcgcgcacgatgacgttggagccgacgcccagcaccgtcaccggaacgccggggtccagcgccttcagaaaggcggcgagatcgtccgcgtcggcgggtatgaacagcgcctcggccgcgccgccgacccggaaccaggtaaagggcgccagcggctcgtcccgcagcagcttgccgcgcacggggggcaggtcgatcacgacagcgcctccagctgcgccggcagggcgtaggcccaggcggtgatgtcgccggcgcccagcagaaccaccaagtccccgtcccgggcctcgtcgcggatcaggcgcggcaggaccgcggcgttctccagcgcctggacgtggcggtggccgtagcggcgcacgccgtcgaccagggcgtgcttgtccacgccctcgatcggcgcctcgcccgccggatagacgtcggcgacgatcacgctgtcggcgtcggagaagctggtggagaactcttccagcaggtcgcgcaagcgggtgtagcggtgcggctggaccacggcgatgacgcgcccgccgtcgctggtctgggtgacctgtcgcgcggccttgagcacggcggcgatctccaccggatggtggccgtagtcgtcgacgatgcgcacgccgtcgaccacgccggtggtggtgaagcgccgcttgaccccgccaaaggaggccaggcccgccttgatcgcctcgtccgccacgtccagctcgcgcgccacggcgatggcggccagggcgttggagacgttgtgccagccggccatgggcagatgcagcccctcgatccgggtggtttcgccgttctggatcaccacgtcgaagcggcagccgtcggcggccatgtcgcagttctcggcccgcaccatggcctggggattgaggccgtaggtaaccaggcgccggttatcgacgccggccaccagcttctgcacctccgggtggtccaggcagacggccgcgaagccgtagaaggggatgttctcgacgaaatccacaaaggcctgccgcacccggtcgaagtcgccgtagtgatccaagtgctcgggatcgatgttggtgacgatggcgaccgtggacttcaggcgcaggaagctgccgtccgattcgtcggcctcgaccacgatccagtcgccgtcgccgaccttggcgttggtgccgtaggcgttgatgatgccgccgttcaccaccgtgggattcagcccgcccgcgtccagcagagccgcgaccatggaggtggtggtggtcttgccgtgcgtgccgccgaccgccaccgagaactgcagccgcatcagctcggccagcatctcggcgcgacgaaccagggggatgcgtcgcgcccgcgcggccttcatctccggattgtccgccttgacggcggtggaatagaccacagccgaaacctcttcgcccagatgcgcggcgtcgtggccgatgaagatgcgcgcgcccagccgctccagccgctcggtgttggcgctgctcttggcgcccgagccctgaaccgaatagccgatcttgagcatgatttcggcgatgccgctcatgccgatcccgccgatgccgatgaagtggaccggaccgaggtcgaacggaatgggacgaaggcgcgcgatcatcgtcgcgccttagcaaggctttacagtgattgcacgatctcagatgcggcggccggcgggcggcgcatcggcggcggtaaacgacggcgttgtcacctgcgtgacctgcgcggcgaagcgcgcgaccgcctccacatagacttcgttgcgctctaccggacccatgtgacccgcctccgggatgcggaccaggtttgcgcgcgggatggcctgggcgatgaactcgcccgcgtgatccttggtcaccacgtcgcggccgccgacgagcaccagcgtgggaacggggatgcccggcaggctgtcggtcaccgaccagcggatcatggccaggttgccatgagcctgcacggccggagacgtcagggtcggcaggcgagcggtcaggtccagctgcgcgcgcgtcggccaggcgccgaagccggcgatccgcatggccagatgggtcgagccgctgagatagctttgccagttcatcagccagacaagcggcgacaggatgatgtccagccgcatcatcagctcgatcagcggtcgcagcgcagtcaccagaccgctcatgatcatggtgcgcaggggattgtggtgggtggtgttctccagcaccacgccggccacccgcccgttcagcatctcgggataccgggcgcaaaaggtctgggtcgtcatgccgccgatgctgtgaccgaccaccacgatcggccgatcctcgggcaggcggtcgattaccgccttcaggtcgtcggcgaagccttcgatcgaccacccccgcgtcggccgggtggagaggcccgcccccggcagatcccaggcggcgacgccgaaacggtctgacagggaggcgctggcgtcggcccagatacgcgaggacatgccccagccgtgggtcagcagcaggatcggcccgtccgcccgtccctcgatctccagacgcaggcgcgatccgtcggcgccgtcgaccatgacgccctcgcgccgcttgtccgacgccatgccgccgccgcggcccaaaagcagcaggatcaggaaacggccaaggaaagagaaggcgagcagccccagcccccagtacaaccggtcgttcgacggatcggcgaagcccagcgcctccgcctcctgctcgcggtcccaccagctccagacaagccagccggataggccaagaaccgccagcgagaccagggcgaagagacgctggagaagagcaaacaggatcatcggaacgcctgacaggagtgttgcggggctaaccgtcgccatgcgcgggcgttccgcggatgccggaaataaccccgccttaaccgtaaggattcaccatcccggcatctgagttgcggggccgctttccatgtccgagttgaagaccgacgtcatccaccggggcgactgcatcgaggtgctgcgcgccctgcccgacgcctcggtcgacatggtgttcgccgacccgccctataatctgcagctgggcggcgacctgctgcgccccgacaactccaaggtcgatgcggtcgacgacgactgggacaagttcgggtcgtttgcggaatacgacgccttcacccgggcctggatggccgaatgccgccgcgtgctgaagcccgatggctccatctgggtgatcggcagctaccacaatgtgttccggctgggctcggcgatccaggacctggggttctgggtgctgaacgacatcgtgtggcgcaagtccaaccccatgccgaacttcaagggcacccgcttcaccaacgcgcacgagacgctgatctgggcggcgcgaagccgggaccagaagcgttacaccttcaactacgatgcgctgaaggccttcaacgaagacgtgcagatgcgctcggactggaccttccccttgtgcaccggcgaggagcggatcaaggacgccgacggcaagaaggcgcatccgacgcagaagcccgaggcgctgctgcaccgcgtgctgctcagcgccacccggcccggcgacgtggtgctggaccccttcttcggcacgggcacgaccggcgcggctgccaagcggctgggccggcgctacatcggcatcgagcgtgaccagacctacgcccaggtggccgagacccgcatcgcctcggtgatcccggccaatgcagaagacctgcaggtcatgggctccaagcggcacgagcccaaggtgccgttcggcgccctggtggaggcgggcctcctgcagccgggcgaccgtctgtactgccccaagggtcagcgcgaggcgcgggtccgcgccgacggctcgctgatctcgggcgccctgaccggctcgatccacaagcggggcgccctgcgggagaccgcccccgcctgcaacggctggacctactggcgcttcaagtccgaccaggggttcaagtccatcgacgcgctgcgggccgaggtgcgggcgggcatgcagtaagcttccccagcggcaactttcgaccggcgcggtgcggaaccttgccggtcttaagacattcatgctcacggccgcgcttgagcgggtcggagcacagacatcatgaagatcgcgcaggtcaccccgctgtacgaggccgtgcctccgaagctgtatggcggcaccgagcgtgtggtggcgcacctgacggacgccctggtcgatctcgggcacgacgtgacgcttttcgccagcgcagacgccgagaccaaggcccgtctcgtgcccgtgcgcgatcaggccatccgcctggatcccgcgccgctgaagtcggacctggccgcgcacatgaccatgctggccgaggtgctgaaccgcgccgacgagttcgacgtgatccacttccacaccgacatgatccactttccgttcttccgaaagtgcgccgacaagaccctgaccaccctgcacggccggctggacatgaaggacctgccggaggtgtatcgccgctggagcgacttcggcctggtgtcgatctccgatgatcaacgcaagcccctgtccttcgccaactggaccgccacggttcaccacggcatgccgggcgaccagtaccggttcagcgccaagtccgacggctacctcgcctttctcggccgcatctcgccggagaagcggcccgaccgcgccatcgaggtcgccaccaagctgggcaagccgctgaagatggccgccaagatcgacgcggccgacaagcgctattgggaagagaccatccggccgctggtcgagggcaatccgttggtggaattcatcggcgagatcggcgaccatcagaagtcggacttccttggccgggccgaggcgctgctgttccccatcgactggcccgaacccttcggcctggtgatgatcgaggccatggcgtgcggcacgcccgtgatcgccttccgttgcggctccacgcctgagatcatcgaggacggcgccacgggcttcctggtcgacaccatggagcaggcgatcgccgccgcgggccgcgcgcacctgctggaccgcgaggcgattcgggcccgcttcgacctgcgcttctcgtcgatcgccatggcccgtcgctatgtcgaggtttacggcgacctgatcgcggcgcgtcggccgaacctgggcgcggggctgaacctcggcctcaacgacgacgtgtccaagctgcgccgcatcggcgaagaccgctccttcgccgtctcggcctgaatggcgtcctgagcatttcgcaggcggcggggtgaaccctcgccgcctgttttcattagattccccaagacgatcccgaaggcggcgaaccggcgccgcattcgcataggacgttccaacggcctcgaactctcaaggagacctcatggacgacgcctatacgacccagatggccgccgccgaatccgcggagagttcaggcctggccgaactgatggcgctgaaggaaggcgacgcctttctggtcgccgatcactggggcgacctgaagggcggggcggacggcctgttcgccggcgacacccgcatgctgtcgcgctggatcatgacggtgggtctggcgcgtccgtccaagctgagttcgggcgtctctcaggacaacgtcttcttctcgtgccacaccaccaaccgcccgctgccgccgatgggcgggcgttcggcgccggccggcgtgctgcacatcgagcgtcggcgctttctgtggaagcggcggatgttcgagcgcgtccgcatggtcaaccacggcgtggaggacgtgctgctgccgctggcgttcgacttcgccgccgacttcgccgacatctttcaggtccgcggcacgccgcgcaccaagcgcggaacggtcgagacgccgaccaccgacggccgccgcgtcgccttccgctaccaggggctggacggcgtcgaacggcgcagctgcttggccttctccgagccgcccgcccgcctgaccgggacccgcgcggagttcatgttcagcctgcccaaaggcaaggaactggatctgttcgtcgaatgcggcgtggacgcctgcgagacgccggaccgcggccgctggcggctgaactcggtcgaggcgaggctggcgatgcgggccaagcggcggcgcggcgcctccgttcgcggcccgcgcagcccccggttcaacgactggctggaccagtcgcgcgccgacatcgccctgttgaccaccgatctgccgacgggcccgtacccttacgcgggcacgccctggttctcgacgccgttcggacgcgacggcatcatcacggcctggcagatgctgtggctcgacccttcgctggccgaaggggtcctgacctatctggccatgcgccaggcgaccgagaccagcgccttccaggacagccagcccggcaagatcatgcacgaaacgcgcggcggcgagatgagcgcattgggcgaggtgccgttcggcctctactacggcgggggcgacaccccccgcctgttcatcgccctggccggcgcctacgtccgccgcaccggcgactacgccctgatccgccggctgtggccgaacctgatcgccgccgccgactggatgcgcgactacggcgacagcaacggcgacggcctgatcgactatcagcgcggcgccgacacgggtctgtccaaccagggctggaaggattcggaggactccatcagccacgccgacggccgtttccccaagggcccgatcgcgcttctggaggtgcagggctacgcctacgccgcctggaaggcgatgggcgagttcggcgaacacctgggcgacccgcgcgccgcggagtggcgtgagcgcgccgagacgatgcaggccctggtggaggagcgcttctggatggaggacgagggcttctacgccatcgcgctcgacggagacggcgagccgtgccgctccatcggttccaacgccgggcatctcctgttcaccggcctgccgctggcgacgcgggcgcacaaggtgacgcgccggctgctgtcggccgagttccgcaccggctggggcgtgaggaccctggcgcatggtcaggcgcgcttcaatccgatgagctaccacaacggctcggtctggccgcatgacaccgcgctggcggcggccggcatggcccagtacggagagcgcgatgcggtggccctcttgctgggcgagatttacgccgccgccgcccacttccacctgcgtctgcccgaactgttctgcggcttcacccggcagccgggcgagccccccatcgcctatccggtcgcctgcctgccccaggcctgggccgccggatcggtgttcctgatgcttcaggcgtgtctgggtgtccaggtggacgcgctggagggcgtggtcacggtggatcgtccggtgctgccggccggcatcgaccgtctgaccatctccaacctgcaggtcggggaggcgacggtggacctggcgttccagcgggtggacggccacactgtggtgatgccgcgcaaccggcgcggcgacgtctcggtgcgctcccttcgttaggccagcgcccggtccagcgccttcttgaacacggtgggcagggccgcgcgcgcctgatccgccgggcgccagtcgaacggccccttagccgtcgcctccatcacccgcagagtcagggcgaagtgggtgaagacgtgctcgaccgcgccggcgtcgcgccactcggccgcgacgggcggatccagcggcggcggctccgaagtccactccgaagtcggcaggccggccatgccgcccagcagccccttgtccggccgccgtaccagcgcgacccggccctcgccgtcccgcagcacataggcgatcccgtgccgatgcgggcgttcggccttcttcgccttcagcggataccgctcgggcgcgccggagcggtaggcctggcaggcgaaggggacggggcacaaagggcacagcggcgacttcggccggcacacggtcgcgcccaggtccatcaccgcctgcgcccagtcgcccggacgcgcctccgcgaccaggccgccggccagccgccgcaactcaggccgggcggcgggcagcggcgtctccaccgcgaacaggcgcgagaccacccgctccacattgccgtccacgacgttggccggctggtcaaaggcgatggccgccaccgccgcggcggtataggcgcccacgcccggcaggctcagcagccccgcctcggtgtcgggaaagacgccgccgtgctcgttcgccaccgcgcgtgcgcaggccagcaggttgcgcgcgcgggcgtagtagccgagccccgcccaggccgccatgacgtcggcgtcctcggccgccgcgaggtcgttcaccgtcggccaacgctcggtgaagcgcaggaaatagggcgtggcgtgcgccaccgtggtctgctgcagcatcacttccgacagccacacgcgatagggttcggtgcgttcggccgcgcccggcgggctgcgccacggcaggacgcgcgcgcccgcgtcgtaccagtcgagcagggcctgtcggagagcggagacgtcggacatcagtcaggctatatagggccatgcgccgccccctgcccaccgacgccgaggtccgcgaaatcctgt

SEQ ID NO: 10 - DNA, 20 bp, synthetic construct
  source 1..20: mol_type = other DNA
gcattcaagtcaacggcgat

SEQ ID NO: 11 - DNA, 20 bp, synthetic construct
  source 1..20: mol_type = other DNA
cgaactgaaccagctcgatg

SEQ ID NO: 12 - DNA, 20 bp, synthetic construct
  source 1..20: mol_type = other DNA
tgaaggcgctgtcgctcgac
